European Patent Application EP 4 506 459 A1, published February 12, 2025. Title: A Nicotiana tabacum plant with mutations in FT and SPL genes and its use as biofactory. Applicant: Consejo Superior de Investigaciones Cientificas (CSIC). The sequence listing filed with the application follows.

SEQUENCE LISTING (139 sequences)

SEQ ID NO: 1 - DNA, 549 bp, Nicotiana tabacum
  source 1..549: mol_type = genomic DNA
atggaaacagctggtcatcataatatctctactagtgaggatgattataagaagaagaaaggcagttgtaataataatattacaacaaataataaccatattaagaaagggtcattaaataatggagggtcaagtactaatcaaaggtgttgtcaagctgagaagtgcagtgctgatttaagtgatgctaagcagtaccataggaggcataaagtctgtgaataccatgcaaaggctcaagtcgtcgtcgtcgccggactccggcaacgcttctgtcaacaatgcagccgatttcatgagctgacggaatttgatgaatcaaaaagaagttgccgaaggcgtttggctggacacaacgaaaggcgaagaaagatcagctcttcatcatctgcagcagagtctcaaattgcagaaagttcaagtagaaaagggacagtgcaactcaataataaggacattaacatgatgtgtggtcaagtaaatgaaaagggaagaattcagatttcaatccaagaaaattccactttcaaaaatttccacccccgttga

SEQ ID NO: 2 - DNA, 546 bp, Nicotiana tabacum
  source 1..546: mol_type = genomic DNA
atggaaacagctggtcatcataatatttctactagtgaagatgattataagaagaagagaggcagttgcaataataatattacaacaaataataaccatattaagaaagggtcattaaataatggagggtcaagtactactcaaaggtgttgtcaagctgagaagtgcagtgctgatttaagtgatgctaagcagtaccataggaggcataaagtctgtgaataccatgcaaaggctcaagtcgtcgtcgtcgccggattccggcaacgcttctgtcaacaatgcagccgatttcatgagttgacggaatttgatgaatcgaaaaggagttgccgaaggcgtttggctggacacaacgaaaggcgaagaaagagctcatcatcaactgcagagtcacataatattgcagaaagttcaagcagaaaagggacagtgcaactcaataataaggacattaacatgatatgtggtcaagtaaatgacaagggaagaattcagatttcaattcaagaaaattccactttcaaaaacttccacctccgttga

SEQ ID NO: 3 - DNA, 516 bp, Nicotiana tabacum
  source 1..516: mol_type = genomic DNA
atggaagcagctgataataatgacttgttcatttttgccactgataatgatgacaagaagaagagaacccccagttataataataggagtagtagtagtagtaataataacaatgaaaagatcaaagggtcaagtacttcaatgaggtgttgccaagctgataagtgtactgttgatttaagtgatgccaaacaataccataagaggcataaagtctgtgaataccatgcaaaggctcaagccgtcgtcgtcgccggactccggcaacgcttttgtcaacaatgcagccgatttcacgaggtaggagagtttgatgaatcgaaaaggagttgcagaaggcgtttggctgggcacaacgaaaggcgaaggaagactactactacttcttcatcatcagatcagtctaatgctgaagtttcatcgagtagaaaagccataatagggacagacactcatcagataataaacttccaagaaaatgcagcagcaggttataaacactttcagattggatga

SEQ ID NO: 4 - DNA, 411 bp, Nicotiana tabacum
  source 1..411: mol_type = genomic DNA
atggaaactagcaaatgggaagagaagagaagcatgatggaagaggaggatgacgaggaagacgaagatgttgtagaggacaacaaaaggaagagggtcttgactcgctcgggaaggaaggtacctggcggagagggttcaaagctgccttcctgtcaaattgaggactgcactgcagatatggcaaatgccaagacataccatcgccgccacaaggtctgtgaatttcatgcaaaggctccggcagtacttattggcggactccgacagcgtttctgtcagcaatgcagcaggtttcatcagttgggggagttcgatgaagcaaaaagaagttgcaggagacgtttggcaggccacaacgaacgccgtcgtaaaagttcatgtgattctcctggagaagggtcaagttaa

SEQ ID NO: 5 - DNA, 423 bp, Nicotiana tabacum
  source 1..423: mol_type = genomic DNA
atggaaactagcaaatgggaagagaagagaagcatgacggcagcagaaatggaagaggaggatgacgaggaagacgaagatgttgtggaggacaacaaaaggaagagggtcttgactcactcgggaaggaaggtacctggcggagagggttcaaagctgccttcctgtcaaattgaggactgcactgcagatatggcaaatgccaagacataccatcgccgccacaaggtctgtgaatttcatgcaaaggctccagcagtacttattggtggactccgacagcgtttctgtcagcaatgcagcaggtttcatcagttgggagagttcgatgaagcaaaaaggagttgcaggagacgtttggcaggccacaatgaacgccgtcgtaaaagttcatgtgattctcctggagaagggtcaagttaa

SEQ ID NO: 6 - DNA, 402 bp, Nicotiana tabacum
  source 1..402: mol_type = genomic DNA
atggaagataacaaatgggaagggaagagaagcatgaatgaagcagaagaggaacatgaaaatgctgaagaggataacaaaaggaagagggtattgactctctctggaaggaatctatctggtggtgggccagcactgccttcttgccaggttgagcagtgcactgcagatatggcaggtgccaagccatatcatcgccgccacaaggtgtgcgagtttcattcaaaggctccggtagtacttattagtggaatccagcagcgcttctgtcagcaatgtagcagatttcatcagttgccagagtttgatgaagcaaaaaggagttgccggaggcgtttggcaggtcataatgagcgccgccgtaaaacttcatatgattctcatggagaaagttcaagctga

SEQ ID NO: 7 - DNA, 411 bp, Nicotiana tabacum
  source 1..411: mol_type = genomic DNA
atggaagataacaaatgggaagggaagagaagcatgaatgaagcagaagaggaagaggaggaacatgaaaatgttgaagaggataacaaaaggaagagggtattgactctctccggaaggaagcaatctagtggtgggccagcactcccttcttgccagatcgagcagtgcactgcagatatggcagatgccaagccataccatcgccgccacaaggtgtgcgagtttcattcaaaggctccggtagtacttattagtggaatccagcaacgcttctgccagcaatgtagcagatttcatcagttagcagagtttgatgaagctaaaaggagttgccggaggcgtttggcaggtcataatgagcgccgccgtaaaacttcatatgattctcatggagaaagttcaagctga

SEQ ID NO: 8 - DNA, 960 bp, Nicotiana tabacum
  source 1..960: mol_type = genomic DNA
atggctatacgcctgaggctaacgggaatagagtggctagcgcttgatcagtttgctcgctgcaatgaagagtactctgtggtttaccttgattggcttggttgttctatctcagtatcagataaagggctaacaatatctttgatcagttgcttctctttgcctggaattaactgttggtactttgcttccaggttccatcggttgccagaatttgaccaagggaaacgcagttgccgcaggcgcctagcaggccataatgagcgtcggaggaaacctccacctggatctcttttgtctaatcgctatggaagtctttcttcatcaatatttgaaaacaatggcagatctggaagttttctggtcgacttcactgcatatccaaatctcactggaggtgcatggccaaatactagatcatctgatcgaggatgggataatcaatccactgcatcagggaagcttctccaaagtcattggctgaacggttctgaaaatcctacatccgaccttgttctgcaaggttcagttgcaaggggtgccaattattctggtcctggtattattccttccggaaattgcttctctggagtctcagattccagtggtgctctctctcttctgtcaaatgagtcatggggctcgaggaaccaatcctctagcctcggggttaacggcttggttaacactgatggcggacataccgttcagccatcgggttcccatgctgctcctgtcaatcactactcaggctctctatggggatttaaaggaaatgaagctagtagcagttcacatgcaatacctcctgatctcgggcttggtcacatttctcaacatgctgtcaatcagtactctgctgagcttgggatggctcagcacagtggaagacagtacatggaactggagcactcaaagggttacgattcttctgttcagaatgtgcactggacactttga

SEQ ID NO: 9 - DNA, 1161 bp, Nicotiana tabacum
  source 1..1161: mol_type = genomic DNA
atgaatgggctcagtaagtcggaaatggaacttctggcttctgcttcttcttctacttctactacttctacttcccctgactctcctcctaacactttaaaatttggtcaaaaaatctactttgaacatgttggacctcaccaccccaaatcagcaactgggtcgtcttcatctccggtcaccggaactccggcgccgacgacgtccaagaaaggaagagggggtggtgtggttcaaggtcgacagccatctaggtgtcaagttgaagggtgtgaagcagatctgagtgatgttaaggcttattattcaaggcacaaagtctgtgctacacattctaagtctcctgtggtcattgttgctggtcttgaacaaagattttgtcaacagtgtagcaggttccatcggttgccagaatttgaccaagggaaacgcagttgccgcaggcgcctagcaggccataatgagcgtcgcaggaaacctccacctggatctcttttgtctaatcgctatggaagtctttcttcatcaatatttgaaaacaatggcagatctggaagttttctggtcgacttcactgcatatccgaatctcactggaggtgcatggccaaatactagatcatctgagcggggatgggataatcaatccactgcatcagggaagcttctccaaagtcattggctgaacagttctgaaaatcctacatccgaccttgttctgcaaggttcagttgctaggggtgccaattattctggtcctggtattattccttccggaaactgcttctctggagtctcagattccagtggtgctctctctcttctgtcaaatgagtcgtggggctcgaggaaccaatcctctagcctcggggttaacgacttggttaacactgatggcggacataccgttcagccatcgggttcccatgctgctcctgtcaatcactactcaggccctcaatggggatttaaaggaaatgaagctagtagcagttcacatgcaatacctcctgatctcgggctgggtcacatttctcaacttgctgtcaatcagtactctgctgagcttgggatggctcagcacagtggaagacagtacatggaactggagcactcaaagggttacgattcttctgttcagaatgtgcactggacactttga

SEQ ID NO: 10 - DNA, 1101 bp, Nicotiana tabacum
  source 1..1101: mol_type = genomic DNA
atgaatgggcagtggaattcggtaatggaactgggttcagtttcttctcctggtagtaattcaagttcctccgactctctcaatggtttgaactttggcaagaaaatctactttgaaaatgtgggtggtgggtcatcgccggtgaccggagccgggaacttgccgccggcgtccaagagggggaggggtgggttgatgcagggtggtcagccacctaggtgtcaagttgaaggttgtcaggtagatctgagtgatgctaaggcttattattcgaggcataaagtttgtggtatgcactctaagtctcctactgttattgttgctggccttgaacagaggttttgtcaacaatgtagcaggttccatcaattgccagaatttgaccaaggaaaaagaagttgccgcaggcgcctggcatgccataatgagcgccgcaggaagcctccatctggatctcttttctctacacattacgggagcctttcttcatcaatttttgaaaataatagcagcaaatctggaagctttctgttagacttcagctcacacccacatgtcaacgagagttcgtggccaaatactagagcatctgaacaaggatgggatcatcaatctactgcatcagggaagtgtcttcagcgtccttggctgaacaattctgaaaatgctacatctgagttagttctgcaaggttcagccaccaggaccaattatgttccttcaggggaatgtttttctggagtctcagactccagtactggtgctctctctcttctgtcaaatcggtcctggggatcaaggaatccaccctcaagtcttggagctaacattgatgggatacacaccattcaaccttctgattcccatggtgcacctaccaatcacttctcaagcccttcgttacggtttaaaggaaatgaagctagcagcagttcacacgagatgccttctgatttgggtttgggtcaaatttcacaggctgctgacgatcagtactgtggtgagctggggataggtcagcagagtggacgacaaaacatggaactggaccactctaacggttatcatccttctgttcagaatgtgcactggtctctttga

SEQ ID NO: 11 - DNA, 1110 bp, Nicotiana tabacum
  source 1..1110: mol_type = genomic DNA
atgaatgggcagtggaattcggtaatggaactgggttcagtttcttcttctggtagtaattcaagttcttccgactctctcaatggtttgaagtttggcaagaaaatctactttgaaaatgtgggtggtgggtcatcgccggtgaccggagacggaaacttgccgccggcgtccaagagggggaggggtggattggtacagggtggtcagccacctaggtgtcaagttgaaggttgtcaggtagatctgagtgatgctaaggcttattattcgaggcataaagtttgtggtatgcactctaagtctcctactgttattgttgctggtcttgaacagaggttttgtcaacaatgtagcaggttccatcaattgacagaatttgaccaaggaaaaagaagttgccgcaggcgcttggcatgccataatgagcgccgcaggaagcctccatctggatctcttttctctacacattacgggagcctttcttcatcaatttttgaaaataatagcagcaaatctggaagctttctgttagacttcagctcacacccacatgtcaacgagagttcgtggccaactagagcatctgaacaaggatgggatcatcaatctactgcatcagggaaatttcttcagcgtccttggctgaataattctgaaaacgctacatctgagtttgttctgcaaggttcagccaccaggaccaattatcccggtcctggtgttccttcaggggaatgtttctctggagtctcagactccagtaccggtgctctctctcttctgtcaaatcggtcctggggatcaacgaatccaccctcaagtcttggggctaacattgatggggtacacacccccattcaaccttccgattcccatgctgcacctaccaatcacttctcaagcccttcactgcagtttaaaggaaatgaagctagcagcagtttgcacgagatgcctgatttgggtttgggtcaaatttcacaggctgctgacaatcagtaccgtggtgagctacggatgggtcatcagagtggacgacaaaacatggaattggaccactctaacggttatcatccttctgttcagaatgtgcactggacgctttga

SEQ ID NO: 12 - DNA, 975 bp, Nicotiana tabacum
  source 1..975: mol_type = genomic DNA
atggaatcatcatcctcatcctcatcctcgtctaagagggcaaaagcacctggcaatattgctcaagtagctcattgcttggttgatggatgtaatgcagaccttagccaatgcagagagtatcaccgccgccataaagtttgtgaggtccattcaaagactgccaaatgtttatctcgatctgatggttccttttgtaggtttcattccttggtagaatttgatgatggaaagagaagctgtcggaaacgtttggatggacataacaggcgtcgaaggaaacctcagccagattctatggccaaaacttctggattactttttactggccagcaagggacgaaacttctgtcatttagcagtcaacaaatttttccaagtgcagctgcatgggctggcgtagtcaaaacggacagcgaaatggtattatacaacaaccaatcgcatataaattgcatggacaatcaaaactcgttccctgattcttcagctcgtagctacaaaggaggaaatcaattccagttcatgcaaggcagtgaccgtagtctccctgaagcttcaatctaccagccacttgttgatcatcccaattctgcagtagcagcagcagttcctagcagcggacaaaagatcttctccagtggattgaacgaaattgtggactctgatcgtgctctctctcttctgtcatcagcacccgctgtaactagggagattggttttagtcacatggtgcagcagcctgccactatcccccggccccagtcacaatctgtcgttcatagcctgcactatggtggtctaagccagtacccttttgctcaagatttcaatagccaacctcaagattctgctgcagattcacatgttagcaacaacagctctctgcatttccatgatatgttacaaaatggagcagatggatcatctacaagtggtggctgtcagcaaacactagcctttatgtgggactaa

SEQ ID NO: 13 - DNA, 981 bp, Nicotiana tabacum
  source 1..981: mol_type = genomic DNA
atggaatcatcctcctcatctaagagggcaaaagcacctggcaatattgctcaagtagctcattgcttggttgatggatgtaatgcagacctcagccaatgcagagagtatcaccgccgccataaagtttgtgaggtccattcaaagactgccaaagtcacgattgggggtcgagaccaacgtttctgtcagcaatgcagcaggtttcattccttggtagaatttgatgatggtaagagaagctgtcggaaacgtctggatggacataacaggcgtcgaaggaaacctcagcctgattctatggccaaaacttctggattactttttactggccagcaagggacgaaagttctgtcatttagcagtcaacaaatttttccaagtgcagttgtgagctctgcatgggctggcgtagtcaaaacggacagcgacatggtattatacaacaatataaattgcatggacaatcaaaactcgttccctgattcttcggctcgtagtagctacaaaggaggaaatcaattccagttcatgcaaggcagtgagcgtagtctccctgaagcttcaatctgccagccacttgttgatcatcccaattctacagcagcagttcctagcagcggacaaaagatcttctccagtggattgaacgaaattgtggactctgatcgtgctctctctcttctgtcatcagcacccgctgtaactagggagattggttttagtcacatggtgcagcagcctgcctctatcccccggccccggccccagtcacaatctgtcgtacatagcctgcactatggtggtctaagccagtacccttttgctcaggatttcaatagccaacctcaagattctgctgcagattcacatgttagcaacagcagctctctgcatttccatgatatgttacaaaatgcaccagatggatcatctacaagtggtggctgtcagcaaacactagcctttatgtgggactaa

SEQ ID NO: 14 - DNA, 1392 bp, Nicotiana tabacum
  source 1..1392: mol_type = genomic DNA
atggagtggaatgcaaagtgggactggggaaacctggtaatgtttggttcagaggccgccaaaagtccaaaagaactacaattaacagattggggagttgaagaagatggagaacttgatgctggatccttcaatttgtcaagtggtggtagtggtagtggtagtggtaccggtggttatgtctctgatgttgggcatggttcttcgatcaagagctcaatatcagcttctactgactcttcacccaaggagggcttgaaagcatgcaacttttctttcgatggctcttctgaggatcttagtaagaaagtgaaactttgctctagaaattcaccccccatggaggcttcagtaggctctgttgaaccacttataggtctgaaacttggtaagcggacatttgagaccatcggcggtgctaaggtttcatccttccccgagaaacacgtatcatctgctgcagcagcaaagaaaacaaaatcatctactcagaatgcaccaactcctcgctgtcaggttgaaggctgcagccatgatctttcatcagctaaagaatattaccggaagcatcgagtttgtgacagtcattccaaatgcccaaaggtcattatagcaggtgtagcacgtcgcttttgtcaacagtgtagcaggttccatagcttgtctgaatttgatgaaaagaagagaagctgtcgcaggaggctctctgatcacaatgcacggcgccgcaaaccacagcaggaaaccatccagttcaactcggcaaggctttcttcattgttttatgatagcaggcaacctatgaatcttgtgctcaaccattcccaactggttcagtctagagctgctgcaaattctacctgggaaagcactgaagaaactaagttcagtataacaagagggtctactccaaagcctgaaagagctggcagtacaaatgggctgtcattattgccagggatccagttgtcacgggccgtgggtgcacacagtaatgtatctagctgcttgctcttgccctccaagggccacacatccgaggttttcaatcgaggtgccacggaatccatgttcaatatgggtacaggacgggaatttcctcgtgctctctctcttctgtcaactaattcatggggttcatccgagcctgagactgtttcactgaacaacccaacacacgcgaatcagagcagcatgcccgagcagatgatgcaggcaattccacaaggtgtgccacttatgtcctgtgaatactggcagggtgaacaaccctcatccgatcctcgtgaccatacattggctgctaatagtcatgctggtggtagctttcagggaatcgagctgttcaaacctccatttgacactgacttttatctcaatgcattgaactga

SEQ ID NO: 15 - DNA, 1389 bp, Nicotiana tabacum
  source 1..1389: mol_type = genomic DNA
atggagtggaatgcaaagtgggactggggaaacctggtaatgtttggttcagaggtcgccaaaagtccaaaagaactacaattaacagattggggagttgaagaagatggagaacttgatgctggatccttcaatttgtcgagtggtggtagtggtagtggtactggtggttatgtctctgatgttgggtgtggttcttcgatcaagagctcaatatcagcttctactgactcttcaccaaaggagggcttgaaagcatccgacttttctttcgatggctctcctgaggatcttagtaagaaagtgaaaccttgctctagaaattcaccccccatggaggctccagtaggctctgttgaaccacttgtaggtctgaaacttggtaagcggacatttgagaccatcggtggtgctaaggtttcatccttccccgataaacacgtatcatctgctgcagcagcaaagaaaacaaaatcatctactcagaatgcaccaactccacgctgtcaggttgaaggctgcaaccttgatctttcatcagctaaagaatattaccggaagcatcgagtttgtgaaaatcattccaaatgcccaaaggtcattatagcaggtgtattacgccgcttttgtcaacagtgtagcaggttccatagcttgtctgaatttgatgaaaagaagagaagctgccgcaggaggctctctgatcacaatgcacgacgccgcaaaccacagcaggaaaccatccagttcaactcggcaaggctttcttcattgttttatgatagcaggcaacctatgaatcttgtgctcaaccattccaacctggttcagtgtagagctgctgcaaattctacctgggaaagcactgaagaaactaagttcagtataacaagaggattagctccaaagcctgaaagagatggcagtacaaatgggcagtcattattgccagggatccagttttcacgggccgtgggtgcacacggtaatgtatctagctgcttgctcttgccctccaagggccacacagccgaggttttcaatcgaggtgccaaggaatccatgttcaatatgggtacaggaccggaatttcctcgtgctctctctcttctgtcaactaattcatggggttcatccgagcctgagactgtttcactgaaccacccaacacatgcaaatcagagcagcatgcccgagcagatgatgcaggcaattccacaaggtgtgccgcttctgtcctgtgaatactggcagggtgatggacaaccttcatccgatcctcgtgaccatacattggctgctaatagtcatgctggtggtagctttcagggaatcgaactgttcaaacctccatttgacactgatttttatctcaatgcattgaactga

SEQ ID NO: 16 - DNA, 1071 bp, Nicotiana tabacum
  source 1..1071: mol_type = genomic DNA
atgcagttgtgtgcgcatagcattctgctgaagtatgacaatcaagttttaatatacttctttgtctgttactggaatccaacagctctgtttgataaagatccgagtcctacttactttattgcattccatgagtggggaactttacaaaagccatctcgtagcttcttccccaagatggagtggaatgcaaagtgggactggggaaaccagaccatcggtggtgctaagatttcatccttcgccgagaaacccgtatcatctgctgcagcagcaaagaaaacaaaatcatctactcagaatgcaccaactcctcgctgtcaggttgaaggctgcagccttgatctttcatcagctaaagaatattatcggaagcatagagtttgtgacagtcattccaaatgcccaaaggtcactatagcaggtgtagcacgccatttttgtcaacaatgtagcaggttccatagcttgtctgaatttgatgaaaagaagagaagctgtcgcaggaggctctctgatcacaatgcacggcgccgcaaaccacagcaggaaatcatccagctgaactcggcaaggctttcttcattgttttatgatagcaggaaacctatgaatcttacccaactggttcactctagagctgctgcaaattctaccagggaaagcactgaagaaactaatttcagtataacaagagggtctactccaaagcctgaaagagctggcagtacaaatgggcagtcattactgtcggggatccagttttccttggccgtgggtgcacacagtaatgtatctagctgcttgctcttgccctccaagggccacatagacgaggttttcaatcgagatgccaaggaatccatgaccggaatttcctcatggggttcatccgagcctgagactgtttcactgaaccacccaacacatgtaaatcagagcagcatgcctgagcagatgatgcaggcaatcccacaaggtgtgccacttatgtcctgtgaatactggcagagaggacaaccttcatccgatcctcgtgaccatacattggctgctaatagtcatgcaagt

SEQ ID NO: 17 - DNA, 1401 bp, Nicotiana tabacum
  source 1..1401: mol_type = genomic DNA
atgacaatcaaagtgaggaaacaacaagtagctgaaaatgatgtggtggagttaagggatgcgatagatggggagatgcattttgtggccttggattggaagggcttgagctctgattctcttcttcccaagacggagtggaatgcaaagtgggactggggaaacctgataatgtttggttcaaaggccgccaaaagtccaaaagaactacaattaacagattggggaattgaagaagatggagaacttgatgctggatccttcaatttgtcgagtggtggtagtggtagtggtacaggtggttatgtctctgatgtggggcgtggttcttcgatcaagagctcaatatcagcttctactgactcttcaccaaaggagggcttgaaagcatccaacttttctttcgatggctctcctgaggatcttagtaagaaagtgaaaccttggtctagaaattcaccccccatggaggctttggtaggctctgttgaaccacttataggtctgaaacttggtaagcggacatttgagaccatcggtggtgctaagatttcatccttccccgagaaccccgtatcatctgctgctgcagcaaagaaaacaaaatcatctactcaaaatgcgccaactcctcgctgtcaggttgaaggctgcaaccttaatctttcatcagctttgaatattactggaagcatcgagtttgtgacagtcattccaaatgcccaaaggcaacctatgaatcttgttctcaaccacacccaactggttcactctagagctgctgcaaaaagcactgaagaaactaagttcagtataacaagagggtctactccaaagcctgaaagagctggcagtacaaatgggcagtcattactgccggggatccagttttcacgggccgtgggtgcacacagtaatggccacacagccgaggttttcaatcgacgtgccaaggaatccatgctcaaaatgggtacaggaccggaatttcctcgtgctctctctcttctgtcaactaattcatggggttcatccgagcctgagactgtttcactgaaccacccaacacatgcaaatcagagcagcatgcccgagcagatgatgcaggcaattccacaaggtgtgccacttatgtcctgtgaatactggcagggtggacaaccttcatccgatcctcgtgaccatacattggctgctaatagtcatgcttgcgtgattcaaaggagtgaaaatgtaagacagaagatataccttcctgaggagaatggcaacgtcagcttgagagtcttcaatggactggctgccacactctgtacacctgacattgtggctgatatttcttgctcttgcctctaccaccctctccttcttcaccgaatcctcttccccctccatagatag

SEQ ID NO: 18 - DNA, 534 bp, Nicotiana tabacum
  source 1..534: mol_type = genomic DNA
atgccaagagaacgtgaacctctggtagttggtcgagtgataggggatgtattggaccctttcacaagatctattggcctaggagttatttatagggatagagaagttaataatgggtgtgagcttaggccttcccaagttattaaccagcccagggttgaagttggtggagatgaccttcgtaccttttacactctggttatggtggaccctgatgctccaagtccaagtgatccaaatctaagagaatacctccattggttggtcactgatattccagctaccacaggtgcaagttttggccaggaaattgtgtgctatgaaagtccaaggccaacaatgggaatacatcgctttgtattcgtattgtttagacaattgggtcgacagacagtgtatgctccaggatggcgtcagaatttcaatacaaaagattttgctgaactctataatcttggtttaccagttgctgctgtctattttaattgtcaaagagagagtggcagtggtggacgtagaaggtctgccgattga

SEQ ID NO: 19 - DNA, 534 bp, Nicotiana tabacum
  source 1..534: mol_type = genomic DNA
atgccaagagaacgtgaacctctggtagttggtcgagtgataggggatgtattggaccctttcacaagatctattggcctaagagttatttatagggatagagaagttaataatgggtgtgagcttaggccttcccaagttgttaaccagccaagggttgaagttggtggagatgaccttcgtaccttttacactctggttatggtggaccctgatgctccaagtccaagatatccaaatctaagagaatacctccattggttggtcactgatattccagctaccacaggtgcaagttttgggcaagaaattgtgtgctatgaaagtccaaggccaacaatgggaatacatcgctttgtattcgtattgtttagacaattgggtcgacagacagtgtatgctccaggatggcgtcagaatttcaatacaaaagactttgctgaactctataatcttggtttaccggttgctgccgtctattttaattgtcaaagagagagtggcagtggtggacgtagaaggtctgccgattga

SEQ ID NO: 20 - DNA, 544 bp, synthetic construct
  source 1..544: mol_type = other DNA
atggaaacagctggtcatcataatatctctactagtgaggatgattataagaagaagaaaggcagttgtaataataatattacaacaaataataaccatattaagaaagggtcattaaataatggagggtcaagtactaatcaaaggtgttgtcaagctgagaagtgcagtgctgatttaagtgatgctaagcagtaccataggaggcataaagtctgtgaataccatgcaaaggctcaagtcgtcgtcgtcgccggactccggcaacgcttctgtcaacaatgcagccgatttcatgagctgacggaatttgatgaatcaaaaagaagttgccgaaggcgtttggctggacgaaaggcgaagaaagatcagctcttcatcatctgcagcagagtctcaaattgcagaaagttcaagtagaaaagggacagtgcaactcaataataaggacattaacatgatgtgtggtcaagtaaatgaaaagggaagaattcagatttcaatccaagaaaattccactttcaaaaatttccacccccgttga

SEQ ID NO: 21 - DNA, 538 bp, synthetic construct
  source 1..538: mol_type = other DNA
atggaaacagctggtcatcataatatttctactagtgaagatgattataagaagaagagaggcagttgcaataataatattacaacaaataataaccatattaagaaagggtcattaaataatggagggtcaagtactactcaaaggtgttgtcaagctgagaagtgcagtgctgatttaagtgatgctaagcagtaccataggaggcataaagtctgtgaataccatgcaaaggctcaagtcgtcgtcgtcgccggattccggcaacgcttctgtcaacaatgcagccgatttcatgagttgacggaatttgatgaatcgaaaaggagttgccgaaggcgtttggctcgaaaggcgaagaaagagctcatcatcaactgcagagtcacataatattgcagaaagttcaagcagaaaagggacagtgcaactcaataataaggacattaacatgatatgtggtcaagtaaatgacaagggaagaattcagatttcaattcaagaaaattccactttcaaaaacttccacctccgttga

SEQ ID NO: 22 - DNA, 544 bp, synthetic construct
  source 1..544: mol_type = other DNA
atggaaacagctggtcatcataatatttctactagtgaagatgattataagaagaagagaggcagttgcaataataatattacaacaaataataaccatattaagaaagggtcattaaataatggagggtcaagtactactcaaaggtgttgtcaagctgagaagtgcagtgctgatttaagtgatgctaagcagtaccataggaggcataaagtctgtgaataccatgcaaaggctcaagtcgtcgtcgtcgccggattccggcaacgcttctgtcaacaatgcagccgatttcatgagttgacggaatttgatgaatcgaaaaggagttgccgaaggcgtttggctggacaccgaaaggcgaagaaagagctcatcatcaactgcagagtcacataatattgcagaaagttcaagcagaaaagggacagtgcaactcaataataaggacattaacatgatatgtggtcaagtaaatgacaagggaagaattcagatttcaattcaagaaaattccactttcaaaaacttccacctccgttga

SEQ ID NO: 23 - DNA, 517 bp, synthetic construct
  source 1..517: mol_type = other DNA
atggaagcagctgataataatgacttgttcatttttgccactgataatgatgacaagaagaagagaacccccagttataataataggagtagtagtagtagtaataataacaatgaaaagatcaaagggtcaagtacttcaaatgaggtgttgccaagctgataagtgtactgttgatttaagtgatgccaaacaataccataagaggcataaagtctgtgaataccatgcaaaggctcaagccgtcgtcgtcgccggactccggcaacgcttttgtcaacaatgcagccgatttcacgaggtaggagagtttgatgaatcgaaaaggagttgcagaaggcgtttggctgggcacaacgaaaggcgaaggaagactactactacttcttcatcatcagatcagtctaatgctgaagtttcatcgagtagaaaagccataatagggacagacactcatcagataataaacttccaagaaaatgcagcagcaggttataaacactttcagattggatga

SEQ ID NO: 24 - DNA, 501 bp, synthetic construct
  source 1..501: mol_type = other DNA
atggaagcagctgataataatgacttgttcatttttgccactgataatgatgacaagaagaagagaacccccagttataataataggagtagtagtagtagtaataataacaatgaaaagatcaaagggtcaagtacttcaaatgaggtgttgccaagctgataagtgtactgttgatttaagtgatgccaaacaataccataagaggcataaagtctgtgaatagccgtcgtcgtcgccggactccggcaacgcttttgtcaacaatgcagccgatttcacgaggtaggagagtttgatgaatcgaaaaggagttgcagaaggcgtttggctgggcacaacgaaaggcgaaggaagactactactacttcttcatcatcagatcagtctaatgctgaagtttcatcgagtagaaaagccataatagggacagacactcatcagataataaacttccaagaaaatgcagcagcaggttataaacactttcagattggatga

SEQ ID NO: 25 - DNA, 435 bp, synthetic construct
  source 1..435: mol_type = other DNA
atggaaactagcaaatgggaagagaagagaagcatgatggaagaggaggatgacgaggaagacgaagatgttgtagaggacaacaaaaggaagagggtcttgactcgctcgggaaggaaggtacctggcggagagggttcaaagctgccttcctgtcaaattgaggactgcactgcagatatggcaaatgccaagacataccatcgccgccaaaggtctgtgaatttcatgcaaaggctccggcagtacttattggcggactccgacagcgtttctgtcagcaatgcagcaggtttcatcagttgggggagttcgatgaagcaaaaagaagttgcaggagacgtttggcaggccacaacgaacgccgtcgtaaaagttcatgtgattctcctggagaagggtcaagttaaaggggcatcagtccaatggcagtaa

SEQ ID NO: 26 - DNA, 468 bp, synthetic construct
  source 1..468: mol_type = other DNA
atggaaactagcaaatgggaagagaagagaagcatgatggaagaggaggatgacgaggaagacgaagatgttgtagaggacaacaaaaggaagagggtcttgactcgctcgggaaggaaggtacctggcggagagggttcaaagctgccttcctgtcaaattgaggactgcactgcagatatggcaaatgccaagacataccatcgccgccaaaggtctgtgaatttcatgcaaaggctccggcagtacttattggcggactccgacagcgtttctgtcagcaatgcagcaggtttcatcagttgggggagttcgatgaagcaaaaagaagttgcaggagacgtttggcaggccacaacgaacgccgtcgtaaaagttcatgtgattctcctggagaagggtcaagttaaaggggcatcagtctcaatggcagtaaaaccacctacttgtggactgatggaaagataa

SEQ ID NO: 27 - DNA, 468 bp, synthetic construct
  source 1..468: mol_type = other DNA
atggaaactagcaaatgggaagagaagagaagcatgatggaagaggaggatgacgaggaagacgaagatgttgtagaggacaacaaaaggaagagggtcttgactcgctcgggaaggaaggtacctggcggagagggttcaaagctgccttcctgtcaaattgaggactgcactgcagatatggcaaatgccaagacataccatcgccgccaaaggtctgtgaatttcatgcaaaggctccggcagtacttattggcggactccgacagcgtttctgtcagcaatgcagcaggtttcatcagttgggggagttcgatgaagcaaaaagaagttgcaggagacgtttggcaggccacaacgaacgccgtcgtaaaagttcatgtgattctcctggagaagggtcaagttaaaggggcatcagtcacaatggcagtaaaaccacctacttgtggactgatggaaagataa

SEQ ID NO: 28 - DNA, 571 bp, synthetic construct
  source 1..571: mol_type = other DNA
atggaaactagcaaatgggaagagaagagaagcatgacggcagcagaaatggaagaggaggatgacgaggaagacgaagatgttgtggaggacaacaaaaggaagagggtcttgactcactcgggaaggaaggtacctggcggagagggttcaaagctgccttcctgtcaaattgaggactgcactgcagatatggcaaatgccaagacataccatcgccgccacaaggtctgtgaatttcatgcaaaggctccagcagtacttattggtggactccgacagcgtttctgtcagcaatgcagcaggtttcatcagttgggagagttcgatgaagcaaaaaggagttgcaggagacgtttggcaggccacaatgaacgccgtcgtaaaagttcatgtgattctcctggagaagggtcaagttaaaggggcatcagtctcaatggcagagaaatcacctacttgtggactgatggaagataaactcccactgaaaaatataatcacggttttaccatgctcgctctcttctgtcactatccaattttcctttttaacaaaaattatcatgtaa

SEQ ID NO: 29 - DNA, 468 bp, synthetic construct
  source 1..468: mol_type = other DNA
atggaaactagcaaatgggaagagaagagaagcatgacggcagcagaaatggaagaggaggatgacgaggaagacgaagatgttgtggaggacaacaaaaggaagagggtcttgactcactcgggaaggaaggtacctggcggagagggttcaaagctgccttcctgtcaaattgaggactgcactgcagatatggcaaatgccaagacataccatcgccgccaaaggtctgtgaatttcatgcaaaggctccagcagtacttattggtggactccgacagcgtttctgtcagcaatgcagcaggtttcatcagttgggagagttcgatgaagcaaaaaggagttgcaggagacgtttggcaggccacaatgaacgccgtcgtaaaagttcatgtgattctcctggagaagggtcaagttaaaggggcatcagtccaatggcagagaaatcacctacttgtggactga

SEQ ID NO: 30 - DNA, 424 bp, synthetic construct
  source 1..424: mol_type = other DNA
atggaaactagcaaatgggaagagaagagaagcatgacggcagcagaaatggaagaggaggatgacgaggaagacgaagatgttgtggaggacaacaaaaggaagagggtcttgactcactcgggaaggaaggtacctggcggagagggttcaaagctgccttcctgtcaaattgaggactgcactgcagatatggcaaatgccaagacataccatcgccgccaacaaggtctgtgaatttcatgcaaaggctccagcagtacttattggtggactccgacagcgtttctgtcagcaatgcagcaggtttcatcagttgggagagttcgatgaagcaaaaaggagttgcaggagacgtttggcaggccacaatgaacgccgtcgtaaaagttcatgtgattctcctggagaagggtcaagttaa

SEQ ID NO: 31 - DNA, 570 bp, synthetic construct
  source 1..570: mol_type = other DNA
atggaaactagcaaatgggaagagaagagaagcatgacggcagcagaaatggaagaggaggatgacgaggaagacgaagatgttgtggaggacaacaaaaggaagagggtcttgactcactcgggaaggaaggtacctggcggagagggttcaaagctgccttcctgtcaaattgaggactgcactgcagatatggcaaatgccaagacataccatcgccgccaaaggtctgtgaatttcatgcaaaggctccagcagtacttattggtggactccgacagcgtttctgtcagcaatgcagcaggtttcatcagttgggagagttcgatgaagcaaaaaggagttgcaggagacgtttggcaggccacaatgaacgccgtcgtaaaagttcatgtgattctcctggagaagggtcaagttaaaggggcatcagtctcaatggcagagaaatcacctacttgtggactgatggaagataaactcccactgaaaaatataatcacggttttaccatgctcgctctcttctgtcactatccaattttcctttttaacaaaaattatcatgtaa

SEQ ID NO: 32 - DNA, 400 bp, synthetic construct
  source 1..400: mol_type = other DNA
atggaagataacaaatgggaagggaagagaagcatgaatgaagcagaagaggaacatgaaaatgctgaagaggataacaaaaggaagagggtattgactctctctggaaggaatctatctggtggtgggccagcactgccttcttgccaggttgagcagtgcactgcagatatggcaggtgccaagccatatcatcgccgccaaggtgtgcgagtttcattcaaaggctccggtagtacttattagtggaatccagcagcgcttctgtcagcaatgtagcagatttcatcagttgccagagtttgatgaagcaaaaaggagttgccggaggcgtttggcaggtcataatgagcgccgccgtaaaacttcatatgattctcatggagaaagttcaagctga

SEQ ID NO: 33 - DNA, 412 bp, synthetic construct
  source 1..412: mol_type = other DNA
atggaagataacaaatgggaagggaagagaagcatgaatgaagcagaagaggaagaggaggaacatgaaaatgttgaagaggataacaaaaggaagagggtattgactctctccggaaggaagcaatctagtggtgggccagcactcccttcttgccagatcgagcagtgcactgcagatatggcagatgccaagccataccatcgccgccaacaaggtgtgcgagtttcattcaaaggctccggtagtacttattagtggaatccagcaacgcttctgccagcaatgtagcagatttcatcagttagcagagtttgatgaagctaaaaggagttgccggaggcgtttggcaggtcataatgagcgccgccgtaaaacttcatatgattctcatggagaaagttcaagctga

SEQ ID NO: 34 - DNA, 961 bp, synthetic construct
  source 1..961: mol_type = other DNA
atggctatacgcctgaggctaacgggaatagagtggctagcgcttgatcagtttgctcgctgcaatgaagagtactctgtggtttaccttgattggcttggttgttctatctcagtatcagataaagggctaacaatatctttgatcagttgcttctctttgcctggaattaactgttggtactttgcttccaggttccatcggttgccagaatttgaccaagggaaacgcagttgccgcaggcgcctagcaggccataatgagcgtcggaggaaacctccacctggactctcttttgtctaatcgctatggaagtctttcttcatcaatatttgaaaacaatggcagatctggaagttttctggtcgacttcactgcatatccaaatctcactggaggtgcatggccaaatactagatcatctgatcgaggatgggataatcaatccactgcatcagggaagcttctccaaagtcattggctgaacggttctgaaaatcctacatccgaccttgttctgcaaggttcagttgcaaggggtgccaattattctggtcctggtattattccttccggaaattgcttctctggagtctcagattccagtggtgctctctctcttctgtcaaatgagtcatggggctcgaggaaccaatcctctagcctcggggttaacggcttggttaacactgatggcggacataccgttcagccatcgggttcccatgctgctcctgtcaatcactactcaggctctctatggggatttaaaggaaatgaagctagtagcagttcacatgcaatacctcctgatctcgggcttggtcacatttctcaacatgctgtcaatcagtactctgctgagcttgggatggctcagcacagtggaagacagtacatggaactggagcactcaaagggttacgattcttctgttcagaatgtgcactggacactttga

SEQ ID NO: 35 - DNA, 1162 bp, synthetic construct
  source 1..1162: mol_type = other DNA
atgaatgggctcagtaagtcggaaatggaacttctggcttctgcttcttcttctacttctactacttctacttcccctgactctcctcctaacactttaaaatttggtcaaaaaatctactttgaacatgttggacctcaccaccccaaatcagcaactgggtcgtcttcatctccggtcaccggaactccggcgccgacgacgtccaagaaaggaagagggggtggtgtggttcaaggtcgacagccatctaggtgtcaagttgaagggtgtgaagcagatctgagtgatgttaaggcttattattcaaggcacaaagtctgtgctacacattctaagtctcctgtggtcattgttgctggtcttgaacaaagattttgtcaacagtgtagcaggttccatcggttgccagaatttgaccaagggaaacgcagttgccgcaggcgcctagcaggccataatgagcgtcgcaggaaacctccacctggattctcttttgtctaatcgctatggaagtctttcttcatcaatatttgaaaacaatggcagatctggaagttttctggtcgacttcactgcatatccgaatctcactggaggtgcatggccaaatactagatcatctgagcggggatgggataatcaatccactgcatcagggaagcttctccaaagtcattggctgaacagttctgaaaatcctacatccgaccttgttctgcaaggttcagttgctaggggtgccaattattctggtcctggtattattccttccggaaactgcttctctggagtctcagattccagtggtgctctctctcttctgtcaaatgagtcgtggggctcgaggaaccaatcctctagcctcggggttaacgacttggttaacactgatggcggacataccgttcagccatcgggttcccatgctgctcctgtcaatcactactcaggccctcaatggggatttaaaggaaatgaagctagtagcagttcacatgcaatacctcctgatctcgggctgggtcacatttctcaacttgctgtcaatcagtactctgctgagcttgggatggctcagcacagtggaagacagtacatggaactggagcactcaaagggttacgattcttctgttcagaatgtgcactggacactttga

SEQ ID NO: 36 - DNA, 1102 bp, synthetic construct
  source 1..1102: mol_type = other DNA
atgaatgggcagtggaattcggtaatggaactgggttcagtttcttctcctggtagtaattcaagttcctccgactctctcaatggtttgaactttggcaagaaaatctactttgaaaatgtgggtggtgggtcatcgccggtgaccggagccgggaacttgccgccggcgtccaagagggggaggggtgggttgatgcagggtggtcagccacctaaggtgtcaagttgaaggttgtcaggtagatctgagtgatgctaaggcttattattcgaggcataaagtttgtggtatgcactctaagtctcctactgttattgttgctggccttgaacagaggttttgtcaacaatgtagcaggttccatcaattgccagaatttgaccaaggaaaaagaagttgccgcaggcgcctggcatgccataatgagcgccgcaggaagcctccatctggatctcttttctctacacattacgggagcctttcttcatcaatttttgaaaataatagcagcaaatctggaagctttctgttagacttcagctcacacccacatgtcaacgagagttcgtggccaaatactagagcatctgaacaaggatgggatcatcaatctactgcatcagggaagtgtcttcagcgtccttggctgaacaattctgaaaatgctacatctgagttagttctgcaaggttcagccaccaggaccaattatgttccttcaggggaatgtttttctggagtctcagactccagtactggtgctctctctcttctgtcaaatcggtcctggggatcaaggaatccaccctcaagtcttggagctaacattgatgggatacacaccattcaaccttctgattcccatggtgcacctaccaatcacttctcaagcccttcgttacggtttaaaggaaatgaagctagcagcagttcacacgagatgccttctgatttgggtttgggtcaaatttcacaggctgctgacgatcagtactgtggtgagctggggataggtcagcagagtggacgacaaaacatggaactggaccactctaacggttatcatccttctgttcagaatgtgcactggtctctttga

SEQ ID NO: 37 - DNA, 1100 bp, synthetic construct
  source 1..1100: mol_type = other DNA
atgaatgggcagtggaattcggtaatggaactgggttcagtttcttctcctggtagtaattcaagttcctccgactctctcaatggtttgaactttggcaagaaaatctactttgaaaatgtgggtggtgggtcatcgccggtgaccggagccgggaacttgccgccggcgtccaagagggggaggggtgggttgatgcagggtggtcagccaccttgtgtcaagttgaaggttgtcaggtagatctgagtgatgctaaggcttattattcgaggcataaagtttgtggtatgcactctaagtctcctactgttattgttgctggccttgaacagaggttttgtcaacaatgtagcaggttccatcaattgccagaatttgaccaaggaaaaagaagttgccgcaggcgcctggcatgccataatgagcgccgcaggaagcctccatctggatctcttttctctacacattacgggagcctttcttcatcaatttttgaaaataatagcagcaaatctggaagctttctgttagacttcagctcacacccacatgtcaacgagagttcgtggccaaatactagagcatctgaacaaggatgggatcatcaatctactgcatcagggaagtgtcttcagcgtccttggctgaacaattctgaaaatgctacatctgagttagttctgcaaggttcagccaccaggaccaattatgttccttcaggggaatgtttttctggagtctcagactccagtactggtgctctctctcttctgtcaaatcggtcctggggatcaaggaatccaccctcaagtcttggagctaacattgatgggatacacaccattcaaccttctgattcccatggtgcacctaccaatcacttctcaagcccttcgttacggtttaaaggaaatgaagctagcagcagttcacacgagatgccttctgatttgggtttgggtcaaatttcacaggctgctgacgatcagtactgtggtgagctggggataggtcagcagagtggacgacaaaacatggaactggaccactctaacggttatcatccttctgttcagaatgtgcactggtctctttga

SEQ ID NO: 38 - DNA, 1093 bp, synthetic construct
  source 1..1093: mol_type = other DNA
atgaatgggcagtggaattcggtaatggaactgggttcagtttcttctcctggtagtaattcaagttcctccgactctctcaatggtttgaactttggcaagaaaatctactttgagggtggtgggtcatcgccggtgaccggagccgggaacttgccgccggcgtccaagagggggaggggtgggttgatgcagggtggtcagccacctgtgtcaagttgaaggttgtcaggtagatctgagtgatgctaaggcttattattcgaggcataaagtttgtggtatgcactctaagtctcctactgttattgttgctggccttgaacagaggttttgtcaacaatgtagcaggttccatcaattgccagaatttgaccaaggaaaaagaagttgccgcaggcgcctggcatgccataatgagcgccgcaggaagcctccatctggatctcttttctctacacattacgggagcctttcttcatcaatttttgaaaataatagcagcaaatctggaagctttctgttagacttcagctcacacccacatgtcaacgagagttcgtggccaaatactagagcatctgaacaaggatgggatcatcaatctactgcatcagggaagtgtcttcagcgtccttggctgaacaattctgaaaatgctacatctgagttagttctgcaaggttcagccaccaggaccaattatgttccttcaggggaatgtttttctggagtctcagactccagtactggtgctctctctcttctgtcaaatcggtcctggggatcaaggaatccaccctcaagtcttggagctaacattgatgggatacacaccattcaaccttctgattcccatggtgcacctaccaatcacttctcaagcccttcgttacggtttaaaggaaatgaagctagcagcagttcacacgagatgccttctgatttgggtttgggtcaaatttcacaggctgctgacgatcagtactgtggtgagctggggataggtcagcagagtggacgacaaaacatggaactggaccactctaacggttatcatccttctgttcagaatgtgcactggtctctttga

SEQ ID NO: 39 - DNA, 1098 bp, synthetic construct
  source 1..1098: mol_type = other DNA
atgaatgggcagtggaattcggtaatggaactgggttcagtttcttctcctggtagtaattcaagttcctccgactctctcaatggtttgaactttggcaagaaaatctactttgaaaatgggtggtgggtcatcgccggtgaccggagccgggaacttgccgccggcgtccaagagggggaggggtgggttgatgcagggtggtcagccacctagtgtcaagttgaaggttgtcaggtagatctgagtgatgctaaggcttattattcgaggcataaagtttgtggtatgcactctaagtctcctactgttattgttgctggccttgaacagaggttttgtcaacaatgtagcaggttccatcaattgccagaatttgaccaaggaaaaagaagttgccgcaggcgcctggcatgccataatgagcgccgcaggaagcctccatctggatctcttttctctacacattacgggagcctttcttcatcaatttttgaaaataatagcagcaaatctggaagctttctgttagacttcagctcacacccacatgtcaacgagagttcgtggccaaatactagagcatctgaacaaggatgggatcatcaatctactgcatcagggaagtgtcttcagcgtccttggctgaacaattctgaaaatgctacatctgagttagttctgcaaggttcagccaccaggaccaattatgttccttcaggggaatgtttttctggagtctcagactccagtactggtgctctctctcttctgtcaaatcggtcctggggatcaaggaatccaccctcaagtcttggagctaacattgatgggatacacaccattcaaccttctgattcccatggtgcacctaccaatcacttctcaagcccttcgttacggtttaaaggaaatgaagctagcagcagttcacacgagatgccttctgatttgggtttgggtcaaatttcacaggctgctgacgatcagtactgtggtgagctggggataggtcagcagagtggacgacaaaacatggaactggaccactctaacggttatcatccttctgttcagaatgtgcactggtctctttga

SEQ ID NO: 40 - DNA, 1099 bp, synthetic construct
  source 1..1099: mol_type = other DNA
atgaatgggcagtggaattcggtaatggaactgggttcagtttcttctcctggtagtaattcaagttcctccgactctctcaatggtttgaactttggcaagaaaatctactttgaaaatgtgggtggtgggtcatcgccggtgaccggagccgggaacttgccgccggcgtccaagagggggaggggtgggttgatgcagggtggtcagccacctgtgtcaagttgaaggttgtcaggtagatctgagtgatgctaaggcttattattcgaggcataaagtttgtggtatgcactctaagtctcctactgttattgttgctggccttgaacagaggttttgtcaacaatgtagcaggttccatcaattgccagaatttgaccaaggaaaaagaagttgccgcaggcgcctggcatgccataatgagcgccgcaggaagcctccatctggatctcttttctctacacattacgggagcctttcttcatcaatttttgaaaataatagcagcaaatctggaagctttctgttagacttcagctcacacccacatgtcaacgagagttcgtggccaaatactagagcatctgaacaaggatgggatcatcaatctactgcatcagggaagtgtcttcagcgtccttggctgaacaattctgaaaatgctacatctgagttagttctgcaaggttcagccaccaggaccaattatgttccttcaggggaatgtttttctggagtctcagactccagtactggtgctctctctcttctgtcaaatcggtcctggggatcaaggaatccaccctcaagtcttggagctaacattgatgggatacacaccattcaaccttctgattcccatggtgcacctaccaatcacttctcaagcccttcgttacggtttaaaggaaatgaagctagcagcagttcacacgagatgccttctgatttgggtttgggtcaaatttcacaggctgctgacgatcagtactgtggtgagctggggataggtcagcagagtggacgacaaaacatggaactggaccactctaacggttatcatccttctgttcagaatgtgcactggtctctttga

SEQ ID NO: 41 - DNA, 1109 bp, synthetic construct
  source 1..1109: mol_type = other DNA
atgaatgggcagtggaattcggtaatggaactgggttcagtttcttcttctggtagtaattcaagttcttccgactctctcaatggtttgaagtttggcaagaaaatctactttgaaaatgtgggtggtgggtcatcgccggtgaccggagacggaaacttgccgccggcgtccaagagggggaggggtggattggtacagggtggtcagccacctggtgtcaagttgaaggttgtcaggtagatctgagtgatgctaaggcttattattcgaggcataaagtttgtggtatgcactctaagtctcctactgttattgttgctggtcttgaacagaggttttgtcaacaatgtagcaggttccatcaattgacagaatttgaccaaggaaaaagaagttgccgcaggcgcttggcatgccataatgagcgccgcaggaagcctccatctggatctcttttctctacacattacgggagcctttcttcatcaatttttgaaaataatagcagcaaatctggaagctttctgttagacttcagctcacacccacatgtcaacgagagttcgtggccaactagagcatctgaacaaggatgggatcatcaatctactgcatcagggaaatttcttcagcgtccttggctgaataattctgaaaacgctacatctgagtttgttctgcaaggttcagccaccaggaccaattatcccggtcctggtgttccttcaggggaatgtttctctggagtctcagactccagtaccggtgctctctctcttctgtcaaatcggtcctggggatcaacgaatccaccctcaagtcttggggctaacattgatggggtacacacccccattcaaccttccgattcccatgctgcacctaccaatcacttctcaagcccttcactgcagtttaaaggaaatgaagctagcagcagtttgcacgagatgcctgatttgggtttgggtcaaatttcacaggctgctgacaatcagtaccgtggtgagctacggatgggtcatcagagtggacgacaaaacatggaattggaccactctaacggttatcatccttctgttcagaatgtgcactggacgctttga

SEQ ID NO: 42 - DNA, 1111 bp, synthetic construct
  source 1..1111: mol_type = other DNA
atgaatgggcagtggaattcggtaatggaactgggttcagtttcttcttctggtagtaattcaagttcttccgactctctcaatggtttgaagtttggcaagaaaatctactttgaaaatgtgggtggtgggtcatcgccggtgaccggagacggaaacttgccgccggcgtccaagagggggaggggtggattggtacagggtggtcagccacctaaggtgtcaagttgaaggttgtcaggtagatctgagtgatgctaaggcttattattcgaggcataaagtttgtggtatgcactctaagtctcctactgttattgttgctggtcttgaacagaggttttgtcaacaatgtagcaggttccatcaattgacagaatttgaccaaggaaaaagaagttgccgcaggcgcttggcatgccataatgagcgccgcaggaagcctccatctggatctcttttctctacacattacgggagcctttcttcatcaatttttgaaaataatagcagcaaatctggaagctttctgttagacttcagctcacacccacatgtcaacgagagttcgtggccaactagagcatctgaacaaggatgggatcatcaatctactgcatcagggaaatttcttcagcgtccttggctgaataattctgaaaacgctacatctgagtttgttctgcaaggttcagccaccaggaccaattatcccggtcctggtgttccttcaggggaatgtttctctggagtctcagactccagtaccggtgctctctctcttctgtcaaatcggtcctggggatcaacgaatccaccctcaagtcttggggctaacattgatggggtacacacccccattcaaccttccgattcccatgctgcacctaccaatcacttctcaagcccttcactgcagtttaaaggaaatgaagctagcagcagtttgcacgagatgcctgatttgggtttgggtcaaatttcacaggctgctgacaatcagtaccgtggtgagctacggatgggtcatcagagtggacgacaaaacatggaattggaccactctaacggttatcatccttctgttcagaatgtgcactggacgctttga

SEQ ID NO: 43 - DNA, 1108 bp, synthetic construct
  source 1..1108: mol_type = other DNA
atgaatgggcagtggaattcggtaatggaactgggttcagtttcttcttctggtagtaattcaagttcttccgactctctcaatggtttgaagtttggcaagaaaatctactttgaaaatgtgggtggtgggtcatcgccggtgaccggagacggaaacttgccgccggcgtccaagagggggaggggtggattggtacagggtggtcagccacctgtgtcaagttgaaggttgtcaggtagatctgagtgatgctaaggcttattattcgaggcataaagtttgtggtatgcactctaagtctcctactgttattgttgctggtcttgaacagaggttttgtcaacaatgtagcaggttccatcaattgacagaatttgaccaaggaaaaagaagttgccgcaggcgcttggcatgccataatgagcgccgcaggaagcctccatctggatctcttttctctacacattacgggagcctttcttcatcaatttttgaaaataatagcagcaaatctggaagctttctgttagacttcagctcacacccacatgtcaacgagagttcgtggccaactagagcatctgaacaaggatgggatcatcaatctactgcatcagggaaatttcttcagcgtccttggctgaataattctgaaaacgctacatctgagtttgttctgcaaggttcagccaccaggaccaattatcccggtcctggtgttccttcaggggaatgtttctctggagtctcagactccagtaccggtgctctctctcttctgtcaaatcggtcctggggatcaacgaatccaccctcaagtcttggggctaacattgatggggtacacacccccattcaaccttccgattcccatgctgcacctaccaatcacttctcaagcccttcactgcagtttaaaggaaatgaagctagcagcagtttgcacgagatgcctgatttgggtttgggtcaaatttcacaggctgctgacaatcagtaccgtggtgagctacggatgggtcatcagagtggacgacaaaacatggaattggaccactctaacggttatcatccttctgttcagaatgtgcactggacgctttga

SEQ ID NO: 44 - DNA, 976 bp, synthetic construct
  source 1..976: mol_type = other DNA
atggaatcatcatcctcatcctcatcctcgtctaagagggcaaaagcacctggcaatattgctcaagtagctcattgcttggttgatggatgtaatgcagaccttagccaatgcagagagtatcaccgccgccataaagtttgtgaggtccattcaaagactgccaaatgtttatctcgatctgatggttccttttgtaggtttcattccttggtagaatttgatgatggaaagagaagctgtcggaaacgtttggatggacataacaggcgtacgaaggaaacctcagccagattctatggccaaaacttctggattactttttactggccagcaagggacgaaacttctgtcatttagcagtcaacaaatttttccaagtgcagctgcatgggctggcgtagtcaaaacggacagcgaaatggtattatacaacaaccaatcgcatataaattgcatggacaatcaaaactcgttccctgattcttcagctcgtagctacaaaggaggaaatcaattccagttcatgcaaggcagtgaccgtagtctccctgaagcttcaatctaccagccacttgttgatcatcccaattctgcagtagcagcagcagttcctagcagcggacaaaagatcttctccagtggattgaacgaaattgtggactctgatcgtgctctctctcttctgtcatcagcacccgctgtaactagggagattggttttagtcacatggtgcagcagcctgccactatcccccggccccagtcacaatctgtcgttcatagcctgcactatggtggtctaagccagtacccttttgctcaagatttcaatagccaacctcaagattctgctgcagattcacatgttagcaacaacagctctctgcatttccatgatatgttacaaaatggagcagatggatcatctacaagtggtggctgtcagcaaacactagcctttatgtgggactaa

SEQ ID NO: 45 - DNA, 976 bp, synthetic construct
  source 1..976: mol_type = other DNA
atggaatcatcatcctcatcctcatcctcgtctaagagggcaaaagcacctggcaatattgctcaagtagctcattgcttggttgatggatgtaatgcagaccttagccaatgcagagagtatcaccgccgccataaagtttgtgaggtccattcaaagactgccaaatgtttatctcgatctgatggttccttttgtaggtttcattccttggtagaatttgatgatggaaagagaagctgtcggaaacgtttggatggacataacaggcgttcgaaggaaacctcagccagattctatggccaaaacttctggattactttttactggccagcaagggacgaaacttctgtcatttagcagtcaacaaatttttccaagtgcagctgcatgggctggcgtagtcaaaacggacagcgaaatggtattatacaacaaccaatcgcatataaattgcatggacaatcaaaactcgttccctgattcttcagctcgtagctacaaaggaggaaatcaattccagttcatgcaaggcagtgaccgtagtctccctgaagcttcaatctaccagccacttgttgatcatcccaattctgcagtagcagcagcagttcctagcagcggacaaaagatcttctccagtggattgaacgaaattgtggactctgatcgtgctctctctcttctgtcatcagcacccgctgtaactagggagattggttttagtcacatggtgcagcagcctgccactatcccccggccccagtcacaatctgtcgttcatagcctgcactatggtggtctaagccagtacccttttgctcaagatttcaatagccaacctcaagattctgctgcagattcacatgttagcaacaacagctctctgcatttccatgatatgttacaaaatggagcagatggatcatctacaagtggtggctgtcagcaaacactagcctttatgtgggactaa

SEQ ID NO: 46 - DNA, 974 bp, synthetic construct
  source 1..974: mol_type = other DNA
atggaatcatcatcctcatcctcatcctcgtctaagagggcaaaagcacctggcaatattgctcaagtagctcattgcttggttgatggatgtaatgcagaccttagccaatgcagagagtatcaccgccgccataaagtttgtgaggtccattcaaagactgccaaatgtttatctcgatctgatggttccttttgtaggtttcattccttggtagaatttgatgatggaaagagaagctgtcggaaacgtttggatggacataacaggctcgaaggaaacctcagccagattctatggccaaaacttctggattactttttactggccagcaagggacgaaacttctgtcatttagcagtcaacaaatttttccaagtgcagctgcatgggctggcgtagtcaaaacggacagcgaaatggtattatacaacaaccaatcgcatataaattgcatggacaatcaaaactcgttccctgattcttcagctcgtagctacaaaggaggaaatcaattccagttcatgcaaggcagtgaccgtagtctccctgaagcttcaatctaccagccacttgttgatcatcccaattctgcagtagcagcagcagttcctagcagcggacaaaagatcttctccagtggattgaacgaaattgtggactctgatcgtgctctctctcttctgtcatcagcacccgctgtaactagggagattggttttagtcacatggtgcagcagcctgccactatcccccggccccagtcacaatctgtcgttcatagcctgcactatggtggtctaagccagtacccttttgctcaagatttcaatagccaacctcaagattctgctgcagattcacatgttagcaacaacagctctctgcatttccatgatatgttacaaaatggagcagatggatcatctacaagtggtggctgtcagcaaacactagcctttatgtgggactaa

SEQ ID NO: 47 - DNA, 971 bp, synthetic construct
  source 1..971: mol_type = other DNA
atggaatcatcatcctcatcctcatcctcgtctaagagggcaaaagcacctggcaatattgctcaagtagctcattgcttggttgatggatgtaatgcagaccttagccaatgcagagagtatcaccgccgccataaagtttgtgaggtccattcaaagactgccaaatgtttatctcgatctgatggttccttttgtaggtttcattccttggtagaatttgatgatggaaagagaagctgtcggaaacgtttggatggacataacatcgaaggaaacctcagccagattctatggccaaaacttctggattactttttactggccagcaagggacgaaacttctgtcatttagcagtcaacaaatttttccaagtgcagctgcatgggctggcgtagtcaaaacggacagcgaaatggtattatacaacaaccaatcgcatataaattgcatggacaatcaaaactcgttccctgattcttcagctcgtagctacaaaggaggaaatcaattccagttcatgcaaggcagtgaccgtagtctccctgaagcttcaatctaccagccacttgttgatcatcccaattctgcagtagcagcagcagttcctagcagcggacaaaagatcttctccagtggattgaacgaaattgtggactctgatcgtgctctctctcttctgtcatcagcacccgctgtaactagggagattggttttagtcacatggtgcagcagcctgccactatcccccggccccagtcacaatctgtcgttcatagcctgcactatggtggtctaagccagtacccttttgctcaagatttcaatagccaacctcaagattctgctgcagattcacatgttagcaacaacagctctctgcatttccatgatatgttacaaaatggagcagatggatcatctacaagtggtggctgtcagcaaacactagcctttatgtgggactaa

SEQ ID NO: 48 - DNA, 974 bp, synthetic construct
  source 1..974: mol_type = other DNA
atggaatcatcatcctcatcctcatcctcgtctaagagggcaaaagcacctggcaatattgctcaagtagctcattgcttggttgatggatgtaatgcagaccttagccaatgcagagagtatcaccgccgccaaagtttgtgaggtccattcaaagactgccaaatgtttatctcgatctgatggttccttttgtaggtttcattccttggtagaatttgatgatggaaagagaagctgtcggaaacgtttggatggacataacaggcgtacgaaggaaacctcagccagattctatggccaaaacttctggattactttttactggccagcaagggacgaaacttctgtcatttagcagtcaacaaatttttccaagtgcagctgcatgggctggcgtagtcaaaacggacagcgaaatggtattatacaacaaccaatcgcatataaattgcatggacaatcaaaactcgttccctgattcttcagctcgtagctacaaaggaggaaatcaattccagttcatgcaaggcagtgaccgtagtctccctgaagcttcaatctaccagccacttgttgatcatcccaattctgcagtagcagcagcagttcctagcagcggacaaaagatcttctccagtggattgaacgaaattgtggactctgatcgtgctctctctcttctgtcatcagcacccgctgtaactagggagattggttttagtcacatggtgcagcagcctgccactatcccccggccccagtcacaatctgtcgttcatagcctgcactatggtggtctaagccagtacccttttgctcaagatttcaatagccaacctcaagattctgctgcagattcacatgttagcaacaacagctctctgcatttccatgatatgttacaaaatggagcagatggatcatctacaagtggtggctgtcagcaaacactagcctttatgtgggactaa

SEQ ID NO: 49 - DNA, 970 bp, synthetic construct
  source 1..970: mol_type = other DNA
atggaatcatcatcctcatcctcatcctcgtctaagagggcaaaagcacctggcaatattgctcaagtagctcattgcttggttgatggatgtaatgcagaccttagccaatgcagagagtatcaccgccgccattgtgaggtccattcaaagactgccaaatgtttatctcgatctgatggttccttttgtaggtttcattccttggtagaatttgatgatggaaagagaagctgtcggaaacgtttggatggacataacaggcgtacgaaggaaacctcagccagattctatggccaaaacttctggattactttttactggccagcaagggacgaaacttctgtcatttagcagtcaacaaatttttccaagtgcagctgcatgggctggcgtagtcaaaacggacagcgaaatggtattatacaacaaccaatcgcatataaattgcatggacaatcaaaactcgttccctgattcttcagctcgtagctacaaaggaggaaatcaattccagttcatgcaaggcagtgaccgtagtctccctgaagcttcaatctaccagccacttgttgatcatcccaattctgcagtagcagcagcagttcctagcagcggacaaaagatcttctccagtggattgaacgaaattgtggactctgatcgtgctctctctcttctgtcatcagcacccgctgtaactagggagattggttttagtcacatggtgcagcagcctgccactatcccccggccccagtcacaatctgtcgttcatagcctgcactatggtggtctaagccagtacccttttgctcaagatttcaatagccaacctcaagattctgctgcagattcacatgttagcaacaacagctctctgcatttccatgatatgttacaaaatggagcagatggatcatctacaagtggtggctgtcagcaaacactagcctttatgtgggactaa

SEQ ID NO: 50 - DNA, 974 bp, synthetic construct
  source 1..974: mol_type = other DNA
atggaatcatcatcctcatcctcatcctcgtctaagagggcaaaagcacctggcaatattgctcaagtagctcattgcttggttgatggatgtaatgcagaccttagccaatgcagagagtatcaccgccgccataaagtttgtgaggtccattcaaagactgccaaatgtttatctcgatctgatggttccttttgtaggtttcattccttggtagaatttgatgatggaaagagaagctgtcggaaacgtttggatggacataacaggcgcgaaggaaacctcagccagattctatggccaaaacttctggattactttttactggccagcaagggacgaaacttctgtcatttagcagtcaacaaatttttccaagtgcagctgcatgggctggcgtagtcaaaacggacagcgaaatggtattatacaacaaccaatcgcatataaattgcatggacaatcaaaactcgttccctgattcttcagctcgtagctacaaaggaggaaatcaattccagttcatgcaaggcagtgaccgtagtctccctgaagcttcaatctaccagccacttgttgatcatcccaattctgcagtagcagcagcagttcctagcagcggacaaaagatcttctccagtggattgaacgaaattgtggactctgatcgtgctctctctcttctgtcatcagcacccgctgtaactagggagattggttttagtcacatggtgcagcagcctgccactatcccccggccccagtcacaatctgtcgttcatagcctgcactatggtggtctaagccagtacccttttgctcaagatttcaatagccaacctcaagattctgctgcagattcacatgttagcaacaacagctctctgcatttccatgatatgttacaaaatggagcagatggatcatctacaagtggtggctgtcagcaaacactagcctttatgtgggactaa

SEQ ID NO: 51 - DNA, 982 bp, synthetic construct
  source 1..982: mol_type = other DNA
atggaatcatcctcctcatctaagagggcaaaagcacctggcaatattgctcaagtagctcattgcttggttgatggatgtaatgcagacctcagccaatgcagagagtatcaccgccgccataaagtttgtgaggtccattcaaagactgccaaagtcacgattgggggtcgagaccaacgtttctgtcagcaatgcagcaggtttcattccttggtagaatttgatgatggtaagagaagctgtcggaaacgtctggatggacataacaggcgttcgaaggaaacctcagcctgattctatggccaaaacttctggattactttttactggccagcaagggacgaaagttctgtcatttagcagtcaacaaatttttccaagtgcagttgtgagctctgcatgggctggcgtagtcaaaacggacagcgacatggtattatacaacaatataaattgcatggacaatcaaaactcgttccctgattcttcggctcgtagtagctacaaaggaggaaatcaattccagttcatgcaaggcagtgagcgtagtctccctgaagcttcaatctgccagccacttgttgatcatcccaattctacagcagcagttcctagcagcggacaaaagatcttctccagtggattgaacgaaattgtggactctgatcgtgctctctctcttctgtcatcagcacccgctgtaactagggagattggttttagtcacatggtgcagcagcctgcctctatcccccggccccggccccagtcacaatctgtcgtacatagcctgcactatggtggtctaagccagtacccttttgctcaggatttcaatagccaacctcaagattctgctgcagattcacatgttagcaacagcagctctctgcatttccatgatatgttacaaaatgcaccagatggatcatctacaagtggtggctgtcagcaaacactagcctttatgtgggactaa

SEQ ID NO: 52 - DNA, 982 bp, synthetic construct
  source 1..982: mol_type = other DNA
atggaatcatcctcctcatctaagagggcaaaagcacctggcaatattgctcaagtagctcattgcttggttgatggatgtaatgcagacctcagccaatgcagagagtatcaccgccgccataaagtttgtgaggtccattcaaagactgccaaagtcacgattgggggtcgagaccaacgtttctgtcagcaatgcagcaggtttcattccttggtagaatttgatgatggtaagagaagctgtcggaaacgtctggatggacataacaggcgtccgaaggaaacctcagcctgattctatggccaaaacttctggattactttttactggccagcaagggacgaaagttctgtcatttagcagtcaacaaatttttccaagtgcagttgtgagctctgcatgggctggcgtagtcaaaacggacagcgacatggtattatacaacaatataaattgcatggacaatcaaaactcgttccctgattcttcggctcgtagtagctacaaaggaggaaatcaattccagttcatgcaaggcagtgagcgtagtctccctgaagcttcaatctgccagccacttgttgatcatcccaattctacagcagcagttcctagcagcggacaaaagatcttctccagtggattgaacgaaattgtggactctgatcgtgctctctctcttctgtcatcagcacccgctgtaactagggagattggttttagtcacatggtgcagcagcctgcctctatcccccggccccggccccagtcacaatctgtcgtacatagcctgcactatggtggtctaagccagtacccttttgctcaggatttcaatagccaacctcaagattctgctgcagattcacatgttagcaacagcagctctctgcatttccatgatatgttacaaaatgcaccagatggatcatctacaagtggtggctgtcagcaaacactagcctttatgtgggactaa

SEQ ID NO: 53 - DNA, 982 bp, synthetic construct
  source 1..982: mol_type = other DNA
atggaatcatcctcctcatctaagagggcaaaagcacctggcaatattgctcaagtagctcattgcttggttgatggatgtaatgcagacctcagccaatgcagagagtatcaccgccgccataaagtttgtgaggtccattcaaagactgccaaagtcacgattgggggtcgagaccaacgtttctgtcagcaatgcagcaggtttcattccttggtagaatttgatgatggtaagagaagctgtcggaaacgtctggatggacataacaggcgtacgaaggaaacctcagcctgattctatggccaaaacttctggattactttttactggccagcaagggacgaaagttctgtcatttagcagtcaacaaatttttccaagtgcagttgtgagctctgcatgggctggcgtagtcaaaacggacagcgacatggtattatacaacaatataaattgcatggacaatcaaaactcgttccctgattcttcggctcgtagtagctacaaaggaggaaatcaattccagttcatgcaaggcagtgagcgtagtctccctgaagcttcaatctgccagccacttgttgatcatcccaattctacagcagcagttcctagcagcggacaaaagatcttctccagtggattgaacgaaattgtggactctgatcgtgctctctctcttctgtcatcagcacccgctgtaactagggagattggttttagtcacatggtgcagcagcctgcctctatcccccggccccggccccagtcacaatctgtcgtacatagcctgcactatggtggtctaagccagtacccttttgctcaggatttcaatagccaacctcaagattctgctgcagattcacatgttagcaacagcagctctctgcatttccatgatatgttacaaaatgcaccagatggatcatctacaagtggtggctgtcagcaaacactagcctttatgtgggactaa

SEQ ID NO: 54 - DNA, 983 bp, synthetic construct
  source 1..983: mol_type = other DNA
atggaatcatcctcctcatctaagagggcaaaagcacctggcaatattgctcaagtagctcattgcttggttgatggatgtaatgcagacctcagccaatgcagagagtatcaccgccgccattaaagtttgtgaggtccattcaaagactgccaaagtcacgattgggggtcgagaccaacgtttctgtcagcaatgcagcaggtttcattccttggtagaatttgatgatggtaagagaagctgtcggaaacgtctggatggacataacaggcgtgcgaaggaaacctcagcctgattctatggccaaaacttctggattactttttactggccagcaagggacgaaagttctgtcatttagcagtcaacaaatttttccaagtgcagttgtgagctctgcatgggctggcgtagtcaaaacggacagcgacatggtattatacaacaatataaattgcatggacaatcaaaactcgttccctgattcttcggctcgtagtagctacaaaggaggaaatcaattccagttcatgcaaggcagtgagcgtagtctccctgaagcttcaatctgccagccacttgttgatcatcccaattctacagcagcagttcctagcagcggacaaaagatcttctccagtggattgaacgaaattgtggactctgatcgtgctctctctcttctgtcatcagcacccgctgtaactagggagattggttttagtcacatggtgcagcagcctgcctctatcccccggccccggccccagtcacaatctgtcgtacatagcctgcactatggtggtctaagccagtacccttttgctcaggatttcaatagccaacctcaagattctgctgcagattcacatgttagcaacagcagctctctgcatttccatgatatgttacaaaatgcaccagatggatcatctacaagtggtggctgtcagcaaacactagcctttatgtgggactaa

SEQ ID NO: 55 - DNA, 983 bp, synthetic construct
  source 1..983: mol_type = other DNA
atggaatcatcctcctcatctaagagggcaaaagcacctggcaatattgctcaagtagctcattgcttggttgatggatgtaatgcagacctcagccaatgcagagagtatcaccgccgccattaaagtttgtgaggtccattcaaagactgccaaagtcacgattgggggtcgagaccaacgtttctgtcagcaatgcagcaggtttcattccttggtagaatttgatgatggtaagagaagctgtcggaaacgtctggatggacataacaggcgtacgaaggaaacctcagcctgattctatggccaaaacttctggattactttttactggccagcaagggacgaaagttctgtcatttagcagtcaacaaatttttccaagtgcagttgtgagctctgcatgggctggcgtagtcaaaacggacagcgacatggtattatacaacaatataaattgcatggacaatcaaaactcgttccctgattcttcggctcgtagtagctacaaaggaggaaatcaattccagttcatgcaaggcagtgagcgtagtctccctgaagcttcaatctgccagccacttgttgatcatcccaattctacagcagcagttcctagcagcggacaaaagatcttctccagtggattgaacgaaattgtggactctgatcgtgctctctctcttctgtcatcagcacccgctgtaactagggagattggttttagtcacatggtgcagcagcctgcctctatcccccggccccggccccagtcacaatctgtcgtacatagcctgcactatggtggtctaagccagtacccttttgctcaggatttcaatagccaacctcaagattctgctgcagattcacatgttagcaacagcagctctctgcatttccatgatatgttacaaaatgcaccagatggatcatctacaagtggtggctgtcagcaaacactagcctttatgtgggactaa

SEQ ID NO: 56 - DNA, 982 bp, synthetic construct
  source 1..982: mol_type = other DNA
atggaatcatcctcctcatctaagagggcaaaagcacctggcaatattgctcaagtagctcattgcttggttgatggatgtaatgcagacctcagccaatgcagagagtatcaccgccgccataaagtttgtgaggtccattcaaagactgccaaagtcacgattgggggtcgagaccaacgtttctgtcagcaatgcagcaggtttcattccttggtagaatttgatgatggtaagagaagctgtcggaaacgtctggatggacataacaggcgtgcgaaggaaacctcagcctgattctatggccaaaacttctggattactttttactggccagcaagggacgaaagttctgtcatttagcagtcaacaaatttttccaagtgcagttgtgagctctgcatgggctggcgtagtcaaaacggacagcgacatggtattatacaacaatataaattgcatggacaatcaaaactcgttccctgattcttcggctcgtagtagctacaaaggaggaaatcaattccagttcatgcaaggcagtgagcgtagtctccctgaagcttcaatctgccagccacttgttgatcatcccaattctacagcagcagttcctagcagcggacaaaagatcttctccagtggattgaacgaaattgtggactctgatcgtgctctctctcttctgtcatcagcacccgctgtaactagggagattggttttagtcacatggtgcagcagcctgcctctatcccccggccccggccccagtcacaatctgtcgtacatagcctgcactatggtggtctaagccagtacccttttgctcaggatttcaatagccaacctcaagattctgctgcagattcacatgttagcaacagcagctctctgcatttccatgatatgttacaaaatgcaccagatggatcatctacaagtggtggctgtcagcaaacactagcctttatgtgggactaa

SEQ ID NO: 57 - DNA, 975 bp, synthetic construct
  source 1..975: mol_type = other DNA
atggaatcatcctcctcatctaagagggcaaaagcacctggcaatattgctcaagtagctcattgcttggttgatggatgtaatgcagacctcagccaatgcagagagtatcaccgccgccaaaagtttgtgaggtccattcaaagactgccaaagtcacgattgggggtcgagaccaacgtttctgtcagcaatgcagcaggtttcattccttggtagaatttgatgatggtaagagaagctgtcggaaacgtctggatggacataacaggcaggaaacctcagcctgattctatggccaaaacttctggattactttttactggccagcaagggacgaaagttctgtcatttagcagtcaacaaatttttccaagtgcagttgtgagctctgcatgggctggcgtagtcaaaacggacagcgacatggtattatacaacaatataaattgcatggacaatcaaaactcgttccctgattcttcggctcgtagtagctacaaaggaggaaatcaattccagttcatgcaaggcagtgagcgtagtctccctgaagcttcaatctgccagccacttgttgatcatcccaattctacagcagcagttcctagcagcggacaaaagatcttctccagtggattgaacgaaattgtggactctgatcgtgctctctctcttctgtcatcagcacccgctgtaactagggagattggttttagtcacatggtgcagcagcctgcctctatcccccggccccggccccagtcacaatctgtcgtacatagcctgcactatggtggtctaagccagtacccttttgctcaggatttcaatagccaacctcaagattctgctgcagattcacatgttagcaacagcagctctctgcatttccatgatatgttacaaaatgcaccagatggatcatctacaagtggtggctgtcagcaaacactagcctttatgtgggactaa

SEQ ID NO: 58 - DNA, 980 bp, synthetic construct
  source 1..980: mol_type = other DNA
atggaatcatcctcctcatctaagagggcaaaagcacctggcaatattgctcaagtagctcattgcttggttgatggatgtaatgcagacctcagccaatgcagagagtatcaccgccgccaaaagtttgtgaggtccattcaaagactgccaaagtcacgattgggggtcgagaccaacgtttctgtcagcaatgcagcaggtttcattccttggtagaatttgatgatggtaagagaagctgtcggaaacgtctggatggacataacaggcgtcgaaggaaacctcagcctgattctatggccaaaacttctggattactttttactggccagcaagggacgaaagttctgtcatttagcagtcaacaaatttttccaagtgcagttgtgagctctgcatgggctggcgtagtcaaaacggacagcgacatggtattatacaacaatataaattgcatggacaatcaaaactcgttccctgattcttcggctcgtagtagctacaaaggaggaaatcaattccagttcatgcaaggcagtgagcgtagtctccctgaagcttcaatctgccagccacttgttgatcatcccaattctacagcagcagttcctagcagcggacaaaagatcttctccagtggattgaacgaaattgtggactctgatcgtgctctctctcttctgtcatcagcacccgctgtaactagggagattggttttagtcacatggtgcagcagcctgcctctatcccccggccccggccccagtcacaatctgtcgtacatagcctgcactatggtggtctaagccagtacccttttgctcaggatttcaatagccaacctcaagattctgctgcagattcacatgttagcaacagcagctctctgcatttccatgatatgttacaaaatgcaccagatggatcatctacaagtggtggctgtcagcaaacactagcctttatgtgggactaa

SEQ ID NO: 59 - DNA, 976 bp, synthetic construct
  source 1..976: mol_type = other DNA
atggaatcatcctcctcatctaagagggcaaaagcacctggcaatattgctcaagtagctcattgcttggttgatggatgtaatgcagacctcagccaatgcagagagtatcaccgccgccataaagtttgtgaggtccattcaaagactgccaaagtcacgattgggggtcgagaccaacgtttctgtcagcaatgcagcaggtttcattccttggtagaatttgatgatggtaagagaagctgtcggaaacgtctggatggacataacaggcaggaaacctcagcctgattctatggccaaaacttctggattactttttactggccagcaagggacgaaagttctgtcatttagcagtcaacaaatttttccaagtgcagttgtgagctctgcatgggctggcgtagtcaaaacggacagcgacatggtattatacaacaatataaattgcatggacaatcaaaactcgttccctgattcttcggctcgtagtagctacaaaggaggaaatcaattccagttcatgcaaggcagtgagcgtagtctccctgaagcttcaatctgccagccacttgttgatcatcccaattctacagcagcagttcctagcagcggacaaaagatcttctccagtggattgaacgaaattgtggactctgatcgtgctctctctcttctgtcatcagcacccgctgtaactagggagattggttttagtcacatggtgcagcagcctgcctctatcccccggccccggccccagtcacaatctgtcgtacatagcctgcactatggtggtctaagccagtacccttttgctcaggatttcaatagccaacctcaagattctgctgcagattcacatgttagcaacagcagctctctgcatttccatgatatgttacaaaatgcaccagatggatcatctacaagtggtggctgtcagcaaacactagcctttatgtgggactaa

SEQ ID NO: 60 - DNA, 1389 bp, synthetic construct
  source 1..1389: mol_type = other DNA
atggagtggaatgcaaagtgggactggggaaacctggtaatgtttggttcagaggccgccaaaagtccaaaagaactacaattaacagattggggagttgaagaagatggagaacttgatgctggatccttcaatttgtcaagtggtggtagtggtagtggtagtggtaccggtggttatgtctctgatgttgggcatggttcttcgatcaagagctcaatatcagcttctactgactcttcacccaaggagggcttgaaagcatgcaacttttctttcgatggctcttctgaggatcttagtaagaaagtgaaactttgctctagaaattcaccccccatggaggcttcagtaggctctgttgaaccacttataggtctgaaacttggtaagcggacatttgagaccatcggcggtgctaaggtttcatccttccccgagaaacacgtatcatctgctgcagcagcaaagaaaacaaaatcatctactcagaatgcaccaactcctcgctgtcaggttgaaggctgcagccatgatctttcatcagctaaagaatattaccggaagcatcgagtttgtgacagtcattccaaatgcccaaaggtcattatagcaggtgtagcacgtcgcttttgtcaacagtgtagcaggttccatagcttgtctgaatttgatgaaaagaagagaagctgtcgcaggaggctctctgatcacaatgcacggcgccgcaaaccacagcaggaaaccatccagaactcggcaaggctttcttcattgttttatgatagcaggcaacctatgaatcttgtgctcaaccattcccaactggttcagtctagagctgctgcaaattctacctgggaaagcactgaagaaactaagttcagtataacaagagggtctactccaaagcctgaaagagctggcagtacaaatgggctgtcattattgccagggatccagttgtcacgggccgtgggtgcacacagtaatgtatctagctgcttgctcttgccctccaagggccacacatccgaggttttcaatcgaggtgccacggaatccatgttcaatatgggtacaggacgggaatttcctcgtgctctctctcttctgtcaactaattcatggggttcatccgagcctgagactgtttcactgaacaacccaacacacgcgaatcagagcagcatgcccgagcagatgatgcaggcaattccacaaggtgtgccacttatgtcctgtgaatactggcagggtgaacaaccctcatccgatcctcgtgaccatacattggctgctaatagtcatgctggtggtagctttcagggaatcgagctgttcaaacctccatttgacactgacttttatctcaatgcattgaactga

SEQ ID NO: 61 - DNA, 1390 bp, synthetic construct
  source 1..1390: mol_type = other DNA
atggagtggaatgcaaagtgggactggggaaacctggtaatgtttggttcagaggccgccaaaagtccaaaagaactacaattaacagattggggagttgaagaagatggagaacttgatgctggatccttcaatttgtcaagtggtggtagtggtagtggtagtggtaccggtggttatgtctctgatgttgggcatggttcttcgatcaagagctcaatatcagcttctactgactcttcacccaaggagggcttgaaagcatgcaacttttctttcgatggctcttctgaggatcttagtaagaaagtgaaactttgctctagaaattcaccccccatggaggcttcagtaggctctgttgaaccacttataggtctgaaacttggtaagcggacatttgagaccatcggcggtgctaaggtttcatccttccccgagaaacacgtatcatctgctgcagcagcaaagaaaacaaaatcatctactcagaatgcaccaactcctcgctgtcaggttgaaggctgcagccatgatctttcatcagctaaagaatattaccggaagcatcgagtttgtgacagtcattccaaatgcccaaaggtcattatagcaggtgtagcacgtcgcttttgtcaacagtgtagcaggttccatagcttgtctgaatttgatgaaaagaagagaagctgtcgcaggaggctctctgatcacaatgcacggcgccgcaaaccacagcaggaaaccatccagttactcggcaaggctttcttcattgttttatgatagcaggcaacctatgaatcttgtgctcaaccattcccaactggttcagtctagagctgctgcaaattctacctgggaaagcactgaagaaactaagttcagtataacaagagggtctactccaaagcctgaaagagctggcagtacaaatgggctgtcattattgccagggatccagttgtcacgggccgtgggtgcacacagtaatgtatctagctgcttgctcttgccctccaagggccacacatccgaggttttcaatcgaggtgccacggaatccatgttcaatatgggtacaggacgggaatttcctcgtgctctctctcttctgtcaactaattcatggggttcatccgagcctgagactgtttcactgaacaacccaacacacgcgaatcagagcagcatgcccgagcagatgatgcaggcaattccacaaggtgtgccacttatgtcctgtgaatactggcagggtgaacaaccctcatccgatcctcgtgaccatacattggctgctaatagtcatgctggtggtagctttcagggaatcgagctgttcaaacctccatttgacactgacttttatctcaatgcattgaactga

SEQ ID NO: 62 - DNA, 1388 bp, synthetic construct
  source 1..1388: mol_type = other DNA
atggagtggaataagtgggactggggaaacctggtaatgtttggttcagaggccgccaaaagtccaaaagaactacaattaacagattggggagttgaagaagatggagaacttgatgctggatccttcaatttgtcaagtggtggtagtggtagtggtagtggtaccggtggttatgtctctgatgttgggcatggttcttcgatcaagagctcaatatcagcttctactgactcttcacccaaggagggcttgaaagcatgcaacttttctttcgatggctcttctgaggatcttagtaagaaagtgaaactttgctctagaaattcaccccccatggaggcttcagtaggctctgttgaaccacttataggtctgaaacttggtaagcggacatttgagaccatcggcggtgctaaggtttcatccttccccgagaaacacgtatcatctgctgcagcagcaaagaaaacaaaatcatctactcagaatgcaccaactcctcgctgtcaggttgaaggctgcagccatgatctttcatcagctaaagaatattaccggaagcatcgagtttgtgacagtcattccaaatgccaaaggtcattatagcaggtgtagcacgtcgcttttgtcaacagtgtagcaggttccatagcttgtctgaatttgatgaaaagaagagaagctgtcgcaggaggctctctgatcacaatgcacggcgccgcaaaccacagcaggaaaccatccagttcaactcggcaaggctttcttcattgttttatgatagcaggcaacctatgaatcttgtgctcaaccattcccaactggttcagtctagagctgctgcaaattctacctgggaaagcactgaagaaactaagttcagtataacaagagggtctactccaaagcctgaaagagctggcagtacaaatgggctgtcattattgccagggatccagttgtcacgggccgtgggtgcacacagtaatgtatctagctgcttgctcttgccctccaagggccacacatccgaggttttcaatcgaggtgccacggaatccatgttcaatatgggtacaggacgggaatttcctcgtgctctctctcttctgtcaactaattcatggggttcatccgagcctgagactgtttcactgaacaacccaacacacgcgaatcagagcagcatgcccgagcagatgatgcaggcaattccacaaggtgtgccacttatgtcctgtgaatactggcagggtgaacaaccctcatccgatcctcgtgaccatacattggctgctaatagtcatgctggtggtagctttcagggaatcgagctgttcaaacctccatttgacactgacttttatctcaatgcattgaactga

SEQ ID NO: 63 - DNA, 1390 bp, synthetic construct
  source 1..1390: mol_type = other DNA
atggagtggaataagtgggactggggaaacctggtaatgtttggttcagaggccgccaaaagtccaaaagaactacaattaacagattggggagttgaagaagatggagaacttgatgctggatccttcaatttgtcaagtggtggtagtggtagtggtagtggtaccggtggttatgtctctgatgttgggcatggttcttcgatcaagagctcaatatcagcttctactgactcttcacccaaggagggcttgaaagcatgcaacttttctttcgatggctcttctgaggatcttagtaagaaagtgaaactttgctctagaaattcaccccccatggaggcttcagtaggctctgttgaaccacttataggtctgaaacttggtaagcggacatttgagaccatcggcggtgctaaggtttcatccttccccgagaaacacgtatcatctgctgcagcagcaaagaaaacaaaatcatctactcagaatgcaccaactcctcgctgtcaggttgaaggctgcagccatgatctttcatcagctaaagaatattaccggaagcatcgagtttgtgacagtcattccaaatgcccaaaggtcattatagcaggtgtagcacgtcgcttttgtcaacagtgtagcaggttccatagcttgtctgaatttgatgaaaagaagagaagctgtcgcaggaggctctctgatcacaatgcacggcgccgcaaaccacagcaggaaaccatccagttcaaactcggcaaggctttcttcattgttttatgatagcaggcaacctatgaatcttgtgctcaaccattcccaactggttcagtctagagctgctgcaaattctacctgggaaagcactgaagaaactaagttcagtataacaagagggtctactccaaagcctgaaagagctggcagtacaaatgggctgtcattattgccagggatccagttgtcacgggccgtgggtgcacacagtaatgtatctagctgcttgctcttgccctccaagggccacacatccgaggttttcaatcgaggtgccacggaatccatgttcaatatgggtacaggacgggaatttcctcgtgctctctctcttctgtcaactaattcatggggttcatccgagcctgagactgtttcactgaacaacccaacacacgcgaatcagagcagcatgcccgagcagatgatgcaggcaattccacaaggtgtgccacttatgtcctgtgaatactggcagggtgaacaaccctcatccgatcctcgtgaccatacattggctgctaatagtcatgctggtggtagctttcagggaatcgagctgttcaaacctccatttgacactgacttttatctcaatgcattgaactga

SEQ ID NO: 64 - DNA, 1391 bp, synthetic construct
  source 1..1391: mol_type = other DNA
atggagtggaatgcaaagtgggactggggaaacctggtaatgtttggttcagaggccgccaaaagtccaaaagaactacaattaacagattggggagttgaagaagatggagaacttgatgctggatccttcaatttgtcaagtggtggtagtggtagtggtagtggtaccggtggttatgtctctgatgttgggcatggttcttcgatcaagagctcaatatcagcttctactgactcttcacccaaggagggcttgaaagcatgcaacttttctttcgatggctcttctgaggatcttagtaagaaagtgaaactttgctctagaaattcaccccccatggaggcttcagtaggctctgttgaaccacttataggtctgaaacttggtaagcggacatttgagaccatcggcggtgctaaggtttcatccttccccgagaaacacgtatcatctgctgcagcagcaaagaaaacaaaatcatctactcagaatgcaccaactcctcgctgtcaggttgaaggctgcagccatgatctttcatcagctaaagaatattaccggaagcatcgagtttgtgacagtcattccaaatgccaaaggtcattatagcaggtgtagcacgtcgcttttgtcaacagtgtagcaggttccatagcttgtctgaatttgatgaaaagaagagaagctgtcgcaggaggctctctgatcacaatgcacggcgccgcaaaccacagcaggaaaccatccagttcaactcggcaaggctttcttcattgttttatgatagcaggcaacctatgaatcttgtgctcaaccattcccaactggttcagtctagagctgctgcaaattctacctgggaaagcactgaagaaactaagttcagtataacaagagggtctactccaaagcctgaaagagctggcagtacaaatgggctgtcattattgccagggatccagttgtcacgggccgtgggtgcacacagtaatgtatctagctgcttgctcttgccctccaagggccacacatccgaggttttcaatcgaggtgccacggaatccatgttcaatatgggtacaggacgggaatttcctcgtgctctctctcttctgtcaactaattcatggggttcatccgagcctgagactgtttcactgaacaacccaacacacgcgaatcagagcagcatgcccgagcagatgatgcaggcaattccacaaggtgtgccacttatgtcctgtgaatactggcagggtgaacaaccctcatccgatcctcgtgaccatacattggctgctaatagtcatgctggtggtagctttcagggaatcgagctgttcaaacctccatttgacactgacttttatctcaatgcattgaactga

SEQ ID NO: 65 - DNA, 1393 bp, synthetic construct
  source 1..1393: mol_type = other DNA
atggagtggaatgcaaagtgggactggggaaacctggtaatgtttggttcagaggccgccaaaagtccaaaagaactacaattaacagattggggagttgaagaagatggagaacttgatgctggatccttcaatttgtcaagtggtggtagtggtagtggtagtggtaccggtggttatgtctctgatgttgggcatggttcttcgatcaagagctcaatatcagcttctactgactcttcacccaaggagggcttgaaagcatgcaacttttctttcgatggctcttctgaggatcttagtaagaaagtgaaactttgctctagaaattcaccccccatggaggcttcagtaggctctgttgaaccacttataggtctgaaacttggtaagcggacatttgagaccatcggcggtgctaaggtttcatccttccccgagaaacacgtatcatctgctgcagcagcaaagaaaacaaaatcatctactcagaatgcaccaactcctcgctgtcaggttgaaggctgcagccatgatctttcatcagctaaagaatattaccggaagcatcgagtttgtgacagtcattccaaatgcccaaaggtcattatagcaggtgtagcacgtcgcttttgtcaacagtgtagcaggttccatagcttgtctgaatttgatgaaaagaagagaagctgtcgcaggaggctctctgatcacaatgcacggcgccgcaaaccacagcaggaaaccatccagttcaaactcggcaaggctttcttcattgttttatgatagcaggcaacctatgaatcttgtgctcaaccattcccaactggttcagtctagagctgctgcaaattctacctgggaaagcactgaagaaactaagttcagtataacaagagggtctactccaaagcctgaaagagctggcagtacaaatgggctgtcattattgccagggatccagttgtcacgggccgtgggtgcacacagtaatgtatctagctgcttgctcttgccctccaagggccacacatccgaggttttcaatcgaggtgccacggaatccatgttcaatatgggtacaggacgggaatttcctcgtgctctctctcttctgtcaactaattcatggggttcatccgagcctgagactgtttcactgaacaacccaacacacgcgaatcagagcagcatgcccgagcagatgatgcaggcaattccacaaggtgtgccacttatgtcctgtgaatactggcagggtgaacaaccctcatccgatcctcgtgaccatacattggctgctaatagtcatgctggtggtagctttcagggaatcgagctgttcaaacctccatttgacactgacttttatctcaatgcattgaactga

SEQ ID NO: 66 - DNA, 1452 bp, synthetic construct
  source 1..1452: mol_type = other DNA
atggagtggaatgcaaagtgggactggggaaacctggtaatgtttggttcagaggccgccaaaagtccaaaagaactacaattaacagattggggagttgaagaagatggagaacttgatgctggatccttcaatttgtcaagtggtggtagtggtagtggtagtggtaccggtggttatgtctctgatgttgggcatggttcttcgatcaagagctcaatatcagcttctactgactcttcacccaaggagggcttgaaagcatgcaacttttctttcgatggctcttctgaggatcttagtaagaaagtgaaactttgctctagaaattcaccccccatggaggcttcagtaggctctgttgaaccacttataggtctgaaacttggtaagcggacatttgagaccatcggcggtgctaaggtttcatccttccccgagaaacacgtatcatctgctgcagcagcaaagaaaacaaaatcatctactcagaatgcaccaactcctcgctgtcaggttgaaggctgcagccatgatctttcatcagctaaagaatattaccggaagcatcgagtttgtgacagtcattccaaatgcccaaaggtcattatagcaggtgtagcacgtcgcttttgtcaacagtgtagcaggttccatagcttgtctgaatttgatgaaaagaagagaagctgtcgcaggaggctctctgatcacaatgcacggcgccgcaaaccacaatttagttgcaatttttgtcaaggatatctacctgctaatagcttgccttttagcaattttcgcaggaggctctctgatcactcggcaaggctttcttcattgttttatgatagcaggcaacctatgaatcttgtgctcaaccattcccaactggttcagtctagagctgctgcaaattctacctgggaaagcactgaagaaactaagttcagtataacaagagggtctactccaaagcctgaaagagctggcagtacaaatgggctgtcattattgccagggatccagttgtcacgggccgtgggtgcacacagtaatgtatctagctgcttgctcttgccctccaagggccacacatccgaggttttcaatcgaggtgccacggaatccatgttcaatatgggtacaggacgggaatttcctcgtgctctctctcttctgtcaactaattcatggggttcatccgagcctgagactgtttcactgaacaacccaacacacgcgaatcagagcagcatgcccgagcagatgatgcaggcaattccacaaggtgtgccacttatgtcctgtgaatactggcagggtgaacaaccctcatccgatcctcgtgaccatacattggctgctaatagtcatgctggtggtagctttcagggaatcgagctgttcaaacctccatttgacactgacttttatctcaatgcattgaactga

SEQ ID NO: 67 - DNA, 1389 bp, synthetic construct
  source 1..1389: mol_type = other DNA
atggagtggaatgcaaagtgggactggggaaacctggtaatgtttggttcagaggccgccaaaagtccaaaagaactacaattaacagattggggagttgaagaagatggagaacttgatgctggatccttcaatttgtcaagtggtggtagtggtagtggtagtggtaccggtggttatgtctctgatgttgggcatggttcttcgatcaagagctcaatatcagcttctactgactcttcacccaaggagggcttgaaagcatgcaacttttctttcgatggctcttctgaggatcttagtaagaaagtgaaactttgctctagaaattcacccctggaggcttcagtaggctctgttgaaccacttataggtctgaaacttggtaagcggacatttgagaccatcggcggtgctaaggtttcatccttccccgagaaacacgtatcatctgctgcagcagcaaagaaaacaaaatcatctactcagaatgcaccaactcctcgctgtcaggttgaaggctgcagccatgatctttcatcagctaaagaatattaccggaagcatcgagtttgtgacagtcattccaaatgcccaaaggtcattatagcaggtgtagcacgtcgcttttgtcaacagtgtagcaggttccatagcttgtctgaatttgatgaaaagaagagaagctgtcgcaggaggctctctgatcacaatgcacggcgccgcaaaccacagcaggaaaccatccagttcaactcggcaaggctttcttcattgttttatgatagcaggcaacctatgaatcttgtgctcaaccattcccaactggttcagtctagagctgctgcaaattctacctgggaaagcactgaagaaactaagttcagtataacaagagggtctactccaaagcctgaaagagctggcagtacaaatgggctgtcattattgccagggatccagttgtcacgggccgtgggtgcacacagtaatgtatctagctgcttgctcttgccctccaagggccacacatccgaggttttcaatcgaggtgccacggaatccatgttcaatatgggtacaggacgggaatttcctcgtgctctctctcttctgtcaactaattcatggggttcatccgagcctgagactgtttcactgaacaacccaacacacgcgaatcagagcagcatgcccgagcagatgatgcaggcaattccacaaggtgtgccacttatgtcctgtgaatactggcagggtgaacaaccctcatccgatcctcgtgaccatacattggctgctaatagtcatgctggtggtagctttcagggaatcgagctgttcaaacctccatttgacactgacttttatctcaatgcattgaactga

SEQ ID NO: 68 - DNA, 1449 bp, synthetic construct
  source 1..1449: mol_type = other DNA
atggagtggaatgcaaagtgggactggggaaacctggtaatgtttggttcagaggccgccaaaagtccaaaagaactacaattaacagattggggagttgaagaagatggagaacttgatgctggatccttcaatttgtcaagtggtggtagtggtagtggtagtggtaccggtggttatgtctctgatgttgggcatggttcttcgatcaagagctcaatatcagcttctactgactcttcacccaaggagggcttgaaagcatgcaacttttctttcgatggctcttctgaggatcttagtaagaaagtgaaactttgctctagaaattcacccctggaggcttcagtaggctctgttgaaccacttataggtctgaaacttggtaagcggacatttgagaccatcggcggtgctaaggtttcatccttccccgagaaacacgtatcatctgctgcagcagcaaagaaaacaaaatcatctactcagaatgcaccaactcctcgctgtcaggttgaaggctgcagccatgatctttcatcagctaaagaatattaccggaagcatcgagtttgtgacagtcattccaaatgcccaaaggtcattatagcaggtgtagcacgtcgcttttgtcaacagtgtagcaggttccatagcttgtctgaatttgatgaaaagaagagaagctgtcgcaggaggctctctgatcacaatgcacggcgccgcaaaccacaatttagttgcaatttttgtcaaggatatctacctgctaatagcttgccttttagcaattttcgcaggaggctctctgatcactcggcaaggctttcttcattgttttatgatagcaggcaacctatgaatcttgtgctcaaccattcccaactggttcagtctagagctgctgcaaattctacctgggaaagcactgaagaaactaagttcagtataacaagagggtctactccaaagcctgaaagagctggcagtacaaatgggctgtcattattgccagggatccagttgtcacgggccgtgggtgcacacagtaatgtatctagctgcttgctcttgccctccaagggccacacatccgaggttttcaatcgaggtgccacggaatccatgttcaatatgggtacaggacgggaatttcctcgtgctctctctcttctgtcaactaattcatggggttcatccgagcctgagactgtttcactgaacaacccaacacacgcgaatcagagcagcatgcccgagcagatgatgcaggcaattccacaaggtgtgccacttatgtcctgtgaatactggcagggtgaacaaccctcatccgatcctcgtgaccatacattggctgctaatagtcatgctggtggtagctttcagggaatcgagctgttcaaacctccatttgacactgacttttatctcaatgcattgaactga

SEQ ID NO: 69 - DNA, 1391 bp, synthetic construct
  source 1..1391: mol_type = other DNA
atggagtggaatgcaaagtgggactggggaaacctggtaatgtttggttcagaggccgccaaaagtccaaaagaactacaattaacagattggggagttgaagaagatggagaacttgatgctggatccttcaatttgtcaagtggtggtagtggtagtggtagtggtaccggtggttatgtctctgatgttgggcatggttcttcgatcaagagctcaatatcagcttctactgactcttcacccaaggagggcttgaaagcatgcaacttttctttcgatggctcttctgaggatcttagtaagaaagtgaaactttgctctagaaattcaccccccatggaggcttcagtaggctctgttgaaccacttataggtctgaaacttggtaagcggacatttgagaccatcggcggtgctaaggtttcatccttccccgagaaacacgtatcatctgctgcagcagcaaagaaaacaaaatcatctactcagaatgcaccaactcctcgctgtcaggttgaaggctgcagccatgatctttcatcagctaaagaatattaccggaagcatcgagtttgtgacagtcattccaaatgcccaaaggtcattatagcaggtgtagcacgtcgcttttgtcaacagtgtagcaggttccatagcttgtctgaatttgatgaaaagaagagaagctgtcgcaggaggctctctgatcacaatgcacggcgccgcaaaccacagcaggaaaccatccagttcactcggcaaggctttcttcattgttttatgatagcaggcaacctatgaatcttgtgctcaaccattcccaactggttcagtctagagctgctgcaaattctacctgggaaagcactgaagaaactaagttcagtataacaagagggtctactccaaagcctgaaagagctggcagtacaaatgggctgtcattattgccagggatccagttgtcacgggccgtgggtgcacacagtaatgtatctagctgcttgctcttgccctccaagggccacacatccgaggttttcaatcgaggtgccacggaatccatgttcaatatgggtacaggacgggaatttcctcgtgctctctctcttctgtcaactaattcatggggttcatccgagcctgagactgtttcactgaacaacccaacacacgcgaatcagagcagcatgcccgagcagatgatgcaggcaattccacaaggtgtgccacttatgtcctgtgaatactggcagggtgaacaaccctcatccgatcctcgtgaccatacattggctgctaatagtcatgctggtggtagctttcagggaatcgagctgttcaaacctccatttgacactgacttttatctcaatgcattgaactga

SEQ ID NO: 70 - DNA, 1369 bp, synthetic construct
  source 1..1369: mol_type = other DNA
atggagtggaatgcaaagtgggactggggaaacctggtaatgtttggttcagaggccgccaaaagtccaaaagaactacaattaacagattggggagttgaagaagatggagaacttgatgctggatccttcaatttgtcaagtggtggtagtggtagtggtagtggtaccggtggttatgtctctgatgttgggcatggttcttcgatcaagagctcaatatcagcttctactgactcttcacccaaggagggcttgaaagcatgcaacttttctttcgatggctcttctgaggatcttagtaagaaagtgaaactttgctctagaaattcaccccccatggaggcttcagtaggctctgttgaaccacttataggtctgaaacttggtaagcggacatttgagaccatcggcggtgctaaggtttcatccttccccgagaaacacgtatcatctgctgcagcagcaaagaaaacaaaatcatctactcagaatgcaccaactcctcgctgtcaggttgaaggctgcagccatgatctttcatcagctaaagaatattaccggaagcatcgagtttgtgacagtcattccaaatgcccaaaggtcattatagcaggtgtagcacgtcgcttttgtcaacagtgtagcaggttccatagcttgtctgaatttgatgaaaagaagagaagctgtcgcaggaggctctctgatcacaatgcacggcgccgcaaagcactcggcaaggctttcttcattgttttatgatagcaggcaacctatgaatcttgtgctcaaccattcccaactggttcagtctagagctgctgcaaattctacctgggaaagcactgaagaaactaagttcagtataacaagagggtctactccaaagcctgaaagagctggcagtacaaatgggctgtcattattgccagggatccagttgtcacgggccgtgggtgcacacagtaatgtatctagctgcttgctcttgccctccaagggccacacatccgaggttttcaatcgaggtgccacggaatccatgttcaatatgggtacaggacgggaatttcctcgtgctctctctcttctgtcaactaattcatggggttcatccgagcctgagactgtttcactgaacaacccaacacacgcgaatcagagcagcatgcccgagcagatgatgcaggcaattccacaaggtgtgccacttatgtcctgtgaatactggcagggtgaacaaccctcatccgatcctcgtgaccatacattggctgctaatagtcatgctggtggtagctttcagggaatcgagctgttcaaacctccatttgacactgacttttatctcaatgcattgaactga

SEQ ID NO: 71 - DNA, 1330 bp, synthetic construct
  source 1..1330: mol_type = other DNA
atggagtggaatgcaaagtgggactggggaaacctggtaatgtttggttcagaggtcgccaaaagtccaaaagaactacaattaacagattggggagttgaagaagatggagaacttgatgctggatccttcaatttgtcgagtggtggtagtggtagtggtactggtggttatgtctctgatgttgggtgtggttcttcgatcaagagctcaatatcagcttctactgactcttcaccaaaggagggcttgaaagcatccgacttttctttcgatggctctcctgaggatcttagtaagaaagtgaaaccttgctctagaaattcaccccccatggaggctccagtaggctctgttgaaccacttgtaggtctgaaacttggtaagcggacatttgagaccatcggtggtgctaaggtttcatccttccccgataaacacgtatcatctgctgcagcagcaaagaaaacaaaatcatctactcagaatgcaccaactccacgctgtcaggttgaaggctgcaaccttgatctttcatcagctaaagaatattaccggaagcatcgagtttgtgaaaatcattccaaatgcccaaaggtcattatagcaggtgtattacgccgcttttgtcaacagtgtagcaggttccatagcttgtctgaatttgatgaaaagaagagaagctgccgcagactcggcaaggctttcttcattgttttatgatagcaggcaacctatgaatcttgtgctcaaccattccaacctggttcagtgtagagctgctgcaaattctacctgggaaagcactgaagaaactaagttcagtataacaagaggattagctccaaagcctgaaagagatggcagtacaaatgggcagtcattattgccagggatccagttttcacgggccgtgggtgcacacggtaatgtatctagctgcttgctcttgccctccaagggccacacagccgaggttttcaatcgaggtgccaaggaatccatgttcaatatgggtacaggaccggaatttcctcgtgctctctctcttctgtcaactaattcatggggttcatccgagcctgagactgtttcactgaaccacccaacacatgcaaatcagagcagcatgcccgagcagatgatgcaggcaattccacaaggtgtgccgcttctgtcctgtgaatactggcagggtgatggacaaccttcatccgatcctcgtgaccatacattggctgctaatagtcatgctggtggtagctttcagggaatcgaactgttcaaacctccatttgacactgatttttatctcaatgcattgaactga

SEQ ID NO: 72 - DNA, 1385 bp, synthetic construct
  source 1..1385: mol_type = other DNA
atggagtggaatgcaaagtgggactggggaaacctggtaatgtttggttcagaggtcgccaaaagtccaaaagaactacaattaacagattggggagttgaagaagatggagaacttgatgctggatccttcaatttgtcgagtggtggtagtggtagtggtactggtggttatgtctctgatgttgggtgtggttcttcgatcaagagctcaatatcagcttctactgactcttcaccaaaggagggcttgaaagcatccgacttttctttcgatggctctcctgaggatcttagtaagaaagtgaaaccttgctctagaaattcaccccccatggaggctccagtaggctctgttgaaccacttgtaggtctgaaacttggtaagcggacatttgagaccatcggtggtgctaaggtttcatccttccccgataaacacgtatcatctgctgcagcagcaaagaaaacaaaatcatctactcagaatgcaccaactccacgctgtcaggttgaaggctgcaaccttgatctttcatcagctaaagaatattaccggaagcatcgagtttgtgaaaatcattccaaatgcccaaaggtcattatagcaggtgtattacgccgcttttgtcaacagtgtagcaggttccatagcttgtctgaatttgatgaaaagaagagaagctgccgcaggctctctgatcacaatgcacgacgccgcaaaccacagcaggaaaccatccagttcactcggcaaggctttcttcattgttttatgatagcaggcaacctatgaatcttgtgctcaaccattccaacctggttcagtgtagagctgctgcaaattctacctgggaaagcactgaagaaactaagttcagtataacaagaggattagctccaaagcctgaaagagatggcagtacaaatgggcagtcattattgccagggatccagttttcacgggccgtgggtgcacacggtaatgtatctagctgcttgctcttgccctccaagggccacacagccgaggttttcaatcgaggtgccaaggaatccatgttcaatatgggtacaggaccggaatttcctcgtgctctctctcttctgtcaactaattcatggggttcatccgagcctgagactgtttcactgaaccacccaacacatgcaaatcagagcagcatgcccgagcagatgatgcaggcaattccacaaggtgtgccgcttctgtcctgtgaatactggcagggtgatggacaaccttcatccgatcctcgtgaccatacattggctgctaatagtcatgctggtggtagctttcagggaatcgaactgttcaaacctccatttgacactgatttttatctcaatgcattgaactga

SEQ ID NO: 73 - DNA, 1390 bp, synthetic construct
  source 1..1390: mol_type = other DNA
atggagtggaatgcaaagtgggactggggaaacctggtaatgtttggttcagaggtcgccaaaagtccaaaagaactacaattaacagattggggagttgaagaagatggagaacttgatgctggatccttcaatttgtcgagtggtggtagtggtagtggtactggtggttatgtctctgatgttgggtgtggttcttcgatcaagagctcaatatcagcttctactgactcttcaccaaaggagggcttgaaagcatccgacttttctttcgatggctctcctgaggatcttagtaagaaagtgaaaccttgctctagaaattcaccccccatggaggctccagtaggctctgttgaaccacttgtaggtctgaaacttggtaagcggacatttgagaccatcggtggtgctaaggtttcatccttccccgataaacacgtatcatctgctgcagcagcaaagaaaacaaaatcatctactcagaatgcaccaactccacgctgtcaggttgaaggctgcaaccttgatctttcatcagctaaagaatattaccggaagcatcgagtttgtgaaaatcattccaaatgcccaaaggtcattatagcaggtgtattacgccgcttttgtcaacagtgtagcaggttccatagcttgtctgaatttgatgaaaagaagagaagctgccgcagtgaggctctctgatcacaatgcacgacgccgcaaaccacagcaggaaaccatccagttcaactcggcaaggctttcttcattgttttatgatagcaggcaacctatgaatcttgtgctcaaccattccaacctggttcagtgtagagctgctgcaaattctacctgggaaagcactgaagaaactaagttcagtataacaagaggattagctccaaagcctgaaagagatggcagtacaaatgggcagtcattattgccagggatccagttttcacgggccgtgggtgcacacggtaatgtatctagctgcttgctcttgccctccaagggccacacagccgaggttttcaatcgaggtgccaaggaatccatgttcaatatgggtacaggaccggaatttcctcgtgctctctctcttctgtcaactaattcatggggttcatccgagcctgagactgtttcactgaaccacccaacacatgcaaatcagagcagcatgcccgagcagatgatgcaggcaattccacaaggtgtgccgcttctgtcctgtgaatactggcagggtgatggacaaccttcatccgatcctcgtgaccatacattggctgctaatagtcatgctggtggtagctttcagggaatcgaactgttcaaacctccatttgacactgatttttatctcaatgcattgaactga

SEQ ID NO: 74 - DNA, 1390 bp, synthetic construct
  source 1..1390: mol_type = other DNA
atggagtggaatgcaaagtgggactggggaaacctggtaatgtttggttcagaggtcgccaaaagtccaaaagaactacaattaacagattggggagttgaagaagatggagaacttgatgctggatccttcaatttgtcgagtggtggtagtggtagtggtactggtggttatgtctctgatgttgggtgtggttcttcgatcaagagctcaatatcagcttctactgactcttcaccaaaggagggcttgaaagcatccgacttttctttcgatggctctcctgaggatcttagtaagaaagtgaaaccttgctctagaaattcaccccccatggaggctccagtaggctctgttgaaccacttgtaggtctgaaacttggtaagcggacatttgagaccatcggtggtgctaaggtttcatccttccccgataaacacgtatcatctgctgcagcagcaaagaaaacaaaatcatctactcagaatgcaccaactccacgctgtcaggttgaaggctgcaaccttgatctttcatcagctaaagaatattaccggaagcatcgagtttgtgaaaatcattccaaatgcccaaaggtcattatagcaggtgtattacgccgcttttgtcaacagtgtagcaggttccatagcttgtctgaatttgatgaaaagaagagaagctgccgcaggaggctctctgatcacaatgcacgacgccgcaaaccacagcaggaaaccatccagttcaaactcggcaaggctttcttcattgttttatgatagcaggcaacctatgaatcttgtgctcaaccattccaacctggttcagtgtagagctgctgcaaattctacctgggaaagcactgaagaaactaagttcagtataacaagaggattagctccaaagcctgaaagagatggcagtacaaatgggcagtcattattgccagggatccagttttcacgggccgtgggtgcacacggtaatgtatctagctgcttgctcttgccctccaagggccacacagccgaggttttcaatcgaggtgccaaggaatccatgttcaatatgggtacaggaccggaatttcctcgtgctctctctcttctgtcaactaattcatggggttcatccgagcctgagactgtttcactgaaccacccaacacatgcaaatcagagcagcatgcccgagcagatgatgcaggcaattccacaaggtgtgccgcttctgtcctgtgaatactggcagggtgatggacaaccttcatccgatcctcgtgaccatacattggctgctaatagtcatgctggtggtagctttcagggaatcgaactgttcaaacctccatttgacactgatttttatctcaatgcattgaactga

SEQ ID NO: 75 - DNA, 1389 bp, synthetic construct
  source 1..1389: mol_type = other DNA
atggagtggaatgcaaagtgggactggggaaacctggtaatgtttggttcagaggtcgccaaaagtccaaaagaactacaattaacagattggggagttgaagaagatggagaacttgatgctggatccttcaatttgtcgagtggtggtagtggtagtggtactggtggttatgtctctgatgttgggtgtggttcttcgatcaagagctcaatatcagcttctactgactcttcaccaaaggagggcttgaaagcatccgacttttctttcgatggctctcctgaggatcttagtaagaaagtgaaaccttgctctagaaattcaccccccatggaggctccagtaggctctgttgaaccacttgtaggtctgaaacttggtaagcggacatttgagaccatcggtggtgctaaggtttcatccttccccgataaacacgtatcatctgctgcagcagcaaagaaaacaaaatcatctactcagaatgcaccaactccacgctgtcaggttgaaggctgcaaccttgatctttcatcagctaaagaatattaccggaagcatcgagtttgtgaaaatcattccaaatgcccaaaggtcattatagcaggtgtattacgccgcttttgtcaacagtgtagcaggttccatagcttgtctgaatttgatgaaaagaagagaagctgccgcagaggctctctgatcacaatgcacgacgccgcaaaccacagcaggaaaccatccagttcaaactcggcaaggctttcttcattgttttatgatagcaggcaacctatgaatcttgtgctcaaccattccaacctggttcagtgtagagctgctgcaaattctacctgggaaagcactgaagaaactaagttcagtataacaagaggattagctccaaagcctgaaagagatggcagtacaaatgggcagtcattattgccagggatccagttttcacgggccgtgggtgcacacggtaatgtatctagctgcttgctcttgccctccaagggccacacagccgaggttttcaatcgaggtgccaaggaatccatgttcaatatgggtacaggaccggaatttcctcgtgctctctctcttctgtcaactaattcatggggttcatccgagcctgagactgtttcactgaaccacccaacacatgcaaatcagagcagcatgcccgagcagatgatgcaggcaattccacaaggtgtgccgcttctgtcctgtgaatactggcagggtgatggacaaccttcatccgatcctcgtgaccatacattggctgctaatagtcatgctggtggtagctttcagggaatcgaactgttcaaacctccatttgacactgatttttatctcaatgcattgaactga

SEQ ID NO: 76 - DNA, 1386 bp, synthetic construct
  source 1..1386: mol_type = other DNA
atggagtggaatgcaaagtgggactggggaaacctggtaatgtttggttcagaggtcgccaaaagtccaaaagaactacaattaacagattggggagttgaagaagatggagaacttgatgctggatccttcaatttgtcgagtggtggtagtggtagtggtactggtggttatgtctctgatgttgggtgtggttcttcgatcaagagctcaatatcagcttctactgactcttcaccaaaggagggcttgaaagcatccgacttttctttcgatggctctcctgaggatcttagtaagaaagtgaaaccttgctctagaaattcaccccccatggaggctccagtaggctctgttgaaccacttgtaggtctgaaacttggtaagcggacatttgagaccatcggtggtgctaaggtttcatccttccccgataaacacgtatcatctgctgcagcagcaaagaaaacaaaatcatctactcagaatgcaccaactccacgctgtcaggttgaaggctgcaaccttgatctttcatcagctaaagaatattaccggaagcatcgagtttgtgaaaatcattccaaatgcccaaaggtcattatagcaggtgtattacgccgcttttgtcaacagtgtagcaggttccatagcttgtctgaatttgatgaaaagaagagaagctgccgcagaggctctctgatcacaatgcacgacgccgcaaaccacagcaggaaaccatccagtaactcggcaaggctttcttcattgttttatgatagcaggcaacctatgaatcttgtgctcaaccattccaacctggttcagtgtagagctgctgcaaattctacctgggaaagcactgaagaaactaagttcagtataacaagaggattagctccaaagcctgaaagagatggcagtacaaatgggcagtcattattgccagggatccagttttcacgggccgtgggtgcacacggtaatgtatctagctgcttgctcttgccctccaagggccacacagccgaggttttcaatcgaggtgccaaggaatccatgttcaatatgggtacaggaccggaatttcctcgtgctctctctcttctgtcaactaattcatggggttcatccgagcctgagactgtttcactgaaccacccaacacatgcaaatcagagcagcatgcccgagcagatgatgcaggcaattccacaaggtgtgccgcttctgtcctgtgaatactggcagggtgatggacaaccttcatccgatcctcgtgaccatacattggctgctaatagtcatgctggtggtagctttcagggaatcgaactgttcaaacctccatttgacactgatttttatctcaatgcattgaactga

SEQ ID NO: 77 - DNA, 1389 bp, synthetic construct; identical to SEQ ID NO: 75
  source 1..1389: mol_type = other DNA

SEQ ID NO: 78 - DNA, 1391 bp, synthetic construct
  source 1..1391: mol_type = other DNA
atggagtggaatgcaaagtgggactggggaaacctggtaatgtttggttcagaggtcgccaaaagtccaaaagaactacaattaacagattggggagttgaagaagatggagaacttgatgctggatccttcaatttgtcgagtggtggtagtggtagtggtactggtggttatgtctctgatgttgggtgtggttcttcgatcaagagctcaatatcagcttctactgactcttcaccaaaggagggcttgaaagcatccgacttttctttcgatggctctcctgaggatcttagtaagaaagtgaaaccttgctctagaaattcaccccccatggaggctccagtaggctctgttgaaccacttgtaggtctgaaacttggtaagcggacatttgagaccatcggtggtgctaaggtttcatccttccccgataaacacgtatcatctgctgcagcagcaaagaaaacaaaatcatctactcagaatgcaccaactccacgctgtcaggttgaaggctgcaaccttgatctttcatcagctaaagaatattaccggaagcatcgagtttgtgaaaatcattccaaatgcccaaaggtcattatagcaggtgtattacgccgcttttgtcaacagtgtagcaggttccatagcttgtctgaatttgatgaaaagaagagaagctgccgcagtgaggctctctgatcacaatgcacgacgccgcaaaccacagcaggaaaccatccagttcagactcggcaaggctttcttcattgttttatgatagcaggcaacctatgaatcttgtgctcaaccattccaacctggttcagtgtagagctgctgcaaattctacctgggaaagcactgaagaaactaagttcagtataacaagaggattagctccaaagcctgaaagagatggcagtacaaatgggcagtcattattgccagggatccagttttcacgggccgtgggtgcacacggtaatgtatctagctgcttgctcttgccctccaagggccacacagccgaggttttcaatcgaggtgccaaggaatccatgttcaatatgggtacaggaccggaatttcctcgtgctctctctcttctgtcaactaattcatggggttcatccgagcctgagactgtttcactgaaccacccaacacatgcaaatcagagcagcatgcccgagcagatgatgcaggcaattccacaaggtgtgccgcttctgtcctgtgaatactggcagggtgatggacaaccttcatccgatcctcgtgaccatacattggctgctaatagtcatgctggtggtagctttcagggaatcgaactgttcaaacctccatttgacactgatttttatctcaatgcattgaactga

SEQ ID NO: 79 - DNA, 1391 bp, synthetic construct
  source 1..1391: mol_type = other DNA
atggagtggaatgcaaagtgggactggggaaacctggtaatgtttggttcagaggtcgccaaaagtccaaaagaactacaattaacagattggggagttgaagaagatggagaacttgatgctggatccttcaatttgtcgagtggtggtagtggtagtggtactggtggttatgtctctgatgttgggtgtggttcttcgatcaagagctcaatatcagcttctactgactcttcaccaaaggagggcttgaaagcatccgacttttctttcgatggctctcctgaggatcttagtaagaaagtgaaaccttgctctagaaattcaccccccatggaggctccagtaggctctgttgaaccacttgtaggtctgaaacttggtaagcggacatttgagaccatcggtggtgctaaggtttcatccttccccgataaacacgtatcatctgctgcagcagcaaagaaaacaaaatcatctactcagaatgcaccaactccacgctgtcaggttgaaggctgcaaccttgatctttcatcagctaaagaatattaccggaagcatcgagtttgtgaaaatcattccaaatgcccaaaggtcattatagcaggtgtattacgccgcttttgtcaacagtgtagcaggttccatagcttgtctgaatttgatgaaaagaagagaagctgccgcagtgaggctctctgatcacaatgcacgacgccgcaaaccacagcaggaaaccatccagttcatactcggcaaggctttcttcattgttttatgatagcaggcaacctatgaatcttgtgctcaaccattccaacctggttcagtgtagagctgctgcaaattctacctgggaaagcactgaagaaactaagttcagtataacaagaggattagctccaaagcctgaaagagatggcagtacaaatgggcagtcattattgccagggatccagttttcacgggccgtgggtgcacacggtaatgtatctagctgcttgctcttgccctccaagggccacacagccgaggttttcaatcgaggtgccaaggaatccatgttcaatatgggtacaggaccggaatttcctcgtgctctctctcttctgtcaactaattcatggggttcatccgagcctgagactgtttcactgaaccacccaacacatgcaaatcagagcagcatgcccgagcagatgatgcaggcaattccacaaggtgtgccgcttctgtcctgtgaatactggcagggtgatggacaaccttcatccgatcctcgtgaccatacattggctgctaatagtcatgctggtggtagctttcagggaatcgaactgttcaaacctccatttgacactgatttttatctcaatgcattgaactga

SEQ ID NO: 80 - DNA, 1388 bp, synthetic construct
  source 1..1388: mol_type = other DNA
atggagtggaatgcaaagtgggactggggaaacctggtaatgtttggttcagaggtcgccaaaagtccaaaagaactacaattaacagattggggagttgaagaagatggagaacttgatgctggatccttcaatttgtcgagtggtggtagtggtagtggtactggtggttatgtctctgatgttgggtgtggttcttcgatcaagagctcaatatcagcttctactgactcttcaccaaaggagggcttgaaagcatccgacttttctttcgatggctctcctgaggatcttagtaagaaagtgaaaccttgctctagaaattcaccccccatggaggctccagtaggctctgttgaaccacttgtaggtctgaaacttggtaagcggacatttgagaccatcggtggtgctaaggtttcatccttccccgataaacacgtatcatctgctgcagcagcaaagaaaacaaaatcatctactcagaatgcaccaactccacgctgtcaggttgaaggctgcaaccttgatctttcatcagctaaagaatattaccggaagcatcgagtttgtgaaaatcattccaaatgcccaaaggtcattatagcaggtgtattacgccgcttttgtcaacagtgtagcaggttccatagcttgtctgaatttgatgaaaagaagagaagctgccgcagggctctctgatcacaatgcacgacgccgcaaaccacagcaggaaaccatccagttcagactcggcaaggctttcttcattgttttatgatagcaggcaacctatgaatcttgtgctcaaccattccaacctggttcagtgtagagctgctgcaaattctacctgggaaagcactgaagaaactaagttcagtataacaagaggattagctccaaagcctgaaagagatggcagtacaaatgggcagtcattattgccagggatccagttttcacgggccgtgggtgcacacggtaatgtatctagctgcttgctcttgccctccaagggccacacagccgaggttttcaatcgaggtgccaaggaatccatgttcaatatgggtacaggaccggaatttcctcgtgctctctctcttctgtcaactaattcatggggttcatccgagcctgagactgtttcactgaaccacccaacacatgcaaatcagagcagcatgcccgagcagatgatgcaggcaattccacaaggtgtgccgcttctgtcctgtgaatactggcagggtgatggacaaccttcatccgatcctcgtgaccatacattggctgctaatagtcatgctggtggtagctttcagggaatcgaactgttcaaacctccatttgacactgatttttatctcaatgcattgaactga

SEQ ID NO: 81 - DNA, 1388 bp, synthetic construct
  source 1..1388: mol_type = other DNA
atggagtggaatgcaaagtgggactggggaaacctggtaatgtttggttcagaggtcgccaaaagtccaaaagaactacaattaacagattggggagttgaagaagatggagaacttgatgctggatccttcaatttgtcgagtggtggtagtggtagtggtactggtggttatgtctctgatgttgggtgtggttcttcgatcaagagctcaatatcagcttctactgactcttcaccaaaggagggcttgaaagcatccgacttttctttcgatggctctcctgaggatcttagtaagaaagtgaaaccttgctctagaaattcaccccccatggaggctccagtaggctctgttgaaccacttgtaggtctgaaacttggtaagcggacatttgagaccatcggtggtgctaaggtttcatccttccccgataaacacgtatcatctgctgcagcagcaaagaaaacaaaatcatctactcagaatgcaccaactccacgctgtcaggttgaaggctgcaaccttgatctttcatcagctaaagaatattaccggaagcatcgagtttgtgaaaatcattccaaatgcccaaaggtcattatagcaggtgtattacgccgcttttgtcaacagtgtagcaggttccatagcttgtctgaatttgatgaaaagaagagaagctgccgcagggctctctgatcacaatgcacgacgccgcaaaccacagcaggaaaccatccagttcatactcggcaaggctttcttcattgttttatgatagcaggcaacctatgaatcttgtgctcaaccattccaacctggttcagtgtagagctgctgcaaattctacctgggaaagcactgaagaaactaagttcagtataacaagaggattagctccaaagcctgaaagagatggcagtacaaatgggcagtcattattgccagggatccagttttcacgggccgtgggtgcacacggtaatgtatctagctgcttgctcttgccctccaagggccacacagccgaggttttcaatcgaggtgccaaggaatccatgttcaatatgggtacaggaccggaatttcctcgtgctctctctcttctgtcaactaattcatggggttcatccgagcctgagactgtttcactgaaccacccaacacatgcaaatcagagcagcatgcccgagcagatgatgcaggcaattccacaaggtgtgccgcttctgtcctgtgaatactggcagggtgatggacaaccttcatccgatcctcgtgaccatacattggctgctaatagtcatgctggtggtagctttcagggaatcgaactgttcaaacctccatttgacactgatttttatctcaatgcattgaactga

SEQ ID NO: 82 - DNA, 1376 bp, synthetic construct
  source 1..1376: mol_type = other DNA
atggagtggaatgcaaagtgggactggggaaacctggtaatgtttggttcagaggtcgccaaaagtccaaaagaactacaattaacagattggggagttgaagaagatggagaacttgatgctggatccttcaatttgtcgagtggtggtagtggtagtggtactggtggttatgtctctgatgttgggtgtggttcttcgatcaagagctcaatatcagcttctactgactcttcaccaaaggagggcttgaaagcatccgacttttctttcgatggctctcctgaggatcttagtaagaaagtgaaaccttgctctagaaattcaccccccatggaggctccagtaggctctgttgaaccacttgtaggtctgaaacttggtaagcggacatttgagaccatcggtggtgctaaggtttcatccttccccgataaacacgtatcatctgctgcagcagcaaagaaaacaaaatcatctactcagaatgcaccaactccacgctgtcaggttgaaggctgcaaccttgatctttcatcagctaaagaatattaccggaagcatcgagtttgtgaaaatcattccaaatgcccaaaggtcattatagcaggtgtattacgccgcttttgtcaacagtgtagcaggttccatagcttgtctgaatttgatgaaaagaagagaagctgccgcagtgaggctctctgatcacaatgcacgacgccgcaaaccacagcaggaaaccatccaggctttcttcattgttttatgatagcaggcaacctatgaatcttgtgctcaaccattccaacctggttcagtgtagagctgctgcaaattctacctgggaaagcactgaagaaactaagttcagtataacaagaggattagctccaaagcctgaaagagatggcagtacaaatgggcagtcattattgccagggatccagttttcacgggccgtgggtgcacacggtaatgtatctagctgcttgctcttgccctccaagggccacacagccgaggttttcaatcgaggtgccaaggaatccatgttcaatatgggtacaggaccggaatttcctcgtgctctctctcttctgtcaactaattcatggggttcatccgagcctgagactgtttcactgaaccacccaacacatgcaaatcagagcagcatgcccgagcagatgatgcaggcaattccacaaggtgtgccgcttctgtcctgtgaatactggcagggtgatggacaaccttcatccgatcctcgtgaccatacattggctgctaatagtcatgctggtggtagctttcagggaatcgaactgttcaaacctccatttgacactgatttttatctcaatgcattgaactga

SEQ ID NO: 83 - DNA, 1072 bp, synthetic construct
  source 1..1072: mol_type = other DNA
atgcagttgtgtgcgcatagcattctgctgaagtatgacaatcaagttttaatatacttctttgtctgttactggaatccaacagctctgtttgataaagatccgagtcctacttactttattgcattccatgagtggggaactttacaaaagccatctcgtagcttcttccccaagatggagtggaatgcaaaagtgggactggggaaaccagaccatcggtggtgctaagatttcatccttcgccgagaaacccgtatcatctgctgcagcagcaaagaaaacaaaatcatctactcagaatgcaccaactcctcgctgtcaggttgaaggctgcagccttgatctttcatcagctaaagaatattatcggaagcatagagtttgtgacagtcattccaaatgcccaaaggtcactatagcaggtgtagcacgccatttttgtcaacaatgtagcaggttccatagcttgtctgaatttgatgaaaagaagagaagctgtcgcaggaggctctctgatcacaatgcacggcgccgcaaaccacagcaggaaatcatccagctgaactcggcaaggctttcttcattgttttatgatagcaggaaacctatgaatcttacccaactggttcactctagagctgctgcaaattctaccagggaaagcactgaagaaactaatttcagtataacaagagggtctactccaaagcctgaaagagctggcagtacaaatgggcagtcattactgtcggggatccagttttccttggccgtgggtgcacacagtaatgtatctagctgcttgctcttgccctccaagggccacatagacgaggttttcaatcgagatgccaaggaatccatgaccggaatttcctcatggggttcatccgagcctgagactgtttcactgaaccacccaacacatgtaaatcagagcagcatgcctgagcagatgatgcaggcaatcccacaaggtgtgccacttatgtcctgtgaatactggcagagaggacaaccttcatccgatcctcgtgaccatacattggctgctaatagtcatgcaagt

SEQ ID NO: 84 - DNA, 1392 bp, synthetic construct
  source 1..1392: mol_type = other DNA
atgacaatcaaagtgaggaaacaacaagtagctgaaaatgatgtggtggagttaagggatgcgatagatggggagatgcattttgtggccttggattggaagggcttgagctctgattctcttcttcccaagacggagtggaatgcaaagtgggactggggaaacctgataatgtttggttcaaaggccgccaaaagtccaaaagaactacaattaacagattggggaattgaagaagatggagaacttgatgctggatccttcaatttgtcgagtggtggtagtggtagtggtacaggtggttatgtctctgatgtggggcgtggttcttcgatcaagagctcaatatcagcttctactgactcttcaccaaaggagggcttgaaagcatccaacttttctttcgatggctctcctgaggatcttagtaagaaagtgaaaccttggtctagaaatttggaggctttggtaggctctgttgaaccacttataggtctgaaacttggtaagcggacatttgagaccatcggtggtgctaagatttcatccttccccgagaaccccgtatcatctgctgctgcagcaaagaaaacaaaatcatctactcaaaatgcgccaactcctcgctgtcaggttgaaggctgcaaccttaatctttcatcagctttgaatattactggaagcatcgagtttgtgacagtcattccaaatgcccaaaggcaacctatgaatcttgttctcaaccacacccaactggttcactctagagctgctgcaaaaagcactgaagaaactaagttcagtataacaagagggtctactccaaagcctgaaagagctggcagtacaaatgggcagtcattactgccggggatccagttttcacgggccgtgggtgcacacagtaatggccacacagccgaggttttcaatcgacgtgccaaggaatccatgctcaaaatgggtacaggaccggaatttcctcgtgctctctctcttctgtcaactaattcatggggttcatccgagcctgagactgtttcactgaaccacccaacacatgcaaatcagagcagcatgcccgagcagatgatgcaggcaattccacaaggtgtgccacttatgtcctgtgaatactggcagggtggacaaccttcatccgatcctcgtgaccatacattggctgctaatagtcatgcttgcgtgattcaaaggagtgaaaatgtaagacagaagatataccttcctgaggagaatggcaacgtcagcttgagagtcttcaatggactggctgccacactctgtacacctgacattgtggctgatatttcttgctcttgcctctaccaccctctccttcttcaccgaatcctcttccccctccatagatag

SEQ ID NO: 85 - DNA, 540 bp, synthetic construct
  source 1..540: mol_type = other DNA
atgccaagagaacgtgaacctctggtagttggtcgagtgataggggatgtattggaccctttcacaagatctattggcctaggagttatttatagggatagagaagttaataatgggtgtgagcttaggccttcccaagttattaaccagcccagggttgaagttggtggagatgaccttcgtaccttttacactctggttatggtggaccctgatgctccaagtccaagtgatccaaatctaagagaataccgttggtcactgatattccagctaccacaggtgcaagttttggccaggaaattgtgtgctatgaaagtccaaggccaacaatgggaatacatcgctttgtattcgtattgtttagacaattgggtcgacagacagtgtatgctccaggatggcgtcagaatttcaatacaaaagattttgctgaactctataatcttggtttaccagttgctgctgtctattttaattgtcaaagagagagtggcagtggtggacgtagaaggtctgccgattgacatgcacttttaa

SEQ ID NO: 86 - DNA, 535 bp, synthetic construct
  source 1..535: mol_type = other DNA
atgccaagagaacgtgaacctctggtagttggtcgagtgataggggatgtattggaccctttcacaagatctattggcctaggagttatttatagggatagagaagttaataatgggtgtgagcttaggccttcccaagttattaaccagcccagggttgaagttggtggagatgaccttcgtaccttttacactctggttatggtggaccctgatgctccaagtccaagtgatccaaatctaagagaatacctccatttggttggtcactgatattccagctaccacaggtgcaagttttggccaggaaattgtgtgctatgaaagtccaaggccaacaatgggaatacatcgctttgtattcgtattgtttagacaattgggtcgacagacagtgtatgctccaggatggcgtcagaatttcaatacaaaagattttgctgaactctataatcttggtttaccagttgctgctgtctattttaattgtcaaagagagagtggcagtggtggacgtagaaggtctgccgattga

SEQ ID NO: 87 - DNA, 535 bp, synthetic construct
  source 1..535: mol_type = other DNA
atgccaagagaacgtgaacctctggtagttggtcgagtgataggggatgtattggaccctttcacaagatctattggcctaggagttatttatagggatagagaagttaataatgggtgtgagcttaggccttcccaagttattaaccagcccagggttgaagttggtggagatgaccttcgtaccttttacactctggttatggtggaccctgatgctccaagtccaagtgatccaaatctaagagaatacctccaattggttggtcactgatattccagctaccacaggtgcaagttttggccaggaaattgtgtgctatgaaagtccaaggccaacaatgggaatacatcgctttgtattcgtattgtttagacaattgggtcgacagacagtgtatgctccaggatggcgtcagaatttcaatacaaaagattttgctgaactctataatcttggtttaccagttgctgctgtctattttaattgtcaaagagagagtggcagtggtggacgtagaaggtctgccgattga

SEQ ID NO: 88 - DNA, 535 bp, synthetic construct
  source 1..535: mol_type = other DNA
atgccaagagaacgtgaacctctggtagttggtcgagtgataggggatgtattggaccctttcacaagatctattggcctaggagttatttatagggatagagaagttaataatgggtgtgagcttaggccttcccaagttattaaccagcccagggttgaagttggtggagatgaccttcgtaccttttacactctggttatggtggaccctgatgctccaagtccaagtgatccaaatctaagagaatacctccacttggttggtcactgatattccagctaccacaggtgcaagttttggccaggaaattgtgtgctatgaaagtccaaggccaacaatgggaatacatcgctttgtattcgtattgtttagacaattgggtcgacagacagtgtatgctccaggatggcgtcagaatttcaatacaaaagattttgctgaactctataatcttggtttaccagttgctgctgtctattttaattgtcaaagagagagtggcagtggtggacgtagaaggtctgccgattga

SEQ ID NO: 89 - DNA, 535 bp, synthetic construct
  source 1..535: mol_type = other DNA
atgccaagagaacgtgaacctctggtagttggtcgagtgataggggatgtattggaccctttcacaagatctattggcctaagagttatttatagggatagagaagttaataatgggtgtgagcttaggccttcccaagttgttaaccagccaagggttgaagttggtggagatgaccttcgtaccttttacactctggttatggtggaccctgatgctccaagtccaagatatccaaatctaagagaatacctccatttggttggtcactgatattccagctaccacaggtgcaagttttgggcaagaaattgtgtgctatgaaagtccaaggccaacaatgggaatacatcgctttgtattcgtattgtttagacaattgggtcgacagacagtgtatgctccaggatggcgtcagaatttcaatacaaaagactttgctgaactctataatcttggtttaccggttgctgccgtctattttaattgtcaaagagagagtggcagtggtggacgtagaaggtctgccgattga

SEQ ID NO: 90 - DNA, 552 bp, synthetic construct
  source 1..552: mol_type = other DNA
atgccaagagaacgtgaacctctggtagttggtcgagtgataggggatgtattggaccctttcacaagatctattggcctaagagttatttatagggatagagaagttaataatgggtgtgagcttaggccttcccaagttgttaaccagccaagggttgaagttggtggagatgaccttcgtaccttttacactctggttatggtggaccctgatgctccaagtccaagatatccaaatctaagagaatacctccaatttggttggtcactgatattccagctaccacaggtgcaagttttgggcaagaaattgtgtgctatgaaagtccaaggccaacaatgggaatacatcgctttgtattcgtattgtttagacaattgggtcgacagacagtgtatgctccaggatggcgtcagaatttcaatacaaaagactttgctgaactctataatcttggtttaccggttgctgccgtctattttaattgtcaaagagagagtggcagtggtggacgtagaaggtctgccgattgatgacatgcttttttaa

SEQ ID NO: 91 - DNA, 535 bp, synthetic construct
  source 1..535: mol_type = other DNA
atgccaagagaacgtgaacctctggtagttggtcgagtgataggggatgtattggaccctttcacaagatctattggcctaagagttatttatagggatagagaagttaataatgggtgtgagcttaggccttcccaagttgttaaccagccaagggttgaagttggtggagatgaccttcgtaccttttacactctggttatggtggaccctgatgctccaagtccaagatatccaaatctaagagaatacctccacttggttggtcactgatattccagctaccacaggtgcaagttttgggcaagaaattgtgtgctatgaaagtccaaggccaacaatgggaatacatcgctttgtattcgtattgtttagacaattgggtcgacagacagtgtatgctccaggatggcgtcagaatttcaatacaaaagactttgctgaactctataatcttggtttaccggttgctgccgtctattttaattgtcaaagagagagtggcagtggtggacgtagaaggtctgccgattga

SEQ ID NO: 92 - DNA, 17896 bp, synthetic construct
  source 1..17896: mol_type = other DNA
ggagagcgatcagcttgcatgccggtcgatctagtaacatagatgacaccgcgcgcgataatttatcctagtttgcgcgctatattttgttttctatcgcgtattaaatgtataattgcgggactctaatcataaaaacccatctcataaataacgtcatgcattacatgttaattattacatgcttaacgtaattcaacagaaattatatgataatcatggcaagaccggcaacaggattcaatcttaagaaactttattgccaaatgtttgaacgatctgcttgactctagctagagtccgaaccccagagtcccgctcagaagaactcgtcaagaaggcgatagaaggctatgcgctgcgaatcgggagcggcgataccgtaaagcacgaggaagcggtcagcccattcgccgccaagctcttcagcaatatcacgggtagccaacgctatgtcctgatagcggtccgccacacccagccggccacagtcgatgaatccagaaaagcggccattttccaccatgatattcggcaagcaggcgtcgccgtgggtcacgacgagatcctcgccgtcgggcatccgcgccttgagcctggcgaacagttcggctggcgcgagcccctgatgctcttcgtccagatcatcctgatcgacaagaccggcttccatccgagtacgtgctcgctcgatgcggtgtttcgcttggtggtcgaatgggcaggtagccggatcaagcgtatgcagccgccgcattgcatcagccatgatggatactttctcggcaggagcaaggtgagatgacaggagatcctgccccggcacttcgcccaatagcagccagtcccttcccgcttcagtgacaacgtcgagcacagctgcgcaaggaacgcccgtcgtggccagccacgatagccgcgctgcctcgtcttggagttcattcagggcaccggacaggtcggtcttgacaaaaagaaccgggcgcccctgcgctgacagccggaacacggcggcatcagagcagccgattgtctgttgtgcccagtcatagccgaatagcctctccacccaagcggccggagaacctgcgtgcaatccatcttgttcaatcatgcctcgatcgagttgagagtgaatatgagactctaattggataccgaggggaatttatggaacgtcagtggagcatttttgacaagaaatatttgctagctgatagtgaccttaggcgacttttgaacgcgcaataatggtttctgacgtatgtgcttagctcattaaactccagaaacccgcggctgagtggctccttcaacgttgcggttctgtcagttccaaacgtaaaacggcttgtcccgcgtcatcggcgggggtcataacgtgactcccttaattctcatgtatctccgtcaggagactagagccaagctgatctcctttgccccggagatcaccatggacgactttctctatctctacgatctaggaagaaagttcgacggagaaggtgacgataccatgttcaccaccgataatgagaagattagcctcttcaatttcagaaagaatgctgacccacagatggttagagaggcctacgcggcaggtctgatcaagacgatctacccgagtaataatctccaggagatcaaataccttcccaagaaggttaaagatgcagtcaaaagattcaggactaactgcatcaagaacacagagaaagatatatttctcaagatcagaagtactattccagtatggacgattcaaggcttgcttcataaaccaaggcaagtaatagagattggagtctctaagaaagtagttcctactgaatcaaaggccatggagtcaaaaattcagatcgaggatctaacagaactcgccgtgaagactggcgaacagttcatacagagtcttttacgactcaatgacaagaagaaaatcttcgtcaacatggtggagcacgacactctcgtctactccaagaatatcaaagatacagtctcagaagaccaaagggctattgagacttttcaacaaagggtaatatcgggaaacctcctcggattccattgcccagctatctgtcacttcatcaaaaggacagtagaaaaggaaggtggcacctacaaatgccatcattgcgataaaggaaaggctatcgttcaagatgcctctgccgacagtggtcccaaagatggacccccacccacgaggagcatcgtggaaaaagaagacgttccaaccacgtcttcaaagcaagtggattgatgtgatatctccactgacgtaagggatgacgcacaatcccactatccttcgcaagacccttcctctatataaggaagttcatttcatttggagaggactccggtatttttacaacaataccacaacaaaacaaacaacaaacaacattacaatttactattctagtcgaaatggacaagaagtactccattgggctcgatatcggcacaaacagcgtcggctgggccgtcattacggacgagtacaaggtgccgagcaaaaaattcaaagttctgggcaataccgatcgccacagcataaagaagaacctcattggcgccctcctgttcgactccggggaaacggccgaagccacgcggctcaaaagaacagcacggcgcagatatacccgcagaaagaatcggatctgctacctgcaggagatctttagtaatgagatggctaaggtggatgactctttcttccataggctggaggagtcctttttggtggaggaggataaaaagcacgagcgccacccaatctttggcaatatcgtggacgaggtggcgtaccatgaaaagtacccaaccatatatcatctgaggaagaagcttgtagacagtactgataaggctgacttgcggttgatctatctcgcgctggcgcatatgatcaaatttcggggacacttcctcatcgagggggacctgaacccagacaacagcgatgtcgacaaactctttatccaactggttcagacttacaatcagcttttcgaagagaacccgatcaacgcatccggagttgacgccaaagcaatcctgagcgctaggctgtccaaatcccggcggctcgaaaacctcatcgcacagctccctggggagaagaagaacggcctgtttggtaatcttatcgccctgtcactcgggctgacccccaactttaaatctaacttcgacctggccgaagatgccaagcttcaactgagcaaagacacctacgatgatgatctcgacaatctgctggcccagatcggcgaccagtacgcagacctttttttggcggcaaagaacctgtcagacgccattctgctgagtgatattctgcgagtgaacacggagatcaccaaagctccgctgagcgctagtatgatcaagcgctatgatgagcaccaccaagacttgactttgctgaaggcccttgtcagacagcaactgcctgagaagtacaaggaaattttcttcgatcagtctaaaaatggctacgccggatacattgacggcggagcaagccaggaggaattttacaaatttattaagcccatcttggaaaaaatggacggcaccgaggagctgctggtaaagcttaacagagaagatctgttgcgcaaacagcgcactttcgacaatggaagcatcccccaccagattcacctgggcgaactgcacgctatcctcaggcggcaagaggatttctacccctttttgaaagataacagggaaaagattgagaaaatcctcacatttcggataccctactatgtaggccccctcgcccggggaaattccagattcgcgtggatgactcgcaaatcagaagagactatcactccctggaacttcgaggaagtcgtggataagggggcctctgcccagtccttcatcgaaaggatgactaactttgataaaaatctgcctaacgaaaaggtgcttcctaaacactctctgctgtacgagtacttcacagtttataacgagctcaccaaggtcaaatacgtcacagaagggatgagaaagccagcattcctgtctggagagcagaagaaagctatcgtggacctcctcttcaagacgaaccggaaagttaccgtgaaacagctcaaagaagattatttcaaaaagattgaatgtttcgactctgttgaaatcagcggagtggaggatcgcttcaacgcatccctgggaacgtatcacgatctcctgaaaatcattaaagacaaggacttcctggacaatgaggagaacgaggacattcttgaggacattgtcctcacccttacgttgtttgaagatagggagatgattgaagaacgcttgaaaacttacgctcatctcttcgacgacaaagtcatgaaacagctcaagaggcgccgatatacaggatgggggcggctgtcaagaaaactgatcaatgggatccgagacaagcagagtggaaagacaatcctggattttcttaagtccgatggatttgccaaccggaacttcatgcagttgatccatgatgactctctcacctttaaggaggacatccagaaagcacaagtttctggccagggggacagtctccacgagcacatcgctaatcttgcaggtagcccagctatcaaaaagggaatactgcagaccgttaaggtcgtggatgaactcgtcaaagtaatgggaaggcataagcccgagaatatcgttatcgagatggcccgagagaaccaaactacccagaagggacagaagaacagtagggaaaggatgaagaggattgaagagggtataaaagaactggggtcccaaatccttaaggaacacccagttgaaaacacccagcttcagaatgagaagctctacctgtactacctgcagaacggcagggacatgtacgtggatcaggaactggacatcaatcggctctccgactacgacgtggatcatatcgtgccccagtcttttctcaaagatgattctattgataataaagtgttgacaagatccgataaaaatagagggaagagtgataacgtcccctcagaagaagttgtcaagaaaatgaaaaattattggcggcagctgctgaacgccaaactgatcacacaacggaagttcgataatctgactaaggctgaacgaggtggcctgtctgagttggataaagccggcttcatcaaaaggcagcttgttgagacacgccagatcaccaagcacgtggcccaaattctcgattcacgcatgaacaccaagtacgatgaaaatgacaaactgattcgagaggtgaaagttattactctgaagtctaagctggtttcagatttcagaaaggactttcagttttataaggtgagagagatcaacaattaccaccatgcgcatgatgcctacctgaatgcagtggtaggcactgcacttatcaaaaaatatcccaagcttgaatctgaatttgtttacggagactataaagtgtacgatgttaggaaaatgatcgcaaagtctgagcaggaaataggcaaggccaccgctaagtacttcttttacagcaatattatgaattttttcaagaccgagattacactggccaatggagagattcggaagcgaccacttatcgaaacaaacggagaaacaggagaaatcgtgtgggacaagggtagggatttcgcgacagtccggaaggtcctgtccatgccgcaggtgaacatcgttaaaaagaccgaagtacagaccggaggcttctccaaggaaagtatcctcccgaaaaggaacagcgacaagctgatcgcacgcaaaaaagattgggaccccaagaaatacggcggattcgattctcctacagtcgcttacagtgtactggttgtggccaaagtggagaaagggaagtctaaaaaactcaaaagcgtcaaggaactgctgggcatcacaatcatggagcgatcaagcttcgaaaaaaaccccatcgactttctcgaggcgaaaggatataaagaggtcaaaaaagacctcatcattaagcttcccaagtactctctctttgagcttgaaaacggccggaaacgaatgctcgctagtgcgggcgagctgcagaaaggtaacgagctggcactgccctctaaatacgttaatttcttgtatctggccagccactatgaaaagctcaaaggatctcccgaagataatgagcagaagcagctgttcgtggaacaacacaaacactaccttgatgagatcatcgagcaaataagcgaattctccaaaagagtgatcctcgccgacgctaacctcgataaggtgctttctgcttacaataagcacagggataagcccatcagggagcaggcagaaaacattatccacttgtttactctgaccaacttgggcgcgcctgcagccttcaagtacttcgacaccaccatagacagaaagcggtacacctctacaaaggaggtcctggacgccacactgattcatcagtcaattacggggctctatgaaacaagaatcgacctctctcagctcggtggagacagcagggctgaccccaagaagaagaggaaggtgtgagcttggaatggatcttcgatcccgatcgttcaaacatttggcaataaagtttcttaagattgaatcctgttgccggtcttgcgacgattatcatataatttctgttgaattacgttaagcatgtaataattaacatgtaatgcatgacgttatttatgagatgggtttttatgattagagtcccgcaattatacatttaatacgcgatagaaaacaaaatatagcgcgcaaactaggataaattatcgcgcdcggtgtcatctatgttactagatcgggaattgccaagctaattcttgaagacgaaagggcctcgtgatacgcctatttttataggttaatgtcatgataataatggtttcttagacgtcaggtggcacttttcggggaaatgtgcgcggaacccctatttgtttatttttctaaatacattcaaatatgtatccgctcatgagacaataaccctgataaatgcttcaataatgggaccgactcgcgctgtcaggagactagagccaagctgatctcctttgccccggagatcaccatggacgactttctctatctctacgatctaggaagaaagttcgacggagaaggtgacgataccatgttcaccaccgataatgagaagattagcctcttcaatttcagaaagaatgctgacccacagatggttagagaggcctacgcggcaggtctgatcaagacgatctacccgagtaataatctccaggagatcaaataccttcccaagaaggttaaagatgcagtcaaaagattcaggactaactgcatcaagaacacagagaaagatatatttctcaagatcagaagtactattccagtatggacgattcaaggcttgcttcataaaccaaggcaagtaatagagattggagtctctaagaaagtagttcctactgaatcaaaggccatggagtcaaaaattcagatcgaggatctaacagaactcgccgtgaagactggcgaacagttcatacagagtcttttacgactcaatgacaagaagaaaatcttcgtcaacatggtggagcacgacactctcgtctactccaagaatatcaaagatacagtctcagaagaccaaagggctattgagacttttcaacaaagggtaatatcgggaaacctcctcggattccattgcccagctatctgtcacttcatcaaaaggacagtagaaaaggaaggtggcacctacaaatgccatcattgcgataaaggaaaggctatcgttcaagatgcctctgccgacagtggtcccaaagatggacccccacccacgaggagcatcgtggaaaaagaagacgttccaaccacgtcttcaaagcaagtggattgatgtgatatctccactgacgtaagggatgacgcacaatcccactatccttcgcaagacccttcctctatataaggaagttcatttcatttggagaggactccggtatttttacaacaataccacaacaaaacaaacaacaaacaacattacaatttactattctagtcgaaatggcctcctccgagaacgtcatcaccgagttcatgcgcttcaaggtgcgcatggagggcaccgtgaacggccacgagttcgagatcgagggcgagggcgagggccgcccctacgagggccacaacaccgtgaagctgaaggtgaccaagggcggccccctgcccttcgcctgggacatcctgtccccccagttccagtacggctccaaggtgtacgtgaagcaccccgccgacatccccgactacaagaagctgtccttccccgagggcttcaagtgggagcgcgtgatgaacttcgaggacggcggcgtggcgaccgtgacccaggactcctccctgcaggacggctgcttcatctacaaggtgaagttcatcggcgtgaacttcccctccgacggccccgtgatgcagaagaagacgatgggctgggaggcctccaccgagcgcctgtacccccgcgacggcgtgctgaagggcgagacacacaaggccctgaagctgaaggacggcggccactacctggtggagttcaagtccatctacatggccaagaagcccgtgcagctgcccggctactactacgtggacgccaagctggacatcacctcccacaacgaggactacaccatcgtggagcagtacgagcgcaccgagggccgccaccacctgttcctgtaggcttcggccatgctagagtccgcaaaaatcaccagtctctctctacaaatctatctctctctatttttctccagaataatgtgtgagtagttcccagataagggaattagggttcttatagggtttcgctcatgtgttgagcatataagaaacccttagtatgtatttgtatttgtaaaatacttctatcaataaaatttctaattcctaaaaccaaaatccagtgacctcgctgtcaggagtctcaatggtaactttactctttatttaaccatacatttttttttatttttttcactttgttcttcatccactattgttctttgttcatcttgaacaaaagctccctccttctttgttcttcatccaccattgttcttcatcaatcatttcgctgtcaggagcatcttcattcttaagatatgaagataatcttcaaaaggcccctgggaatctgaaagaagagaagcaggcccatttatatgggaaagaacaatagtatttcttatataggcccatttaagttgaaaacaatcttcaaaagtcccacatcgcttagataagaaaacgaagctgagtttatatacagctagagtcgaagtagtgattgaacaaagcaccagtggtctagtggtagaatagtaccctgccacggtacagacccgggttcgattcccggctggtgcacttctgttcagaatgtgcacgttttagagctagaaatagcaagttaaaataaggctagtccgttatcaacttgaaaaagtggcaccgagtcggtgcaacaaagcaccagtggtctagtggtagaatagtaccctgccacggtacagacccgggttcgattcccggctggtgcaaaggaaaaagaagttgccgcgttttagagctagaaatagcaagttaaaataaggctagtccgttatcaacttgaaaaagtggcaccgagtcggtgcaacaaagcaccagtggtctagtggtagaatagtaccctgccacggtacagacccgggttcgattcccggctggtgcacgattagacaaaagagatccgttttagagctagaaatagcaagttaaaataaggctagtccgttatcaacttgaaaaagtggcaccgagtcggtgctttttttctagacccagctttcttgtacaaagttggcattacgctgtcaggagcatcttcattcttaagatatgaagataatcttcaaaaggcccctgggaatctgaaagaagagaagcaggcccatttatatgggaaagaacaatagtatttcttatataggcccatttaagttgaaaacaatcttcaaaagtcccacatcgcttagataagaaaacgaagctgagtttatatacagctagagtcgaagtagtgattgaacaaagcaccagtggtctagtggtagaatagtaccctgccacggtacagacccgggttcgattcccggctggtgcacatgtgattctcctggagaagttttagagctagaaatagcaagttaaaataaggctagtccgttatcaacttgaaaaagtggcaccgagtcggtgcaacaaagcaccagtggtctagtggtagaatagtaccctgccacggtacagacccgggttcgattcccggctggtgcagaaattcacagaccttgtgggttttagagctagaaatagcaagttaaaataaggctagtccgttatcaacttgaaaaagtggcaccgagtcggtgcaacaaagcaccagtggtctagtggtagaatagtaccctgccacggtacagacccgggttcgattcccggctggtgcagaaactcgcacaccttgtgggttttagagctagaaatagcaagttaaaataaggctagtccgttatcaacttgaaaaagtggcaccgagtcggtgctttttttctagacccagctttcttgtacaaagttggcattacgctgtcaggagcatcttcattcttaagatatgaagataatcttcaaaaggcccctgggaatctgaaagaagagaagcaggcccatttatatgggaaagaacaatagtatttcttatataggcccatttaagttgaaaacaatcttcaaaagtcccacatcgcttagataagaaaacgaagctgagtttatatacagctagagtcgaagtagtgattgaacaaagcaccagtggtctagtggtagaatagtaccctgccacggtacagacccgggttcgattcccggctggtgcaaatcatatgaagttttacgggttttagagctagaaatagcaagttaaaataaggctagtccgttatcaacttgaaaaagtggcaccgagtcggtgcaacaaagcaccagtggtctagtggtagaatagtaccctgccacggtacagacccgggttcgattcccggctggtgcagagggtcaagtactactcaagttttagagctagaaatagcaagttaaaataaggctagtccgttatcaacttgaaaaagtggcaccgagtcggtgcaacaaagcaccagtggtctagtggtagaatagtaccctgccacggtacagacccgggttcgattcccggctggtgcagtttggctggacacaacgaagttttagagctagaaatagcaagttaaaataaggctagtccgttatcaacttgaaaaagtggcaccgagtcggtgctttttttctagacccagctttcttgtacaaagttggcattacgctgtcatgagacgaattctgacaggatatattggcgggtaaacctaagagaaaagagcgtttattagaataatcggatatttaaaagggcgtgaaaaggtttatccgttcgtccatttgtatgtgcatgccaaccacagggttcccctcgggatcaaagtactttgatccaacccctccgctgctatagtgcagtcggcttctgacgttcagtgcagccgtcatctgaaaacgacatgtcgcacaagtcctaagttacgcgacaggctgccgccctgcccttttcctggcgttttcttgtcgcgtgttttagtcgcataaagtagaatacttgcgactagaaccggagacattacgccatgaacaagagcgccgccgctggcctgctgggctatgcccgcgtcagcaccgacgaccaggacttgaccaaccaacgggccgaactgcacgcggccggctgcaccaagctgttttccgagaagatcaccggcaccaggcgcgaccgcccggagctggccaggatgcttgaccacctacgccctggcgacgttgtgacagtgaccaggctagaccgcctggcccgcagcacccgcgacctactggacattgccgagcgcatccaggaggccggcgcgggcctgcgtagcctggcagagccgtgggccgacaccaccacgccggccggccgcatggtgttgaccgtgttcgccggcattgccgagttcgagcgttccctaatcatcgaccgcacccggagcgggcgcgaggccgccaaggcccgaggcgtgaagtttggcccccgccctaccctcaccccggcacagatcgcgcacgcccgcgagctgatcgaccaggaaggccgcaccgtgaaagaggcggctgcactgcttggcgtgcatcgctcgaccctgtaccgcgcacttgagcgcagcgaggaagtgacgcccaccgaggccaggcggcgcggtgccttccgtgaggacgcattgaccgaggccgacgccctggcggccgccgagaatgaacgccaagaggaacaagcatgaaaccgcaccaggacggccaggacgaaccgtttttcattaccgaagagatcgaggcggagatgatcgcggccgggtacgtgttcgagccgcccgcgcacctctcaaccgtgcggctgcatgaaatcctggccggtttgtctgatgccaagctggcggcctggccggccagcttggccgctgaagaaaccgagcgccgccgtctaaaaaggtgatgtgtatttgagtaaaacagcttgcgtcatgcggtcgctgcgtatatgatccgatgagtaaataaacaaatacgcaaggggaacgcatgaaggttatcgctgtacttaaccagaaaggcgggtcaggcaagacgaccatcggaacccatctagcccgcgccctgcaactcgccggggccgatgttctgttagtcgattccgatccccagggcagtgcccgcgattgggcggccgtgcgggaagatcaaccgctaaccgttgtcggcatcgaccgcccgacgattgaccgcgacgtgaaggccatcggccggcgcgacttcgtagtgatcgacggagcgccccaggcggcggacttggctgtgtccgcgatcaaggcagccgacttcgtgctgattccggtgcagccaagcccttacgacatatgggccaccgccgacctggtggagctggttaagcagcgcattgaggtcacggatggaaggctacaagcggcctttgtcgtgtcgcgggcgatcaaaggcacgcgcatcggcggtgaggttgccgaggcgctggccgggtacgagctgcccattcttgagtcccgtatcacgcagcgcgtgagctacccaggcactgccgccgccggcacaaccgttcttgaatcagaacccgagggcgacgctgcccgcgaggtccaggcgctggccgctgaaattaaatcaaaactcatttgagttaatgaggtaaagagaaaatgagcaaaagcacaaacacgctaagtgccggccgtccgagcgcacgcagcagcaaggctgcaacgttggccagcctggcagacacgccagccatgaagcgggtcaactttcagttgccggcggaggatcacaccaagctgaagatgtacgcggtacgccaaggcaagaccattaccgagctgctatctgaatagatcgcgcagctaccagagtaaatgagcaaatgaataaatgagtagatgaattttagcggctaaaggaggcggcatggaaaatcaagaacaaccaggcaccgacgccgtggaatgccccatgtgtggaggaacgggcggttggccaggcgtaagcggctgggttgtctgccggccctgcaatggcactggaacccccaagcccgaggaatcggcgtgacggtcgcaaaccatccggcccggtacaaatcggcgcggcgctgggtgatgacctggtggagaagttgaaggccgcgcaggccgcccagcggcaacgcatcgaggcagaagcacgccccggtgaatcgtggcaagcggccgctgatcgaatccgcaaagaatcccggcaaccgccggcagccggtgcgccgtcgattaggaagccgcccaagggcgacgagcaaccagattttttcgttccgatgctctatgacgtgggcacccgcgatagtcgcagcatcatggacgtggccgttttccgtctgtcgaagcgtgaccgacgagctggcgaggtgatccgctacgagcttccagacgggcacgtagaggtttccgcagggccggccggcatggccagtgtgtgggattacgacctggtactgatggcggtttcccatctaaccgaatccatgaaccgataccgggaagggaagggagacaagcccggccgcgtgttccgtccacacgttgcggacgtactcaagttctgccggcgagccgatggcggaaagcagaaagacgacctggtagaaacctgcattcggttaaacaccacgcacgttgccatgcagcgtacgaagaaggccaagaacggccgcctggtgacggtatccgagggtgaagccttgattagccgctacaagatcgtaaagagcgaaaccgggcggccggagtacatcgagatcgagctagctgattggatgtaccgcgagatcacagaaggcaagaacccggacgtgctgacggttcaccccgattactttttgatcgatcccggcatcggccgttttctctaccgcctggcacgccgcgccgcaggcaaggcagaagccagatggttgttcaagacgatctacgaacgcagtggcagcgccggagagttcaagaagttctgtttcaccgtgcgcaagctgatcgggtcaaatgacctgccggagtacgatttgaaggaggaggcggggcaggctggcccgatcctagtcatgcgctaccgcaacctgatcgagggcgaagcatccgccggttcctaatgtacggagcagatgctagggcaaattgccctagcaggggaaaaaggtcgaaaaggactctttcctgtggatagcacgtacattgggaacccaaagccgtacattgggaaccggaacccgtacattgggaacccaaagccgtacattgggaaccggtcacacatgtaagtgactgatataaaagagaaaaaaggcgatttttccgcctaaaactctttaaaacttattaaaactcttaaaacccgcctggcctgtgcataactgtctggccagcgcacagccgaagagctgcaaaaagcgcctacccttcggtcgctgcgctccctacgccccgccgcttcgcgtcggcctatcgcggccgctggccgctcaaaaatggctggcctacggccaggcaatctaccagggcgcggacaagccgcgccgtcgccactcgaccgccggcgcccacatcaaggcaccctgcctcgcgcgtttcggtgatgacggtgaaaacctctgacacatgcagctcccggtgacggtcacagcttgtctgtaagcggatgccgggagcagacaagcccgtcagggcgcgtcagcgggtgttggcgggtgtcggggcgcagccatgacccagtcacgtagcgatagcggagtgtatactggcttaactatgcggcatcagagcagattgtactgagagtgcaccatatgcggtgtgaaataccgcacagatgcgtaaggagaaaataccgcatcaggcgctcttccgcttcctcgctcactgactcgctgcgctcggtcgttcggctgcggcgagcggtatcagctcactcaaaggcggtaatacggttatccacagaatcaggggataacgcaggaaagaacatgtgagcaaaaggccagcaaaaggccaggaaccgtaaaaaggccgcgttgctggcgtttttccataggctccgcccccctgacgagcatcacaaaaatcgacgctcaagtcagaggtggcgaaacccgacaggactataaagataccaggcgtttccccctggaagctccctcgtgcgctctcctgttccgaccctgccgcttaccggatacctgtccgcctttctcccttcgggaagcgtggcgctttctcatagctcacgctgtaggtatctcagttcggtgtaggtcgttcgctccaagctgggctgtgtgcacgaaccccccgttcagcccgaccgctgcgccttatccggtaactatcgtcttgagtccaacccggtaagacacgacttatcgccactggcagcagccactggtaacaggattagcagagcgaggtatgtaggcggtgctacagagttcttgaagtggtggcctaactacggctacactagaaggacagtatttggtatctgcgctctgctgaagccagttaccttcggaaaaagagttggtagctcttgatccggcaaacaaaccaccgctggtagcggtggtttttttgtttgcaagcagcagattacgcgcagaaaaaaaggatctcaagaagatcctttgatcttttctacggggtctgacgctcagtggaacgaaaactcacgttaagggattttggtcatgcattctaggtgattagaaaaactcatcgagcatcaaatgaaactgcaatttattcatatcaggattatcaataccatatttttgaaaaagccgtttctgtaatgaaggagaaaactcaccgaggcagttccataggatggcaagatcctggtatcggtctgcgattccgactcgtccaacatcaatacaacctattaatttcccctcgtcaaaaataaggttatcaagtgagaaatcaccatgagtgacgactgaatccggtgagaatggcaaaagtttatgcatttctttccagacttgttcaacaggccagccattacgctcgtcatcaaaatcactcgcatcaaccaaaccgttattcattcgtgattgcgcctgagcgagtcgaaatacgcgatcgctgttaaaaggacaattacaaacaggaatcgaatgcaaccggcgcaggaacactgccagcgcatcaacaatattttcacctgaatcaggatattcttctaatacctggaatgctgttttccctgggatcgcagtggtgagtaaccatgcatcatcaggagtacggataaaatgcttgatggtcggaagaggcataaattccgtcagccagtttagtctgaccatctcatctgtaacatcattggcaacgctacctttgccatgtttcagaaacaactctggcgcatcgggcttcccatacaatcggtagattgtcgcacctgattgcccgacattatcgcgagcccatttatacccatataaatcagcatccatgttggaatttaatcgcggccttgagcaagacgtttcccgttgaatatggctcataacagaacttattatttccttcctcttttctacagtatttaaagataccccaagaagctaattataacaagacgaactccaattcactgttccttgcattctaaaaccttaaataccagaaaacagctttttcaaagttgttttcaaagttggcgtataacatagtatcgacggagccgattttgaaaccgcggtgatcacaggcagcaacgctctgtcatcgttacaatcaacatgctaccctccgcgagatcatccgtgtttcaaacccggcagcttagttgccgttcttccgaatagcatcggtaacatgagcaaagtctgccgccttacaacggctctcccgctgacgccgtcccggactgatgggctgcctgtatcgagtggtgattttgtgccgagctgccggtcggggagctgttggctggctggtggcaggatatattgtggtgtaaacataacgaattcgtctca

SEQ ID NO: 93 - DNA, 19773 bp, synthetic construct
  source 1..19773: mol_type = other DNA
ggagagcgatcagcttgcatgccggtcgatctagtaacatagatgacaccgcgcgcgataatttatcctagtttgcgcgctatattttgttttctatcgcgtattaaatgtataattgcgggactctaatcataaaaacccatctcataaataacgtcatgcattacatgttaattattacatgcttaacgtaattcaacagaaattatatgataatcatggcaagaccggcaacaggattcaatcttaagaaactttattgccaaatgtttgaacgatctgcttgactctagctagagtccgaaccccagagtcccgctcagaagaactcgtcaagaaggcgatagaaggctatgcgctgcgaatcgggagcggcgataccgtaaagcacgaggaagcggtcagcccattcgccgccaagctcttcagcaatatcacgggtagccaacgctatgtcctgatagcggtccgccacacccagccggccacagtcgatgaatccagaaaagcggccattttccaccatgatattcggcaagcaggcgtcgccgtgggtcacgacgagatcctcgccgtcgggcatccgcgccttgagcctggcgaacagttcggctggcgcgagcccctgatgctcttcgtccagatcatcctgatcgacaagaccggcttccatccgagtacgtgctcgctcgatgcggtgtttcgcttggtggtcgaatgggcaggtagccggatcaagcgtatgcagccgccgcattgcatcagccatgatggatactttctcggcaggagcaaggtgagatgacaggagatcctgccccggcacttcgcccaatagcagccagtcccttcccgcttcagtgacaacgtcgagcacagctgcgcaaggaacgcccgtcgtggccagccacgatagccgcgctgcctcgtcttggagttcattcagggcaccggacaggtcggtcttgacaaaaagaaccgggcgcccctgcgctgacagccggaacacggcggcatcagagcagccgattgtctgttgtgcccagtcatagccgaatagcctctccacccaagcggccggagaacctgcgtgcaatccatcttgttcaatcatgcctcgatcgagttgagagtgaatatgagactctaattggataccgaggggaatttatggaacgtcagtggagcatttttgacaagaaatatttgctagctgatagtgaccttaggcgacttttgaacgcgcaataatggtttctgacgtatgtgcttagctcattaaactccagaaacccgcggctgagtggctccttcaacgttgcggttctgtcagttccaaacgtaaaacggcttgtcccgcgtcatcggcgggggtcataacgtgactcccttaattctcatgtatctccgtcaggagactagagccaagctgatctcctttgccccggagatcaccatggacgactttctctatctctacgatctaggaagaaagttcgacggagaaggtgacgataccatgttcaccaccgataatgagaagattagcctcttcaatttcagaaagaatgctgacccacagatggttagagaggcctacgcggcaggtctgatcaagacgatctacccgagtaataatctccaggagatcaaataccttcccaagaaggttaaagatgcagtcaaaagattcaggactaactgcatcaagaacacagagaaagatatatttctcaagatcagaagtactattccagtatggacgattcaaggcttgcttcataaaccaaggcaagtaatagagattggagtctctaagaaagtagttcctactgaatcaaaggccatggagtcaaaaattcagatcgaggatctaacagaactcgccgtgaagactggcgaacagttcatacagagtcttttacgactcaatgacaagaagaaaatcttcgtcaacatggtggagcacgacactctcgtctactccaagaatatcaaagatacagtctcagaagaccaaagggctattgagacttttcaacaaagggtaatatcgggaaacctcctcggattccattgcccagctatctgtcacttcatcaaaaggacagtagaaaaggaaggtggcacctacaaatgccatcattgcgataaaggaaaggctatcgttcaagatgcctctgccgacagtggtcccaaagatggacccccacccacgaggagcatcgtggaaaaagaagacgttccaaccacgtcttcaaagcaagtggattgatgtgatatctccactgacgtaagggatgacgcacaatcccactatccttcgcaagacccttcctctatataaggaagttcatttcatttggagaggactccggtatttttacaacaataccacaacaaaacaaacaacaaacaacattacaatttactattctagtcgaaatggacaagaagtactccattgggctcgatatcggcacaaacagcgtcggctgggccgtcattacggacgagtacaaggtgccgagcaaaaaattcaaagttctgggcaataccgatcgccacagcataaagaagaacctcattggcgccctcctgttcgactccggggaaacggccgaagccacgcggctcaaaagaacagcacggcgcagatatacccgcagaaagaatcggatctgctacctgcaggagatctttagtaatgagatggctaaggtggatgactctttcttccataggctggaggagtcctttttggtggaggaggataaaaagcacgagcgccacccaatctttggcaatatcgtggacgaggtggcgtaccatgaaaagtacccaaccatatatcatctgaggaagaagcttgtagacagtactgataaggctgacttgcggttgatctatctcgcgctggcgcatatgatcaaatttcggggacacttcctcatcgagggggacctgaacccagacaacagcgatgtcgacaaactctttatccaactggttcagacttacaatcagcttttcgaagagaacccgatcaacgcatccggagttgacgccaaagcaatcctgagcgctaggctgtccaaatcccggcggctcgaaaacctcatcgcacagctccctggggagaagaagaacggcctgtttggtaatcttatcgccctgtcactcgggctgacccccaactttaaatctaacttcgacctggccgaagatgccaagcttcaactgagcaaagacacctacgatgatgatctcgacaatctgctggcccagatcggcgaccagtacgcagacctttttttggcggcaaagaacctgtcagacgccattctgctgagtgatattctgcgagtgaacacggagatcaccaaagctccgctgagcgctagtatgatcaagcgctatgatgagcaccaccaagacttgactttgctgaaggcccttgtcagacagcaactgcctgagaagtacaaggaaattttcttcgatcagtctaaaaatggctacgccggatacattgacggcggagcaagccaggaggaattttacaaatttattaagcccatcttggaaaaaatggacggcaccgaggagctgctggtaaagcttaacagagaagatctgttgcgcaaacagcgcactttcgacaatggaagcatcccccaccagattcacctgggcgaactgcacgctatcctcaggcggcaagaggatttctacccctttttgaaagataacagggaaaagattgagaaaatcctcacatttcggataccctactatgtaggccccctcgcccggggaaattccagattcgcgtggatgactcgcaaatcagaagagactatcactccctggaacttcgaggaagtcgtggataagggggcctctgcccagtccttcatcgaaaggatgactaactttgataaaaatctgcctaacgaaaaggtgcttcctaaacactctctgctgtacgagtacttcacagtttataacgagctcaccaaggtcaaatacgtcacagaagggatgagaaagccagcattcctgtctggagagcagaagaaagctatcgtggacctcctcttcaagacgaaccggaaagttaccgtgaaacagctcaaagaagattatttcaaaaagattgaatgtttcgactctgttgaaatcagcggagtggaggatcgcttcaacgcatccctgggaacgtatcacgatctcctgaaaatcattaaagacaaggacttcctggacaatgaggagaacgaggacattcttgaggacattgtcctcacccttacgttgtttgaagatagggagatgattgaagaacgcttgaaaacttacgctcatctcttcgacgacaaagtcatgaaacagctcaagaggcgccgatatacaggatgggggcggctgtcaagaaaactgatcaatgggatccgagacaagcagagtggaaagacaatcctggattttcttaagtccgatggatttgccaaccggaacttcatgcagttgatccatgatgactctctcacctttaaggaggacatccagaaagcacaagtttctggccagggggacagtctccacgagcacatcgctaatcttgcaggtagcccagctatcaaaaagggaatactgcagaccgttaaggtcgtggatgaactcgtcaaagtaatgggaaggcataagcccgagaatatcgttatcgagatggcccgagagaaccaaactacccagaagggacagaagaacagtagggaaaggatgaagaggattgaagagggtataaaagaactggggtcccaaatccttaaggaacacccagttgaaaacacccagcttcagaatgagaagctctacctgtactacctgcagaacggcagggacatgtacgtggatcaggaactggacatcaatcggctctccgactacgacgtggatcatatcgtgccccagtcttttctcaaagatgattctattgataataaagtgttgacaagatccgataaaaatagagggaagagtgataacgtcccctcagaagaagttgtcaagaaaatgaaaaattattggcggcagctgctgaacgccaaactgatcacacaacggaagttcgataatctgactaaggctgaacgaggtggcctgtctgagttggataaagccggcttcatcaaaaggcagcttgttgagacacgccagatcaccaagcacgtggcccaaattctcgattcacgcatgaacaccaagtacgatgaaaatgacaaactgattcgagaggtgaaagttattactctgaagtctaagctggtttcagatttcagaaaggactttcagttttataaggtgagagagatcaacaattaccaccatgcgcatgatgcctacctgaatgcagtggtaggcactgcacttatcaaaaaatatcccaagcttgaatctgaatttgtttacggagactataaagtgtacgatgttaggaaaatgatcgcaaagtctgagcaggaaataggcaaggccaccgctaagtacttcttttacagcaatattatgaattttttcaagaccgagattacactggccaatggagagattcggaagcgaccacttatcgaaacaaacggagaaacaggagaaatcgtgtgggacaagggtagggatttcgcgacagtccggaaggtcctgtccatgccgcaggtgaacatcgttaaaaagaccgaagtacagaccggaggcttctccaaggaaagtatcctcccgaaaaggaacagcgacaagctgatcgcacgcaaaaaagattgggaccccaagaaatacggcggattcgattctcctacagtcgcttacagtgtactggttgtggccaaagtggagaaagggaagtctaaaaaactcaaaagcgtcaaggaactgctgggcatcacaatcatggagcgatcaagcttcgaaaaaaaccccatcgactttctcgaggcgaaaggatataaagaggtcaaaaaagacctcatcattaagcttcccaagtactctctctttgagcttgaaaacggccggaaacgaatgctcgctagtgcgggcgagctgcagaaaggtaacgagctggcactgccctctaaatacgttaatttcttgtatctggccagccactatgaaaagctcaaaggatctcccgaagataatgagcagaagcagctgttcgtggaacaacacaaacactaccttgatgagatcatcgagcaaataagcgaattctccaaaagagtgatcctcgccgacgctaacctcgataaggtgctttctgcttacaataagcacagggataagcccatcagggagcaggcagaaaacattatccacttgtttactctgaccaacttgggcgcgcctgcagccttcaagtacttcgacaccaccatagacagaaagcggtacacctctacaaaggaggtcctggacgccacactgattcatcagtcaattacggggctctatgaaacaagaatcgacctctctcagctcggtggagacagcagggctgaccccaagaagaagaggaaggtgtgagcttggaatggatcttcgatcccgatcgttcaaacatttggcaataaagtttcttaagattgaatcctgttgccggtcttgcgacgattatcatataatttctgttgaattacgttaagcatgtaataattaacatgtaatgcatgacgttatttatgagatgggtttttatgattagagtcccgcaattatacatttaatacgcgatagaaaacaaaatatagcgcgcaaactaggataaattatcgcgcdcggtgtcatctatgttactagatcgggaattgccaagctaattcttgaagacgaaagggcctcgtgatacgcctatttttataggttaatgtcatgataataatggtttcttagacgtcaggtggcacttttcggggaaatgtgcgcggaacccctatttgtttatttttctaaatacattcaaatatgtatccgctcatgagacaataaccctgataaatgcttcaataatgggaccgactcgcgctgtcaggagactagagccaagctgatctcctttgccccggagatcaccatggacgactttctctatctctacgatctaggaagaaagttcgacggagaaggtgacgataccatgttcaccaccgataatgagaagattagcctcttcaatttcagaaagaatgctgacccacagatggttagagaggcctacgcggcaggtctgatcaagacgatctacccgagtaataatctccaggagatcaaataccttcccaagaaggttaaagatgcagtcaaaagattcaggactaactgcatcaagaacacagagaaagatatatttctcaagatcagaagtactattccagtatggacgattcaaggcttgcttcataaaccaaggcaagtaatagagattggagtctctaagaaagtagttcctactgaatcaaaggccatggagtcaaaaattcagatcgaggatctaacagaactcgccgtgaagactggcgaacagttcatacagagtcttttacgactcaatgacaagaagaaaatcttcgtcaacatggtggagcacgacactctcgtctactccaagaatatcaaagatacagtctcagaagaccaaagggctattgagacttttcaacaaagggtaatatcgggaaacctcctcggattccattgcccagctatctgtcacttcatcaaaaggacagtagaaaaggaaggtggcacctacaaatgccatcattgcgataaaggaaaggctatcgttcaagatgcctctgccgacagtggtcccaaagatggacccccacccacgaggagcatcgtggaaaaagaagacgttccaaccacgtcttcaaagcaagtggattgatgtgatatctccactgacgtaagggatgacgcacaatcccactatccttcgcaagacccttcctctatataaggaagttcatttcatttggagaggactccggtatttttacaacaataccacaacaaaacaaacaacaaacaacattacaatttactattctagtcgaaatggcctcctccgagaacgtcatcaccgagttcatgcgcttcaaggtgcgcatggagggcaccgtgaacggccacgagttcgagatcgagggcgagggcgagggccgcccctacgagggccacaacaccgtgaagctgaaggtgaccaagggcggccccctgcccttcgcctgggacatcctgtccccccagttccagtacggctccaaggtgtacgtgaagcaccccgccgacatccccgactacaagaagctgtccttccccgagggcttcaagtgggagcgcgtgatgaacttcgaggacggcggcgtggcgaccgtgacccaggactcctccctgcaggacggctgcttcatctacaaggtgaagttcatcggcgtgaacttcccctccgacggccccgtgatgcagaagaagacgatgggctgggaggcctccaccgagcgcctgtacccccgcgacggcgtgctgaagggcgagacacacaaggccctgaagctgaaggacggcggccactacctggtggagttcaagtccatctacatggccaagaagcccgtgcagctgcccggctactactacgtggacgccaagctggacatcacctcccacaacgaggactacaccatcgtggagcagtacgagcgcaccgagggccgccaccacctgttcctgtaggcttcggccatgctagagtccgcaaaaatcaccagtctctctctacaaatctatctctctctatttttctccagaataatgtgtgagtagttcccagataagggaattagggttcttatagggtttcgctcatgtgttgagcatataagaaacccttagtatgtatttgtatttgtaaaatacttctatcaataaaatttctaattcctaaaaccaaaatccagtgacctcgctgtcaggagtctcaatggtaactttactctttatttaaccatacatttttttttatttttttcactttgttcttcatccactattgttctttgttcatcttgaacaaaagctccctccttctttgttcttcatccaccattgttcttcatcaatcatttcgctgtcaggagtctcaatggtaactttactctttatttaaccatacatttttttttatttttttcactttgttcttcatccactattgttctttgttcatcttgaacaaaagctccctccttctttgttcttcatccaccattgttcttcatcaatcatttcgctgtcaggagcatcttcattcttaagatatgaagataatcttcaaaaggcccctgggaatctgaaagaagagaagcaggcccatttatatgggaaagaacaatagtatttcttatataggcccatttaagttgaaaacaatcttcaaaagtcccacatcgcttagataagaaaacgaagctgagtttatatacagctagagtcgaagtagtgattgaacaaagcaccagtggtctagtggtagaatagtaccctgccacggtacagacccgggttcgattcccggctggtgcacgacggcttgagactttgcagttttagagctagaaatagcaagttaaaataaggctagtccgttatcaacttgaaaaagtggcaccgagtcggtgcaacaaagcaccagtggtctagtggtagaatagtaccctgccacggtacagacccgggttcgattcccggctggtgcaaatcgaaaaggagttgcagggttttagagctagaaatagcaagttaaaataaggctagtccgttatcaacttgaaaaagtggcaccgagtcggtgcaacaaagcaccagtggtctagtggtagaatagtaccctgccacggtacagacccgggttcgattcccggctggtgcaaagggtcaagtacttcaatggttttagagctagaaatagcaagttaaaataaggctagtccgttatcaacttgaaaaagtggcaccgagtcggtgcaacaaagcaccagtggtctagtggtagaatagtaccctgccacggtacagacccgggttcgattcccggctggtgcacgacggcttgagcctttgcagttttagagctagaaatagcaagttaaaataaggctagtccgttatcaacttgaaaaagtggcaccgagtcggtgcaacaaagcaccagtggtctagtggtagaatagtaccctgccacggtacagacccgggttcgattcccggctggtgcaggacctcacaaactttatgggttttagagctagaaatagcaagttaaaataaggctagtccgttatcaacttgaaaaagtggcaccgagtcggtgcaacaaagcaccagtggtctagtggtagaatagtaccctgccacggtacagacccgggttcgattcccggctggtgcaatggacataacaggcgtcgagttttagagctagaaatagcaagttaaaataaggctagtccgttatcaacttgaaaaagtggcaccgagtcggtgctttttttctagacccagctttcttgtacaaagttggcattacgctgtcaggagcatcttcattcttaagatatgaagataatcttcaaaaggcccctgggaatctgaaagaagagaagcaggcccatttatatgggaaagaacaatagtatttcttatataggcccatttaagttgaaaacaatcttcaaaagtcccacatcgcttagataagaaaacgaagctgagtttatatacagctagagtcgaagtagtgattgaacaaagcaccagtggtctagtggtagaatagtaccctgccacggtacagacccgggttcgattcccggctggtgcacgaacagttgaaagcaacaggttttagagctagaaatagcaagttaaaataaggctagtccgttatcaacttgaaaaagtggcaccgagtcggtgcaacaaagcaccagtggtctagtggtagaatagtaccctgccacggtacagacccgggttcgattcccggctggtgcatcatcataggaggtgccgaggttttagagctagaaatagcaagttaaaataaggctagtccgttatcaacttgaaaaagtggcaccgagtcggtgcaacaaagcaccagtggtctagtggtagaatagtaccctgccacggtacagacccgggttcgattcccggctggtgcatagaaattcaccccccatgggttttagagctagaaatagcaagttaaaataaggctagtccgttatcaacttgaaaaagtggcaccgagtcggtgcaacaaagcaccagtggtctagtggtagaatagtaccctgccacggtacagacccgggttcgattcccggctggtgcatgtgatcagagagcctcctggttttagagctagaaatagcaagttaaaataaggctagtccgttatcaacttgaaaaagtggcaccgagtcggtgcaacaaagcaccagtggtctagtggtagaatagtaccctgccacggtacagacccgggttcgattcccggctggtgcaggaaaccatccagttcaactgttttagagctagaaatagcaagttaaaataaggctagtccgttatcaacttgaaaaagtggcaccgagtcggtgctttttttctagacccagctttcttgtacaaagttggcattacgctgtcaggagcatcttcattcttaagatatgaagataatcttcaaaaggcccctgggaatctgaaagaagagaagcaggcccatttatatgggaaagaacaatagtatttcttatataggcccatttaagttgaaaacaatcttcaaaagtcccacatcgcttagataagaaaacgaagctgagtttatatacagctagagtcgaagtagtgattgaacaaagcaccagtggtctagtggtagaatagtaccctgccacggtacagacccgggttcgattcccggctggtgcattaaaggggcatcagtccaagttttagagctagaaatagcaagttaaaataaggctagtccgttatcaacttgaaaaagtggcaccgagtcggtgcaacaaagcaccagtggtctagtggtagaatagtaccctgccacggtacagacccgggttcgattcccggctggtgcaatctactttgaaaatgtggggttttagagctagaaatagcaagttaaaataaggctagtccgttatcaacttgaaaaagtggcaccgagtcggtgcaacaaagcaccagtggtctagtggtagaatagtaccctgccacggtacagacccgggttcgattcccggctggtgcagaaattcacagaccttgtgggttttagagctagaaatagcaagttaaaataaggctagtccgttatcaacttgaaaaagtggcaccgagtcggtgcaacaaagcaccagtggtctagtggtagaatagtaccctgccacggtacagacccgggttcgattcccggctggtgcacagtcattccaaatgcccaagttttagagctagaaatagcaagttaaaataaggctagtccgttatcaacttgaaaaagtggcaccgagtcggtgcaacaaagcaccagtggtctagtggtagaatagtaccctgccacggtacagacccgggttcgattcccggctggtgcaagatggagtggaatgcaaaggttttagagctagaaatagcaagttaaaataaggctagtccgttatcaacttgaaaaagtggcaccgagtcggtgcaacaaagcaccagtggtctagtggtagaatagtaccctgccacggtacagacccgggttcgattcccggctggtgcaccttcaacttgacacctagggttttagagctagaaatagcaagttaaaataaggctagtccgttatcaacttgaaaaagtggcaccgagtcggtgctttttttctagacccagctttcttgtacaaagttggcattacgctgtcatgagaccggatcctgacaggatatattggcgggtaaacctaagagaaaagagcgtttattagaataatcggatatttaaaagggcgtgaaaaggtttatccgttcgtccatttgtatgtgcatgccaaccacagggttcccctcgggatcaaagtactttgatccaacccctccgctgctatagtgcagtcggcttctgacgttcagtgcagccgtcatctgaaaacgacatgtcgcacaagtcctaagttacgcgacaggctgccgccctgcccttttcctggcgttttcttgtcgcgtgttttagtcgcataaagtagaatacttgcgactagaaccggagacattacgccatgaacaagagcgccgccgctggcctgctgggctatgcccgcgtcagcaccgacgaccaggacttgaccaaccaacgggccgaactgcacgcggccggctgcaccaagctgttttccgagaagatcaccggcaccaggcgcgaccgcccggagctggccaggatgcttgaccacctacgccctggcgacgttgtgacagtgaccaggctagaccgcctggcccgcagcacccgcgacctactggacattgccgagcgcatccaggaggccggcgcgggcctgcgtagcctggcagagccgtgggccgacaccaccacgccggccggccgcatggtgttgaccgtgttcgccggcattgccgagttcgagcgttccctaatcatcgaccgcacccggagcgggcgcgaggccgccaaggcccgaggcgtgaagtttggcccccgccctaccctcaccccggcacagatcgcgcacgcccgcgagctgatcgaccaggaaggccgcaccgtgaaagaggcggctgcactgcttggcgtgcatcgctcgaccctgtaccgcgcacttgagcgcagcgaggaagtgacgcccaccgaggccaggcggcgcggtgccttccgtgaggacgcattgaccgaggccgacgccctggcggccgccgagaatgaacgccaagaggaacaagcatgaaaccgcaccaggacggccaggacgaaccgtttttcattaccgaagagatcgaggcggagatgatcgcggccgggtacgtgttcgagccgcccgcgcacctctcaaccgtgcggctgcatgaaatcctggccggtttgtctgatgccaagctggcggcctggccggccagcttggccgctgaagaaaccgagcgccgccgtctaaaaaggtgatgtgtatttgagtaaaacagcttgcgtcatgcggtcgctgcgtatatgatccgatgagtaaataaacaaatacgcaaggggaacgcatgaaggttatcgctgtacttaaccagaaaggcgggtcaggcaagacgaccatcggaacccatctagcccgcgccctgcaactcgccggggccgatgttctgttagtcgattccgatccccagggcagtgcccgcgattgggcggccgtgcgggaagatcaaccgctaaccgttgtcggcatcgaccgcccgacgattgaccgcgacgtgaaggccatcggccggcgcgacttcgtagtgatcgacggagcgccccaggcggcggacttggctgtgtccgcgatcaaggcagccgacttcgtgctgattccggtgcagccaagcccttacgacatatgggccaccgccgacctggtggagctggttaagcagcgcattgaggtcacggatggaaggctacaagcggcctttgtcgtgtcgcgggcgatcaaaggcacgcgcatcggcggtgaggttgccgaggcgctggccgggtacgagctgcccattcttgagtcccgtatcacgcagcgcgtgagctacccaggcactgccgccgccggcacaaccgttcttgaatcagaacccgagggcgacgctgcccgcgaggtccaggcgctggccgctgaaattaaatcaaaactcatttgagttaatgaggtaaagagaaaatgagcaaaagcacaaacacgctaagtgccggccgtccgagcgcacgcagcagcaaggctgcaacgttggccagcctggcagacacgccagccatgaagcgggtcaactttcagttgccggcggaggatcacaccaagctgaagatgtacgcggtacgccaaggcaagaccattaccgagctgctatctgaatagatcgcgcagctaccagagtaaatgagcaaatgaataaatgagtagatgaattttagcggctaaaggaggcggcatggaaaatcaagaacaaccaggcaccgacgccgtggaatgccccatgtgtggaggaacgggcggttggccaggcgtaagcggctgggttgtctgccggccctgcaatggcactggaacccccaagcccgaggaatcggcgtgacggtcgcaaaccatccggcccggtacaaatcggcgcggcgctgggtgatgacctggtggagaagttgaaggccgcgcaggccgcccagcggcaacgcatcgaggcagaagcacgccccggtgaatcgtggcaagcggccgctgatcgaatccgcaaagaatcccggcaaccgccggcagccggtgcgccgtcgattaggaagccgcccaagggcgacgagcaaccagattttttcgttccgatgctctatgacgtgggcacccgcgatagtcgcagcatcatggacgtggccgttttccgtctgtcgaagcgtgaccgacgagctggcgaggtgatccgctacgagcttccagacgggcacgtagaggtttccgcagggccggccggcatggccagtgtgtgggattacgacctggtactgatggcggtttcccatctaaccgaatccatgaaccgataccgggaagggaagggagacaagcccggccgcgtgttccgtccacacgttgcggacgtactcaagttctgccggcgagccgatggcggaaagcagaaagacgacctggtagaaacctgcattcggttaaacaccacgcacgttgccatgcagcgtacgaagaaggccaagaacggccgcctggtgacggtatccgagggtgaagccttgattagccgctacaagatcgtaaagagcgaaaccgggcggccggagtacatcgagatcgagctagctgattggatgtaccgcgagatcacagaaggcaagaacccggacgtgctgacggttcaccccgattactttttgatcgatcccggcatcggccgttttctctaccgcctggcacgccgcgccgcaggcaaggcagaagccagatggttgttcaagacgatctacgaacgcagtggcagcgccggagagttcaagaagttctgtttcaccgtgcgcaagctgatcgggtcaaatgacctgccggagtacgatttgaaggaggaggcggggcaggctggcccgatcctagtcatgcgctaccgcaacctgatcgagggcgaagcatccgccggttcctaatgtacggagcagatgctagggcaaattgccctagcaggggaaaaaggtcgaaaaggactctttcctgtggatagcacgtacattgggaacccaaagccgtacattgggaaccggaacccgtacattgggaacccaaagccgtacattgggaaccggtcacacatgtaagtgactgatataaaagagaaaaaaggcgatttttccgcctaaaactctttaaaacttattaaaactcttaaaacccgcctggcctgtgcataactgtctggccagcgcacagccgaagagctgcaaaaagcgcctacccttcggtcgctgcgctccctacgccccgccgcttcgcgtcggcctatcgcggccgctggccgctcaaaaatggctggcctacggccaggcaatctaccagggcgcggacaagccgcgccgtcgccactcgaccgccggcgcccacatcaaggcaccctgcctcgcgcgtttcggtgatgacggtgaaaacctctgacacatgcagctcccggtgacggtcacagcttgtctgtaagcggatgccgggagcagacaagcccgtcagggcgcgtcagcgggtgttggcgggtgtcggggcgcagccatgacccagtcacgtagcgatagcggagtgtatactggcttaactatgcggcatcagagcagattgtactgagagtgcaccatatgcggtgtgaaataccgcacagatgcgtaaggagaaaataccgcatcaggcgctcttccgcttcctcgctcactgactcgctgcgctcggtcgttcggctgcggcgagcggtatcagctcactcaaaggcggtaatacggttatccacagaatcaggggataacgcaggaaagaacatgtgagcaaaaggccagcaaaaggccaggaaccgtaaaaaggccgcgttgctggcgtttttccataggctccgcccccctgacgagcatcacaaaaatcgacgctcaagtcagaggtggcgaaacccgacaggactataaagataccaggcgtttccccctggaagctccctcgtgcgctctcctgttccgaccctgccgcttaccggatacctgtccgcctttctcccttcgggaagcgtggcgctttctcatagctcacgctgtaggtatctcagttcggtgtaggtcgttcgctccaagctgggctgtgtgcacgaaccccccgttcagcccgaccgctgcgccttatccggtaactatcgtcttgagtccaacccggtaagacacgacttatcgccactggcagcagccactggtaacaggattagcagagcgaggtatgtaggcggtgctacagagttcttgaagtggtggcctaactacggctacactagaaggacagtatttggtatctgcgctctgctgaagccagttaccttcggaaaaagagttggtagctcttgatccggcaaacaaaccaccgctggtagcggtggtttttttgtttgcaagcagcagattacgcgcagaaaaaaaggatctcaagaagatcctttgatcttttctacggggtctgacgctcagtggaacgaaaactcacgttaagggattttggtcatgcattctaggtgattatttgccgactaccttggtgatctcgcctttcacgtagtggacaaattcttccaactgatctgcgcgcgaggccaagcgatcttcttcttgtccaagataagcctgtctagcttcaagtatgacgggctgatactgggccggcaggcgctccattgcccagtcggcagcgacatccttcggcgcgattttgccggttactgcgctgtaccaaatgcgggacaacgtaagcactacatttcgctcatcaccagcccagtcgggcggcgagttccatagcgttaaggtttcatttagcgcctcaaatagatcctgttcaggaaccggatcaaagagttcctccgccgctggacctaccaaggcaacgctatgttctcttgcttttgtcagcaagatagccagatcaatgtcgatcgtggctggctcgaagatacctgcaagaatgtcattgcgctgccattctccaaattgcagttcgcgcttagctggataacgccacggaatgatgtcgtcgtgcacaacaatggtgacttctacagcgcggagaatctcgctctctccaggggaagccgaagtttccaaaaggtcgttgatcaaagctcgccgcgttgtttcatcaagccttacggtcaccgtaaccagcaaatcaatatcactgtgtggcttcaggccgccatccactgcggagccgtacaaatgtacggccagcaacgtcggttcgagatggcgctcgatgacgccaactacctctgatagttgagtcgatacttcggcgatcaccgcttccctcataatgtttaactttgttttagggcgactgccctgctgcgtaacatcgttgctgctccataacatcaaacatcgacccacggcgtaacgcgcttgctgcttggatgcccgaggcatagactgtaccccaaaaaaacagtcataacaagccatgaaaaccgccactgcgccgttaccaccgctgcgttcggtcaaggttctggaccagttgcgtgagcgcatacgctacttgcattacagcttacgaaccgaacaggcttatgtccactgggttcgtgccttcatccgtttccacggtgtgcgtcacccggcaaccttgggtagcagcgaagtcgaggcatttctgtcctggctggaacagaacttattatttccttcctcttttctacagtatttaaagataccccaagaagctaattataacaagacgaactccaattcactgttccttgcattctaaaaccttaaataccagaaaacagctttttcaaagttgttttcaaagttggcgtataacatagtatcgacggagccgattttgaaaccgcggtgatcacaggcagcaacgctctgtcatcgttacaatcaacatgctaccctccgcgagatcatccgtgtttcaaacccggcagcttagttgccgttcttccgaatagcatcggtaacatgagcaaagtctgccgccttacaacggctctcccgctgacgccgtcccggactgatgggctgcctgtatcgagtggtgattttgtgccgagctgccggtcggggagctgttggctggctggtggcaggatatattgtggtgtaaacataacggatccggtctca

SEQ ID NO: 94 - DNA, 17190 bp, synthetic construct
  source 1..17190: mol_type = other DNA
ggagagcgatcagcttgcatgccggtcgatctagtaacatagatgacaccgcgcgcgataatttatcctagtttgcgcgctatattttgttttctatcgcgtattaaatgtataattgcgggactctaatcataaaaacccatctcataaataacgtcatgcattacatgttaattattacatgcttaacgtaattcaacagaaattatatgataatcatggcaagaccggcaacaggattcaatcttaagaaactttattgccaaatgtttgaacgatctgcttgactctagctagagtccgaaccccagagtcccgctcagaagaactcgtcaagaaggcgatagaaggctatgcgctgcgaatcgggagcggcgataccgtaaagcacgaggaagcggtcagcccattcgccgccaagctcttcagcaatatcacgggtagccaacgctatgtcctgatagcggtccgccacacccagccggccacagtcgatgaatccagaaaagcggccattttccaccatgatattcggcaagcaggcgtcgccgtgggtcacgacgagatcctcgccgtcgggcatccgcgccttgagcctggcgaacagttcggctggcgcgagcccctgatgctcttcgtccagatcatcctgatcgacaagaccggcttccatccgagtacgtgctcgctcgatgcggtgtttcgcttggtggtcgaatgggcaggtagccggatcaagcgtatgcagccgccgcattgcatcagccatgatggatactttctcggcaggagcaaggtgagatgacaggagatcctgccccggcacttcgcccaatagcagccagtcccttcccgcttcagtgacaacgtcgagcacagctgcgcaaggaacgcccgtcgtggccagccacgatagccgcgctgcctcgtcttggagttcattcagggcaccggacaggtcggtcttgacaaaaagaaccgggcgcccctgcgctgacagccggaacacggcggcatcagagcagccgattgtctgttgtgcccagtcatagccgaatagcctctccacccaagcggccggagaacctgcgtgcaatccatcttgttcaatcatgcctcgatcgagttgagagtgaatatgagactctaattggataccgaggggaatttatggaacgtcagtggagcatttttgacaagaaatatttgctagctgatagtgaccttaggcgacttttgaacgcgcaataatggtttctgacgtatgtgcttagctcattaaactccagaaacccgcggctgagtggctccttcaacgttgcggttctgtcagttccaaacgtaaaacggcttgtcccgcgtcatcggcgggggtcataacgtgactcccttaattctcatgtatctccgtcaggagactagagccaagctgatctcctttgccccggagatcaccatggacgactttctctatctctacgatctaggaagaaagttcgacggagaaggtgacgataccatgttcaccaccgataatgagaagattagcctcttcaatttcagaaagaatgctgacccacagatggttagagaggcctacgcggcaggtctgatcaagacgatctacccgagtaataatctccaggagatcaaataccttcccaagaaggttaaagatgcagtcaaaagattcaggactaactgcatcaagaacacagagaaagatatatttctcaagatcagaagtactattccagtatggacgattcaaggcttgcttcataaaccaaggcaagtaatagagattggagtctctaagaaagtagttcctactgaatcaaaggccatggagtcaaaaattcagatcgaggatctaacagaactcgccgtgaagactggcgaacagttcatacagagtcttttacgactcaatgacaagaagaaaatcttcgtcaacatggtggagcacgacactctcgtctactccaagaatatcaaagatacagtctcagaagaccaaagggctattgagacttttcaacaaagggtaatatcgggaaacctcctcggattccattgcccagctatctgtcacttcatcaaaaggacagtagaaaaggaaggtggcacctacaaatgccatcattgcgataaaggaaaggctatcgttcaagatgcctctgccgacagtggtcccaaagatggacccccacccacgaggagcatcgtggaaaaagaagacgttccaaccacgtcttcaaagcaagtggattgatgtgatatctccactgacgtaagggatgacgcacaatcccactatccttcgcaagacccttcctctatataaggaagttcatttcatttggagaggactccggtatttttacaacaataccacaacaaaacaaacaacaaacaacattacaatttactattctagtcgaaatggacaagaagtactccattgggctcgatatcggcacaaacagcgtcggctgggccgtcattacggacgagtacaaggtgccgagcaaaaaattcaaagttctgggcaataccgatcgccacagcataaagaagaacctcattggcgccctcctgttcgactccggggaaacggccgaagccacgcggctcaaaagaacagcacggcgcagatatacccgcagaaagaatcggatctgctacctgcaggagatctttagtaatgagatggctaaggtggatgactctttcttccataggctggaggagtcctttttggtggaggaggataaaaagcacgagcgccacccaatctttggcaatatcgtggacgaggtggcgtaccatgaaaagtacccaaccatatatcatctgaggaagaagcttgtagacagtactgataaggctgacttgcggttgatctatctcgcgctggcgcatatgatcaaatttcggggacacttcctcatcgagggggacctgaacccagacaacagcgatgtcgacaaactctttatccaactggttcagacttacaatcagcttttcgaagagaacccgatcaacgcatccggagttgacgccaaagcaatcctgagcgctaggctgtccaaatcccggcggctcgaaaacctcatcgcacagctccctggggagaagaagaacggcctgtttggtaatcttatcgccctgtcactcgggctgacccccaactttaaatctaacttcgacctggccgaagatgccaagcttcaactgagcaaagacacctacgatgatgatctcgacaatctgctggcccagatcggcgaccagtacgcagacctttttttggcggcaaagaacctgtcagacgccattctgctgagtgatattctgcgagtgaacacggagatcaccaaagctccgctgagcgctagtatgatcaagcgctatgatgagcaccaccaagacttgactttgctgaaggcccttgtcagacagcaactgcctgagaagtacaaggaaattttcttcgatcagtctaaaaatggctacgccggatacattgacggcggagcaagccaggaggaattttacaaatttattaagcccatcttggaaaaaatggacggcaccgaggagctgctggtaaagcttaacagagaagatctgttgcgcaaacagcgcactttcgacaatggaagcatcccccaccagattcacctgggcgaactgcacgctatcctcaggcggcaagaggatttctacccctttttgaaagataacagggaaaagattgagaaaatcctcacatttcggataccctactatgtaggccccctcgcccggggaaattccagattcgcgtggatgactcgcaaatcagaagagactatcactccctggaacttcgaggaagtcgtggataagggggcctctgcccagtccttcatcgaaaggatgactaactttgataaaaatctgcctaacgaaaaggtgcttcctaaacactctctgctgtacgagtacttcacagtttataacgagctcaccaaggtcaaatacgtcacagaagggatgagaaagccagcattcctgtctggagagcagaagaaagctatcgtggacctcctcttcaagacgaaccggaaagttaccgtgaaacagctcaaagaagattatttcaaaaagattgaatgtttcgactctgttgaaatcagcggagtggaggatcgcttcaacgcatccctgggaacgtatcacgatctcctgaaaatcattaaagacaaggacttcctggacaatgaggagaacgaggacattcttgaggacattgtcctcacccttacgttgtttgaagatagggagatgattgaagaacgcttgaaaacttacgctcatctcttcgacgacaaagtcatgaaacagctcaagaggcgccgatatacaggatgggggcggctgtcaagaaaactgatcaatgggatccgagacaagcagagtggaaagacaatcctggattttcttaagtccgatggatttgccaaccggaacttcatgcagttgatccatgatgactctctcacctttaaggaggacatccagaaagcacaagtttctggccagggggacagtctccacgagcacatcgctaatcttgcaggtagcccagctatcaaaaagggaatactgcagaccgttaaggtcgtggatgaactcgtcaaagtaatgggaaggcataagcccgagaatatcgttatcgagatggcccgagagaaccaaactacccagaagggacagaagaacagtagggaaaggatgaagaggattgaagagggtataaaagaactggggtcccaaatccttaaggaacacccagttgaaaacacccagcttcagaatgagaagctctacctgtactacctgcagaacggcagggacatgtacgtggatcaggaactggacatcaatcggctctccgactacgacgtggatcatatcgtgccccagtcttttctcaaagatgattctattgataataaagtgttgacaagatccgataaaaatagagggaagagtgataacgtcccctcagaagaagttgtcaagaaaatgaaaaattattggcggcagctgctgaacgccaaactgatcacacaacggaagttcgataatctgactaaggctgaacgaggtggcctgtctgagttggataaagccggcttcatcaaaaggcagcttgttgagacacgccagatcaccaagcacgtggcccaaattctcgattcacgcatgaacaccaagtacgatgaaaatgacaaactgattcgagaggtgaaagttattactctgaagtctaagctggtttcagatttcagaaaggactttcagttttataaggtgagagagatcaacaattaccaccatgcgcatgatgcctacctgaatgcagtggtaggcactgcacttatcaaaaaatatcccaagcttgaatctgaatttgtttacggagactataaagtgtacgatgttaggaaaatgatcgcaaagtctgagcaggaaataggcaaggccaccgctaagtacttcttttacagcaatattatgaattttttcaagaccgagattacactggccaatggagagattcggaagcgaccacttatcgaaacaaacggagaaacaggagaaatcgtgtgggacaagggtagggatttcgcgacagtccggaaggtcctgtccatgccgcaggtgaacatcgttaaaaagaccgaagtacagaccggaggcttctccaaggaaagtatcctcccgaaaaggaacagcgacaagctgatcgcacgcaaaaaagattgggaccccaagaaatacggcggattcgattctcctacagtcgcttacagtgtactggttgtggccaaagtggagaaagggaagtctaaaaaactcaaaagcgtcaaggaactgctgggcatcacaatcatggagcgatcaagcttcgaaaaaaaccccatcgactttctcgaggcgaaaggatataaagaggtcaaaaaagacctcatcattaagcttcccaagtactctctctttgagcttgaaaacggccggaaacgaatgctcgctagtgcgggcgagctgcagaaaggtaacgagctggcactgccctctaaatacgttaatttcttgtatctggccagccactatgaaaagctcaaaggatctcccgaagataatgagcagaagcagctgttcgtggaacaacacaaacactaccttgatgagatcatcgagcaaataagcgaattctccaaaagagtgatcctcgccgacgctaacctcgataaggtgctttctgcttacaataagcacagggataagcccatcagggagcaggcagaaaacattatccacttgtttactctgaccaacttgggcgcgcctgcagccttcaagtacttcgacaccaccatagacagaaagcggtacacctctacaaaggaggtcctggacgccacactgattcatcagtcaattacggggctctatgaaacaagaatcgacctctctcagctcggtggagacagcagggctgaccccaagaagaagaggaaggtgtgagcttggaatggatcttcgatcccgatcgttcaaacatttggcaataaagtttcttaagattgaatcctgttgccggtcttgcgacgattatcatataatttctgttgaattacgttaagcatgtaataattaacatgtaatgcatgacgttatttatgagatgggtttttatgattagagtcccgcaattatacatttaatacgcgatagaaaacaaaatatagcgcgcaaactaggataaattatcgcgcdcggtgtcatctatgttactagatcgggaattgccaagctaattcttgaagacgaaagggcctcgtgatacgcctatttttataggttaatgtcatgataataatggtttcttagacgtcaggtggcacttttcggggaaatgtgcgcggaacccctatttgtttatttttctaaatacattcaaatatgtatccgctcatgagacaataaccctgataaatgcttcaataatgggaccgactcgcgctgtcaggagactagagccaagctgatctcctttgccccggagatcaccatggacgactttctctatctctacgatctaggaagaaagttcgacggagaaggtgacgataccatgttcaccaccgataatgagaagattagcctcttcaatttcagaaagaatgctgacccacagatggttagagaggcctacgcggcaggtctgatcaagacgatctacccgagtaataatctccaggagatcaaataccttcccaagaaggttaaagatgcagtcaaaagattcaggactaactgcatcaagaacacagagaaagatatatttctcaagatcagaagtactattccagtatggacgattcaaggcttgcttcataaaccaaggcaagtaatagagattggagtctctaagaaagtagttcctactgaatcaaaggccatggagtcaaaaattcagatcgaggatctaacagaactcgccgtgaagactggcgaacagttcatacagagtcttttacgactcaatgacaagaagaaaatcttcgtcaacatggtggagcacgacactctcgtctactccaagaatatcaaagatacagtctcagaagaccaaagggctattgagacttttcaacaaagggtaatatcgggaaacctcctcggattccattgcccagctatctgtcacttcatcaaaaggacagtagaaaaggaaggtggcacctacaaatgccatcattgcgataaaggaaaggctatcgttcaagatgcctctgccgacagtggtcccaaagatggacccccacccacgaggagcatcgtggaaaaagaagacgttccaaccacgtcttcaaagcaagtggattgatgtgatatctccactgacgtaagggatgacgcacaatcccactatccttcgcaagacccttcctctatataaggaagttcatttcatttggagaggactccggtatttttacaacaataccacaacaaaacaaacaacaaacaacattacaatttactattctagtcgaaatggcctcctccgagaacgtcatcaccgagttcatgcgcttcaaggtgcgcatggagggcaccgtgaacggccacgagttcgagatcgagggcgagggcgagggccgcccctacgagggccacaacaccgtgaagctgaaggtgaccaagggcggccccctgcccttcgcctgggacatcctgtccccccagttccagtacggctccaaggtgtacgtgaagcaccccgccgacatccccgactacaagaagctgtccttccccgagggcttcaagtgggagcgcgtgatgaacttcgaggacggcggcgtggcgaccgtgacccaggactcctccctgcaggacggctgcttcatctacaaggtgaagttcatcggcgtgaacttcccctccgacggccccgtgatgcagaagaagacgatgggctgggaggcctccaccgagcgcctgtacccccgcgacggcgtgctgaagggcgagacacacaaggccctgaagctgaaggacggcggccactacctggtggagttcaagtccatctacatggccaagaagcccgtgcagctgcccggctactactacgtggacgccaagctggacatcacctcccacaacgaggactacaccatcgtggagcagtacgagcgcaccgagggccgccaccacctgttcctgtaggcttcggccatgctagagtccgcaaaaatcaccagtctctctctacaaatctatctctctctatttttctccagaataatgtgtgagtagttcccagataagggaattagggttcttatagggtttcgctcatgtgttgagcatataagaaacccttagtatgtatttgtatttgtaaaatacttctatcaataaaatttctaattcctaaaaccaaaatccagtgacctcgctgtcaggagtctcaatggtaactttactctttatttaaccatacatttttttttatttttttcactttgttcttcatccactattgttctttgttcatcttgaacaaaagctccctccttctttgttcttcatccaccattgttcttcatcaatcatttcgctgtcaggagcatcttcattcttaagatatgaagataatcttcaaaaggcccctgggaatctgaaagaagagaagcaggcccatttatatgggaaagaacaatagtatttcttatataggcccatttaagttgaaaacaatcttcaaaagtcccacatcgcttagataagaaaacgaagctgagtttatatacagctagagtcgaagtagtgattgaacaaagcaccagtggtctagtggtagaatagtaccctgccacggtacagacccgggttcgattcccggctggtgcaagggaagtcaacaatgcatggttttagagctagaaatagcaagttaaaataaggctagtccgttatcaacttgaaaaagtggcaccgagtcggtgcaacaaagcaccagtggtctagtggtagaatagtaccctgccacggtacagacccgggttcgattcccggctggtgcaatcaggatccaccataacctgttttagagctagaaatagcaagttaaaataaggctagtccgttatcaacttgaaaaagtggcaccgagtcggtgcaacaaagcaccagtggtctagtggtagaatagtaccctgccacggtacagacccgggttcgattcccggctggtgcaagtttgtatctgtagttgctgttttagagctagaaatagcaagttaaaataaggctagtccgttatcaacttgaaaaagtggcaccgagtcggtgcaacaaagcaccagtggtctagtggtagaatagtaccctgccacggtacagacccgggttcgattcccggctggtgcaaaggaagtcaacaatgcatggttttagagctagaaatagcaagttaaaataaggctagtccgttatcaacttgaaaaagtggcaccgagtcggtgcaacaaagcaccagtggtctagtggtagaatagtaccctgccacggtacagacccgggttcgattcccggctggtgcaccagagtgtaaaaggtacgagttttagagctagaaatagcaagttaaaataaggctagtccgttatcaacttgaaaaagtggcaccgagtcggtgcaacaaagcaccagtggtctagtggtagaatagtaccctgccacggtacagacccgggttcgattcccggctggtgcaaggacgatactaaccaatgggttttagagctagaaatagcaagttaaaataaggctagtccgttatcaacttgaaaaagtggcaccgagtcggtgctttttttctagacccagctttcttgtacaaagttggcattacgctgtcatgagaccggatcctgacaggatatattggcgggtaaacctaagagaaaagagcgtttattagaataatcggatatttaaaagggcgtgaaaaggtttatccgttcgtccatttgtatgtgcatgccaaccacagggttcccctcgggatcaaagtactttgatccaacccctccgctgctatagtgcagtcggcttctgacgttcagtgcagccgtcatctgaaaacgacatgtcgcacaagtcctaagttacgcgacaggctgccgccctgcccttttcctggcgttttcttgtcgcgtgttttagtcgcataaagtagaatacttgcgactagaaccggagacattacgccatgaacaagagcgccgccgctggcctgctgggctatgcccgcgtcagcaccgacgaccaggacttgaccaaccaacgggccgaactgcacgcggccggctgcaccaagctgttttccgagaagatcaccggcaccaggcgcgaccgcccggagctggccaggatgcttgaccacctacgccctggcgacgttgtgacagtgaccaggctagaccgcctggcccgcagcacccgcgacctactggacattgccgagcgcatccaggaggccggcgcgggcctgcgtagcctggcagagccgtgggccgacaccaccacgccggccggccgcatggtgttgaccgtgttcgccggcattgccgagttcgagcgttccctaatcatcgaccgcacccggagcgggcgcgaggccgccaaggcccgaggcgtgaagtttggcccccgccctaccctcaccccggcacagatcgcgcacgcccgcgagctgatcgaccaggaaggccgcaccgtgaaagaggcggctgcactgcttggcgtgcatcgctcgaccctgtaccgcgcacttgagcgcagcgaggaagtgacgcccaccgaggccaggcggcgcggtgccttccgtgaggacgcattgaccgaggccgacgccctggcggccgccgagaatgaacgccaagaggaacaagcatgaaaccgcaccaggacggccaggacgaaccgtttttcattaccgaagagatcgaggcggagatgatcgcggccgggtacgtgttcgagccgcccgcgcacctctcaaccgtgcggctgcatgaaatcctggccggtttgtctgatgccaagctggcggcctggccggccagcttggccgctgaagaaaccgagcgccgccgtctaaaaaggtgatgtgtatttgagtaaaacagcttgcgtcatgcggtcgctgcgtatatgatccgatgagtaaataaacaaatacgcaaggggaacgcatgaaggttatcgctgtacttaaccagaaaggcgggtcaggcaagacgaccatcggaacccatctagcccgcgccctgcaactcgccggggccgatgttctgttagtcgattccgatccccagggcagtgcccgcgattgggcggccgtgcgggaagatcaaccgctaaccgttgtcggcatcgaccgcccgacgattgaccgcgacgtgaaggccatcggccggcgcgacttcgtagtgatcgacggagcgccccaggcggcggacttggctgtgtccgcgatcaaggcagccgacttcgtgctgattccggtgcagccaagcccttacgacatatgggccaccgccgacctggtggagctggttaagcagcgcattgaggtcacggatggaaggctacaagcggcctttgtcgtgtcgcgggcgatcaaaggcacgcgcatcggcggtgaggttgccgaggcgctggccgggtacgagctgcccattcttgagtcccgtatcacgcagcgcgtgagctacccaggcactgccgccgccggcacaaccgttcttgaatcagaacccgagggcgacgctgcccgcgaggtccaggcgctggccgctgaaattaaatcaaaactcatttgagttaatgaggtaaagagaaaatgagcaaaagcacaaacacgctaagtgccggccgtccgagcgcacgcagcagcaaggctgcaacgttggccagcctggcagacacgccagccatgaagcgggtcaactttcagttgccggcggaggatcacaccaagctgaagatgtacgcggtacgccaaggcaagaccattaccgagctgctatctgaatagatcgcgcagctaccagagtaaatgagcaaatgaataaatgagtagatgaattttagcggctaaaggaggcggcatggaaaatcaagaacaaccaggcaccgacgccgtggaatgccccatgtgtggaggaacgggcggttggccaggcgtaagcggctgggttgtctgccggccctgcaatggcactggaacccccaagcccgaggaatcggcgtgacggtcgcaaaccatccggcccggtacaaatcggcgcggcgctgggtgatgacctggtggagaagttgaaggccgcgcaggccgcccagcggcaacgcatcgaggcagaagcacgccccggtgaatcgtggcaagcggccgctgatcgaatccgcaaagaatcccggcaaccgccggcagccggtgcgccgtcgattaggaagccgcccaagggcgacgagcaaccagattttttcgttccgatgctctatgacgtgggcacccgcgatagtcgcagcatcatggacgtggccgttttccgtctgtcgaagcgtgaccgacgagctggcgaggtgatccgctacgagcttccagacgggcacgtagaggtttccgcagggccggccggcatggccagtgtgtgggattacgacctggtactgatggcggtttcccatctaaccgaatccatgaaccgataccgggaagggaagggagacaagcccggccgcgtgttccgtccacacgttgcggacgtactcaagttctgccggcgagccgatggcggaaagcagaaagacgacctggtagaaacctgcattcggttaaacaccacgcacgttgccatgcagcgtacgaagaaggccaagaacggccgcctggtgacggtatccgagggtgaagccttgattagccgctacaagatcgtaaagagcgaaaccgggcggccggagtacatcgagatcgagctagctgattggatgtaccgcgagatcacagaaggcaagaacccggacgtgctgacggttcaccccgattactttttgatcgatcccggcatcggccgttttctctaccgcctggcacgccgcgccgcaggcaaggcagaagccagatggttgttcaagacgatctacgaacgcagtggcagcgccggagagttcaagaagttctgtttcaccgtgcgcaagctgatcgggtcaaatgacctgccggagtacgatttgaaggaggaggcggggcaggctggcccgatcctagtcatgcgctaccgcaacctgatcgagggcgaagcatccgccggttcctaatgtacggagcagatgctagggcaaattgccctagcaggggaaaaaggtcgaaaaggactctttcctgtggatagcacgtacattgggaacccaaagccgtacattgggaaccggaacccgtacattgggaacccaaagccgtacattgggaaccggtcacacatgtaagtgactgatataaaagagaaaaaaggcgatttttccgcctaaaactctttaaaacttattaaaactcttaaaacccgcctggcctgtgcataactgtctggccagcgcacagccgaagagctgcaaaaagcgcctacccttcggtcgctgcgctccctacgccccgccgcttcgcgtcggcctatcgcggccgctggccgctcaaaaatggctggcctacggccaggcaatctaccagggcgcggacaagccgcgccgtcgccactcgaccgccggcgcccacatcaaggcaccctgcctcgcgcgtttcggtgatgacggtgaaaacctctgacacatgcagctcccggtgacggtcacagcttgtctgtaagcggatgccgggagcagacaagcccgtcagggcgcgtcagcgggtgttggcgggtgtcggggcgcagccatgacccagtcacgtagcgatagcggagtgtatactggcttaactatgcggcatcagagcagattgtactgagagtgcaccatatgcggtgtgaaataccgcacagatgcgtaaggagaaaataccgcatcaggcgctcttccgcttcctcgctcactgactcgctgcgctcggtcgttcggctgcggcgagcggtatcagctcactcaaaggcggtaatacggttatccacagaatcaggggataacgcaggaaagaacatgtgagcaaaaggccagcaaaaggccaggaaccgtaaaaaggccgcgttgctggcgtttttccataggctccgcccccctgacgagcatcacaaaaatcgacgctcaagtcagaggtggcgaaacccgacaggactataaagataccaggcgtttccccctggaagctccctcgtgcgctctcctgttccgaccctgccgcttaccggatacctgtccgcctttctcccttcgggaagcgtggcgctttctcatagctcacgctgtaggtatctcagttcggtgtaggtcgttcgctccaagctgggctgtgtgcacgaaccccccgttcagcccgaccgctgcgccttatccggtaactatcgtcttgagtccaacccggtaagacacgacttatcgccactggcagcagccactggtaacaggattagcagagcgaggtatgtaggcggtgctacagagttcttgaagtggtggcctaactacggctacactagaaggacagtatttggtatctgcgctctgctgaagccagttaccttcggaaaaagagttggtagctcttgatccggcaaacaaaccaccgctggtagcggtggtttttttgtttgcaagcagcagattacgcgcagaaaaaaaggatctcaagaagatcctttgatcttttctacggggtctgacgctcagtggaacgaaaactcacgttaagggattttggtcatgcattctaggtgattatttgccgactaccttggtgatctcgcctttcacgtagtggacaaattcttccaactgatctgcgcgcgaggccaagcgatcttcttcttgtccaagataagcctgtctagcttcaagtatgacgggctgatactgggccggcaggcgctccattgcccagtcggcagcgacatccttcggcgcgattttgccggttactgcgctgtaccaaatgcgggacaacgtaagcactacatttcgctcatcaccagcccagtcgggcggcgagttccatagcgttaaggtttcatttagcgcctcaaatagatcctgttcaggaaccggatcaaagagttcctccgccgctggacctaccaaggcaacgctatgttctcttgcttttgtcagcaagatagccagatcaatgtcgatcgtggctggctcgaagatacctgcaagaatgtcattgcgctgccattctccaaattgcagttcgcgcttagctggataacgccacggaatgatgtcgtcgtgcacaacaatggtgacttctacagcgcggagaatctcgctctctccaggggaagccgaagtttccaaaaggtcgttgatcaaagctcgccgcgttgtttcatcaagccttacggtcaccgtaaccagcaaatcaatatcactgtgtggcttcaggccgccatccactgcggagccgtacaaatgtacggccagcaacgtcggttcgagatggcgctcgatgacgccaactacctctgatagttgagtcgatacttcggcgatcaccgcttccctcataatgtttaactttgttttagggcgactgccctgctgcgtaacatcgttgctgctccataacatcaaacatcgacccacggcgtaacgcgcttgctgcttggatgcccgaggcatagactgtaccccaaaaaaacagtcataacaagccatgaaaaccgccactgcgccgttaccaccgctgcgttcggtcaaggttctggaccagttgcgtgagcgcatacgctacttgcattacagcttacgaaccgaacaggcttatgtccactgggttcgtgccttcatccgtttccacggtgtgcgtcacccggcaaccttgggtagcagcgaagtcgaggcatttctgtcctggctggaacagaacttattatttccttcctcttttctacagtatttaaagataccccaagaagctaattataacaagacgaactccaattcactgttccttgcattctaaaaccttaaataccagaaaacagctttttcaaagttgttttcaaagttggcgtataacatagtatcgacggagccgattttgaaaccgcggtgatcacaggcagcaacgctctgtcatcgttacaatcaacatgctaccctccgcgagatcatccgtgtttcaaacccggcagcttagttgccgttcttccgaatagcatcggtaacatgagcaaagtctgccgccttacaacggctctcccgctgacgccgtcccggactgatgggctgcctgtatcgagtggtgattttgtgccgagctgccggtcggggagctgttggctggctggtggcaggatatattgtggtgtaaacataacggatccggtctca

SEQ ID NO: 95 - DNA, 20908 bp, synthetic construct
  source 1..20908: mol_type = other DNA
ggagagcgatcagcttgcatgccggtcgatctagtaacatagatgacaccgcgcgcgataatttatcctagtttgcgcgctatattttgttttctatcgcgtattaaatgtataattgcgggactctaatcataaaaacccatctcataaataacgtcatgcattacatgttaattattacatgcttaacgtaattcaacagaaattatatgataatcatggcaagaccggcaacaggattcaatcttaagaaactttattgccaaatgtttgaacgatctgcttgactctagctagagtccgaaccccagagtcccgctcagaagaactcgtcaagaaggcgatagaaggctatgcgctgcgaatcgggagcggcgataccgtaaagcacgaggaagcggtcagcccattcgccgccaagctcttcagcaatatcacgggtagccaacgctatgtcctgatagcggtccgccacacccagccggccacagtcgatgaatccagaaaagcggccattttccaccatgatattcggcaagcaggcgtcgccgtgggtcacgacgagatcctcgccgtcgggcatccgcgccttgagcctggcgaacagttcggctggcgcgagcccctgatgctcttcgtccagatcatcctgatcgacaagaccggcttccatccgagtacgtgctcgctcgatgcggtgtttcgcttggtggtcgaatgggcaggtagccggatcaagcgtatgcagccgccgcattgcatcagccatgatggatactttctcggcaggagcaaggtgagatgacaggagatcctgccccggcacttcgcccaatagcagccagtcccttcccgcttcagtgacaacgtcgagcacagctgcgcaaggaacgcccgtcgtggccagccacgatagccgcgctgcctcgtcttggagttcattcagggcaccggacaggtcggtcttgacaaaaagaaccgggcgcccctgcgctgacagccggaacacggcggcatcagagcagccgattgtctgttgtgcccagtcatagccgaatagcctctccacccaagcggccggagaacctgcgtgcaatccatcttgttcaatcatgcctcgatcgagttgagagtgaatatgagactctaattggataccgaggggaatttatggaacgtcagtggagcatttttgacaagaaatatttgctagctgatagtgaccttaggcgacttttgaacgcgcaataatggtttctgacgtatgtgcttagctcattaaactccagaaacccgcggctgagtggctccttcaacgttgcggttctgtcagttccaaacgtaaaacggcttgtcccgcgtcatcggcgggggtcataacgtgactcccttaattctcatgtatctccgtcaggagactagagccaagctgatctcctttgccccggagatcaccatggacgactttctctatctctacgatctaggaagaaagttcgacggagaaggtgacgataccatgttcaccaccgataatgagaagattagcctcttcaatttcagaaagaatgctgacccacagatggttagagaggcctacgcggcaggtctgatcaagacgatctacccgagtaataatctccaggagatcaaataccttcccaagaaggttaaagatgcagtcaaaagattcaggactaactgcatcaagaacacagagaaagatatatttctcaagatcagaagtactattccagtatggacgattcaaggcttgcttcataaaccaaggcaagtaatagagattggagtctctaagaaagtagttcctactgaatcaaaggccatggagtcaaaaattcagatcgaggatctaacagaactcgccgtgaagactggcgaacagttcatacagagtcttttacgactcaatgacaagaagaaaatcttcgtcaacatggtggagcacgacactctcgtctactccaagaatatcaaagatacagtctcagaagaccaaagggctattgagacttttcaacaaagggtaatatcgggaaacctcctcggattccattgcccagctatctgtcacttcatcaaaaggacagtagaaaaggaaggtggcacctacaaatgccatcattgcgataaaggaaaggctatcgttcaagatgcctctgccgacagtggtcccaaagatggacccccacccacgaggagcatcgtggaaaaagaagacgttccaaccacgtcttcaaagcaagtggattgatgtgatatctccactgacgtaagggatgacgcacaatcccactatccttcgcaagacccttcctctatataaggaagttcatttcatttggagaggactccggtatttttacaacaataccacaacaaaacaaacaacaaacaacattacaatttactattctagtcgaaatggacaagaagtactccattgggctcgatatcggcacaaacagcgtcggctgggccgtcattacggacgagtacaaggtgccgagcaaaaaattcaaagttctgggcaataccgatcgccacagcataaagaagaacctcattggcgccctcctgttcgactccggggaaacggccgaagccacgcggctcaaaagaacagcacggcgcagatatacccgcagaaagaatcggatctgctacctgcaggagatctttagtaatgagatggctaaggtggatgactctttcttccataggctggaggagtcctttttggtggaggaggataaaaagcacgagcgccacccaatctttggcaatatcgtggacgaggtggcgtaccatgaaaagtacccaaccatatatcatctgaggaagaagcttgtagacagtactgataaggctgacttgcggttgatctatctcgcgctggcgcatatgatcaaatttcggggacacttcctcatcgagggggacctgaacccagacaacagcgatgtcgacaaactctttatccaactggttcagacttacaatcagcttttcgaagagaacccgatcaacgcatccggagttgacgccaaagcaatcctgagcgctaggctgtccaaatcccggcggctcgaaaacctcatcgcacagctccctggggagaagaagaacggcctgtttggtaatcttatcgccctgtcactcgggctgacccccaactttaaatctaacttcgacctggccgaagatgccaagcttcaactgagcaaagacacctacgatgatgatctcgacaatctgctggcccagatcggcgaccagtacgcagacctttttttggcggcaaagaacctgtcagacgccattctgctgagtgatattctgcgagtgaacacggagatcaccaaagctccgctgagcgctagtatgatcaagcgctatgatgagcaccaccaagacttgactttgctgaaggcccttgtcagacagcaactgcctgagaagtacaaggaaattttcttcgatcagtctaaaaatggctacgccggatacattgacggcggagcaagccaggaggaattttacaaatttattaagcccatcttggaaaaaatggacggcaccgaggagctgctggtaaagcttaacagagaagatctgttgcgcaaacagcgcactttcgacaatggaagcatcccccaccagattcacctgggcgaactgcacgctatcctcaggcggcaagaggatttctacccctttttgaaagataacagggaaaagattgagaaaatcctcacatttcggataccctactatgtaggccccctcgcccggggaaattccagattcgcgtggatgactcgcaaatcagaagagactatcactccctggaacttcgaggaagtcgtggataagggggcctctgcccagtccttcatcgaaaggatgactaactttgataaaaatctgcctaacgaaaaggtgcttcctaaacactctctgctgtacgagtacttcacagtttataacgagctcaccaaggtcaaatacgtcacagaagggatgagaaagccagcattcctgtctggagagcagaagaaagctatcgtggacctcctcttcaagacgaaccggaaagttaccgtgaaacagctcaaagaagattatttcaaaaagattgaatgtttcgactctgttgaaatcagcggagtggaggatcgcttcaacgcatccctgggaacgtatcacgatctcctgaaaatcattaaagacaaggacttcctggacaatgaggagaacgaggacattcttgaggacattgtcctcacccttacgttgtttgaagatagggagatgattgaagaacgcttgaaaacttacgctcatctcttcgacgacaaagtcatgaaacagctcaagaggcgccgatatacaggatgggggcggctgtcaagaaaactgatcaatgggatccgagacaagcagagtggaaagacaatcctggattttcttaagtccgatggatttgccaaccggaacttcatgcagttgatccatgatgactctctcacctttaaggaggacatccagaaagcacaagtttctggccagggggacagtctccacgagcacatcgctaatcttgcaggtagcccagctatcaaaaagggaatactgcagaccgttaaggtcgtggatgaactcgtcaaagtaatgggaaggcataagcccgagaatatcgttatcgagatggcccgagagaaccaaactacccagaagggacagaagaacagtagggaaaggatgaagaggattgaagagggtataaaagaactggggtcccaaatccttaaggaacacccagttgaaaacacccagcttcagaatgagaagctctacctgtactacctgcagaacggcagggacatgtacgtggatcaggaactggacatcaatcggctctccgactacgacgtggatcatatcgtgccccagtcttttctcaaagatgattctattgataataaagtgttgacaagatccgataaaaatagagggaagagtgataacgtcccctcagaagaagttgtcaagaaaatgaaaaattattggcggcagctgctgaacgccaaactgatcacacaacggaagttcgataatctgactaaggctgaacgaggtggcctgtctgagttggataaagccggcttcatcaaaaggcagcttgttgagacacgccagatcaccaagcacgtggcccaaattctcgattcacgcatgaacaccaagtacgatgaaaatgacaaactgattcgagaggtgaaagttattactctgaagtctaagctggtttcagatttcagaaaggactttcagttttataaggtgagagagatcaacaattaccaccatgcgcatgatgcctacctgaatgcagtggtaggcactgcacttatcaaaaaatatcccaagcttgaatctgaatttgtttacggagactataaagtgtacgatgttaggaaaatgatcgcaaagtctgagcaggaaataggcaaggccaccgctaagtacttcttttacagcaatattatgaattttttcaagaccgagattacactggccaatggagagattcggaagcgaccacttatcgaaacaaacggagaaacaggagaaatcgtgtgggacaagggtagggatttcgcgacagtccggaaggtcctgtccatgccgcaggtgaacatcgttaaaaagaccgaagtacagaccggaggcttctccaaggaaagtatcctcccgaaaaggaacagcgacaagctgatcgcacgcaaaaaagattgggaccccaagaaatacggcggattcgattctcctacagtcgcttacagtgtactggttgtggccaaagtggagaaagggaagtctaaaaaactcaaaagcgtcaaggaactgctgggcatcacaatcatggagcgatcaagcttcgaaaaaaaccccatcgactttctcgaggcgaaaggatataaagaggtcaaaaaagacctcatcattaagcttcccaagtactctctctttgagcttgaaaacggccggaaacgaatgctcgctagtgcgggcgagctgcagaaaggtaacgagctggcactgccctctaaatacgttaatttcttgtatctggccagccactatgaaaagctcaaaggatctcccgaagataatgagcagaagcagctgttcgtggaacaacacaaacactaccttgatgagatcatcgagcaaataagcgaattctccaaaagagtgatcctcgccgacgctaacctcgataaggtgctttctgcttacaataagcacagggataagcccatcagggagcaggcagaaaacattatccacttgtttactctgaccaacttgggcgcgcctgcagccttcaagtacttcgacaccaccatagacagaaagcggtacacctctacaaaggaggtcctggacgccacactgattcatcagtcaattacggggctctatgaaacaagaatcgacctctctcagctcggtggagacagcagggctgaccccaagaagaagaggaaggtgtgagcttggaatggatcttcgatcccgatcgttcaaacatttggcaataaagtttcttaagattgaatcctgttgccggtcttgcgacgattatcatataatttctgttgaattacgttaagcatgtaataattaacatgtaatgcatgacgttatttatgagatgggtttttatgattagagtcccgcaattatacatttaatacgcgatagaaaacaaaatatagcgcgcaaactaggataaattatcgcgcdcggtgtcatctatgttactagatcgggaattgccaagctaattcttgaagacgaaagggcctcgtgatacgcctatttttataggttaatgtcatgataataatggtttcttagacgtcaggtggcacttttcggggaaatgtgcgcggaacccctatttgtttatttttctaaatacattcaaatatgtatccgctcatgagacaataaccctgataaatgcttcaataatgggaccgactcgcgctgtcaggagactagagccaagctgatctcctttgccccggagatcaccatggacgactttctctatctctacgatctaggaagaaagttcgacggagaaggtgacgataccatgttcaccaccgataatgagaagattagcctcttcaatttcagaaagaatgctgacccacagatggttagagaggcctacgcggcaggtctgatcaagacgatctacccgagtaataatctccaggagatcaaataccttcccaagaaggttaaagatgcagtcaaaagattcaggactaactgcatcaagaacacagagaaagatatatttctcaagatcagaagtactattccagtatggacgattcaaggcttgcttcataaaccaaggcaagtaatagagattggagtctctaagaaagtagttcctactgaatcaaaggccatggagtcaaaaattcagatcgaggatctaacagaactcgccgtgaagactggcgaacagttcatacagagtcttttacgactcaatgacaagaagaaaatcttcgtcaacatggtggagcacgacactctcgtctactccaagaatatcaaagatacagtctcagaagaccaaagggctattgagacttttcaacaaagggtaatatcgggaaacctcctcggattccattgcccagctatctgtcacttcatcaaaaggacagtagaaaaggaaggtggcacctacaaatgccatcattgcgataaaggaaaggctatcgttcaagatgcctctgccgacagtggtcccaaagatggacccccacccacgaggagcatcgtggaaaaagaagacgttccaaccacgtcttcaaagcaagtggattgatgtgatatctccactgacgtaagggatgacgcacaatcccactatccttcgcaagacccttcctctatataaggaagttcatttcatttggagaggactccggtatttttacaacaataccacaacaaaacaaacaacaaacaacattacaatttactattctagtcgaaatggcctcctccgagaacgtcatcaccgagttcatgcgcttcaaggtgcgcatggagggcaccgtgaacggccacgagttcgagatcgagggcgagggcgagggccgcccctacgagggccacaacaccgtgaagctgaaggtgaccaagggcggccccctgcccttcgcctgggacatcctgtccccccagttccagtacggctccaaggtgtacgtgaagcaccccgccgacatccccgactacaagaagctgtccttccccgagggcttcaagtgggagcgcgtgatgaacttcgaggacggcggcgtggcgaccgtgacccaggactcctccctgcaggacggctgcttcatctacaaggtgaagttcatcggcgtgaacttcccctccgacggccccgtgatgcagaagaagacgatgggctgggaggcctccaccgagcgcctgtacccccgcgacggcgtgctgaagggcgagacacacaaggccctgaagctgaaggacggcggccactacctggtggagttcaagtccatctacatggccaagaagcccgtgcagctgcccggctactactacgtggacgccaagctggacatcacctcccacaacgaggactacaccatcgtggagcagtacgagcgcaccgagggccgccaccacctgttcctgtaggcttcggccatgctagagtccgcaaaaatcaccagtctctctctacaaatctatctctctctatttttctccagaataatgtgtgagtagttcccagataagggaattagggttcttatagggtttcgctcatgtgttgagcatataagaaacccttagtatgtatttgtatttgtaaaatacttctatcaataaaatttctaattcctaaaaccaaaatccagtgacctcgctgtcaggagtctcaatggtaactttactctttatttaaccatacatttttttttatttttttcactttgttcttcatccactattgttctttgttcatcttgaacaaaagctccctccttctttgttcttcatccaccattgttcttcatcaatcatttcgctgtcaggagcatcttcattcttaagatatgaagataatcttcaaaaggcccctgggaatctgaaagaagagaagcaggcccatttatatgggaaagaacaatagtatttcttatataggcccatttaagttgaaaacaatcttcaaaagtcccacatcgcttagataagaaaacgaagctgagtttatatacagctagagtcgaagtagtgattgaacaaagcaccagtggtctagtggtagaatagtaccctgccacggtacagacccgggttcgattcccggctggtgcaagggaagtcaacaatgcatggttttagagctagaaatagcaagttaaaataaggctagtccgttatcaacttgaaaaagtggcaccgagtcggtgcaacaaagcaccagtggtctagtggtagaatagtaccctgccacggtacagacccgggttcgattcccggctggtgcaatcaggatccaccataacctgttttagagctagaaatagcaagttaaaataaggctagtccgttatcaacttgaaaaagtggcaccgagtcggtgcaacaaagcaccagtggtctagtggtagaatagtaccctgccacggtacagacccgggttcgattcccggctggtgcaagtttgtatctgtagttgctgttttagagctagaaatagcaagttaaaataaggctagtccgttatcaacttgaaaaagtggcaccgagtcggtgcaacaaagcaccagtggtctagtggtagaatagtaccctgccacggtacagacccgggttcgattcccggctggtgcaaaggaagtcaacaatgcatggttttagagctagaaatagcaagttaaaataaggctagtccgttatcaacttgaaaaagtggcaccgagtcggtgcaacaaagcaccagtggtctagtggtagaatagtaccctgccacggtacagacccgggttcgattcccggctggtgcaccagagtgtaaaaggtacgagttttagagctagaaatagcaagttaaaataaggctagtccgttatcaacttgaaaaagtggcaccgagtcggtgcaacaaagcaccagtggtctagtggtagaatagtaccctgccacggtacagacccgggttcgattcccggctggtgcaaggacgatactaaccaatgggttttagagctagaaatagcaagttaaaataaggctagtccgttatcaacttgaaaaagtggcaccgagtcggtgctttttttctagacccagctttcttgtacaaagttggcattacgctgtcaggagcatcttcattcttaagatatgaagataatcttcaaaaggcccctgggaatctgaaagaagagaagcaggcccatttatatgggaaagaacaatagtatttcttatataggcccatttaagttgaaaacaatcttcaaaagtcccacatcgcttagataagaaaacgaagctgagtttatatacagctagagtcgaagtagtgattgaacaaagcaccagtggtctagtggtagaatagtaccctgccacggtacagacccgggttcgattcccggctggtgcacgacggcttgagactttgcagttttagagctagaaatagcaagttaaaataaggctagtccgttatcaacttgaaaaagtggcaccgagtcggtgcaacaaagcaccagtggtctagtggtagaatagtaccctgccacggtacagacccgggttcgattcccggctggtgcaaatcgaaaaggagttgcagggttttagagctagaaatagcaagttaaaataaggctagtccgttatcaacttgaaaaagtggcaccgagtcggtgcaacaaagcaccagtggtctagtggtagaatagtaccctgccacggtacagacccgggttcgattcccggctggtgcaaagggtcaagtacttcaatggttttagagctagaaatagcaagttaaaataaggctagtccgttatcaacttgaaaaagtggcaccgagtcggtgcaacaaagcaccagtggtctagtggtagaatagtaccctgccacggtacagacccgggttcgattcccggctggtgcacgacggcttgagcctttgcagttttagagctagaaatagcaagttaaaataaggctagtccgttatcaacttgaaaaagtggcaccgagtcggtgcaacaaagcaccagtggtctagtggtagaatagtaccctgccacggtacagacccgggttcgattcccggctggtgcaggacctcacaaactttatgggttttagagctagaaatagcaagttaaaataaggctagtccgttatcaacttgaaaaagtggcaccgagtcggtgcaacaaagcaccagtggtctagtggtagaatagtaccctgccacggtacagacccgggttcgattcccggctggtgcaatggacataacaggcgtcgagttttagagctagaaatagcaagttaaaataaggctagtccgttatcaacttgaaaaagtggcaccgagtcggtgctttttttctagacccagctttcttgtacaaagttggcattacgctgtcaggagcatcttcattcttaagatatgaagataatcttcaaaaggcccctgggaatctgaaagaagagaagcaggcccatttatatgggaaagaacaatagtatttcttatataggcccatttaagttgaaaacaatcttcaaaagtcccacatcgcttagataagaaaacgaagctgagtttatatacagctagagtcgaagtagtgattgaacaaagcaccagtggtctagtggtagaatagtaccctgccacggtacagacccgggttcgattcccggctggtgcacgaacagttgaaagcaacaggttttagagctagaaatagcaagttaaaataaggctagtccgttatcaacttgaaaaagtggcaccgagtcggtgcaacaaagcaccagtggtctagtggtagaatagtaccctgccacggtacagacccgggttcgattcccggctggtgcatcatcataggaggtgccgaggttttagagctagaaatagcaagttaaaataaggctagtccgttatcaacttgaaaaagtggcaccgagtcggtgcaacaaagcaccagtggtctagtggtagaatagtaccctgccacggtacagacccgggttcgattcccggctggtgcatagaaattcaccccccatgggttttagagctagaaatagcaagttaaaataaggctagtccgttatcaacttgaaaaagtggcaccgagtcggtgcaacaaagcaccagtggtctagtggtagaatagtaccctgccacggtacagacccgggttcgattcccggctggtgcatgtgatcagagagcctcctggttttagagctagaaatagcaagttaaaataaggctagtccgttatcaacttgaaaaagtggcaccgagtcggtgcaacaaagcaccagtggtctagtggtagaatagtaccctgccacggtacagacccgggttcgattcccggctggtgcaggaaaccatccagttcaactgttttagagctagaaatagcaagttaaaataaggctagtccgttatcaacttgaaaaagtggcaccgagtcggtgctttttttctagacccagctttcttgtacaaagttggcattacgctgtcaggagcatcttcattcttaagatatgaagataatcttcaaaaggcccctgggaatctgaaagaagagaagcaggcccatttatatgggaaagaacaatagtatttcttatataggcccatttaagttgaaaacaatcttcaaaagtcccacatcgcttagataagaaaacgaagctgagtttatatacagctagagtcgaagtagtgattgaacaaagcaccagtggtctagtggtagaatagtaccctgccacggtacagacccgggttcgattcccggctggtgcattaaaggggcatcagtccaagttttagagctagaaatagcaagttaaaataaggctagtccgttatcaacttgaaaaagtggcaccgagtcggtgcaacaaagcaccagtggtctagtggtagaatagtaccctgccacggtacagacccgggttcgattcccggctggtgcaatctactttgaaaatgtggggttttagagctagaaatagcaagttaaaataaggctagtccgttatcaacttgaaaaagtggcaccgagtcggtgcaacaaagcaccagtggtctagtggtagaatagtaccctgccacggtacagacccgggttcgattcccggctggtgcagaaattcacagaccttgtgggttttagagctagaaatagcaagttaaaataaggctagtccgttatcaacttgaaaaagtggcaccgagtcggtgcaacaaagcaccagtggtctagtggtagaatagtaccctgccacggtacagacccgggttcgattcccggctggtgcacagtcattccaaatgcccaagttttagagctagaaatagcaagttaaaataaggctagtccgttatcaacttgaaaaagtggcaccgagtcggtgcaacaaagcaccagtggtctagtggtagaatagtaccctgccacggtacagacccgggttcgattcccggctggtgcaagatggagtggaatgcaaaggttttagagctagaaatagcaagttaaaataaggctagtccgttatcaacttgaaaaagtggcaccgagtcggtgcaacaaagcaccagtggtctagtggtagaatagtaccctgccacggtacagacccgggttcgattcccggctggtgcaccttcaacttgacacctagggttttagagctagaaatagcaagttaaaataaggctagtccgttatcaacttgaaaaagtggcaccgagtcggtgctttttttctagacccagctttcttgtacaaagttggcattacgctgtcatgagaccggatcctgacaggatatattggcgggtaaacctaagagaaaagagcgtttattagaataatcggatatttaaaagggcgtgaaaaggtttatccgttcgtccatttgtatgtgcatgccaaccacagggttcccctcgggatcaaagtactttgatccaacccctccgctgctatagtgcagtcggcttctgacgttcagtgcagccgtcatctgaaaacgacatgtcgcacaagtcctaagttacgcgacaggctgccgccctgcccttttcctggcgttttcttgtcgcgtgttttagtcgcataaagtagaatacttgcgactagaaccggagacattacgccatgaacaagagcgccgccgctggcctgctgggctatgcccgcgtcagcaccgacgaccaggacttgaccaaccaacgggccgaactgcacgcggccggctgcaccaagctgttttccgagaagatcaccggcaccaggcgcgaccgcccggagctggccaggatgcttgaccacctacgccctggcgacgttgtgacagtgaccaggctagaccgcctggcccgcagcacccgcgacctactggacattgccgagcgcatccaggaggccggcgcgggcctgcgtagcctggcagagccgtgggccgacaccaccacgccggccggccgcatggtgttgaccgtgttcgccggcattgccgagttcgagcgttccctaatcatcgaccgcacccggagcgggcgcgaggccgccaaggcccgaggcgtgaagtttggcccccgccctaccctcaccccggcacagatcgcgcacgcccgcgagctgatcgaccaggaaggccgcaccgtgaaagaggcggctgcactgcttggcgtgcatcgctcgaccctgtaccgcgcacttgagcgcagcgaggaagtgacgcccaccgaggccaggcggcgcggtgccttccgtgaggacgcattgaccgaggccgacgccctggcggccgccgagaatgaacgccaagaggaacaagcatgaaaccgcaccaggacggccaggacgaaccgtttttcattaccgaagagatcgaggcggagatgatcgcggccgggtacgtgttcgagccgcccgcgcacctctcaaccgtgcggctgcatgaaatcctggccggtttgtctgatgccaagctggcggcctggccggccagcttggccgctgaagaaaccgagcgccgccgtctaaaaaggtgatgtgtatttgagtaaaacagcttgcgtcatgcggtcgctgcgtatatgatccgatgagtaaataaacaaatacgcaaggggaacgcatgaaggttatcgctgtacttaaccagaaaggcgggtcaggcaagacgaccatcggaacccatctagcccgcgccctgcaactcgccggggccgatgttctgttagtcgattccgatccccagggcagtgcccgcgattgggcggccgtgcgggaagatcaaccgctaaccgttgtcggcatcgaccgcccgacgattgaccgcgacgtgaaggccatcggccggcgcgacttcgtagtgatcgacggagcgccccaggcggcggacttggctgtgtccgcgatcaaggcagccgacttcgtgctgattccggtgcagccaagcccttacgacatatgggccaccgccgacctggtggagctggttaagcagcgcattgaggtcacggatggaaggctacaagcggcctttgtcgtgtcgcgggcgatcaaaggcacgcgcatcggcggtgaggttgccgaggcgctggccgggtacgagctgcccattcttgagtcccgtatcacgcagcgcgtgagctacccaggcactgccgccgccggcacaaccgttcttgaatcagaacccgagggcgacgctgcccgcgaggtccaggcgctggccgctgaaattaaatcaaaactcatttgagttaatgaggtaaagagaaaatgagcaaaagcacaaacacgctaagtgccggccgtccgagcgcacgcagcagcaaggctgcaacgttggccagcctggcagacacgccagccatgaagcgggtcaactttcagttgccggcggaggatcacaccaagctgaagatgtacgcggtacgccaaggcaagaccattaccgagctgctatctgaatagatcgcgcagctaccagagtaaatgagcaaatgaataaatgagtagatgaattttagcggctaaaggaggcggcatggaaaatcaagaacaaccaggcaccgacgccgtggaatgccccatgtgtggaggaacgggcggttggccaggcgtaagcggctgggttgtctgccggccctgcaatggcactggaacccccaagcccgaggaatcggcgtgacggtcgcaaaccatccggcccggtacaaatcggcgcggcgctgggtgatgacctggtggagaagttgaaggccgcgcaggccgcccagcggcaacgcatcgaggcagaagcacgccccggtgaatcgtggcaagcggccgctgatcgaatccgcaaagaatcccggcaaccgccggcagccggtgcgccgtcgattaggaagccgcccaagggcgacgagcaaccagattttttcgttccgatgctctatgacgtgggcacccgcgatagtcgcagcatcatggacgtggccgttttccgtctgtcgaagcgtgaccgacgagctggcgaggtgatccgctacgagcttccagacgggcacgtagaggtttccgcagggccggccggcatggccagtgtgtgggattacgacctggtactgatggcggtttcccatctaaccgaatccatgaaccgataccgggaagggaagggagacaagcccggccgcgtgttccgtccacacgttgcggacgtactcaagttctgccggcgagccgatggcggaaagcagaaagacgacctggtagaaacctgcattcggttaaacaccacgcacgttgccatgcagcgtacgaagaaggccaagaacggccgcctggtgacggtatccgagggtgaagccttgattagccgctacaagatcgtaaagagcgaaaccgggcggccggagtacatcgagatcgagctagctgattggatgtaccgcgagatcacagaaggcaagaacccggacgtgctgacggttcaccccgattactttttgatcgatcccggcatcggccgttttctctaccgcctggcacgccgcgccgcaggcaaggcagaagccagatggttgttcaagacgatctacgaacgcagtggcagcgccggagagttcaagaagttctgtttcaccgtgcgcaagctgatcgggtcaaatgacctgccggagtacgatttgaaggaggaggcggggcaggctggcccgatcctagtcatgcgctaccgcaacctgatcgagggcgaagcatccgccggttcctaatgtacggagcagatgctagggcaaattgccctagcaggggaaaaaggtcgaaaaggactctttcctgtggatagcacgtacattgggaacccaaagccgtacattgggaaccggaacccgtacattgggaacccaaagccgtacattgggaaccggtcacacatgtaagtgactgatataaaagagaaaaaaggcgatttttccgcctaaaactctttaaaacttattaaaactcttaaaacccgcctggcctgtgcataactgtctggccagcgcacagccgaagagctgcaaaaagcgcctacccttcggtcgctgcgctccctacgccccgccgcttcgcgtcggcctatcgcggccgctggccgctcaaaaatggctggcctacggccaggcaatctaccagggcgcggacaagccgcgccgtcgccactcgaccgccggcgcccacatcaaggcaccctgcctcgcgcgtttcggtgatgacggtgaaaacctctgacacatgcagctcccggtgacggtcacagcttgtctgtaagcggatgccgggagcagacaagcccgtcagggcgcgtcagcgggtgttggcgggtgtcggggcgcagccatgacccagtcacgtagcgatagcggagtgtatactggcttaactatgcggcatcagagcagattgtactgagagtgcaccatatgcggtgtgaaataccgcacagatgcgtaaggagaaaataccgcatcaggcgctcttccgcttcctcgctcactgactcgctgcgctcggtcgttcggctgcggcgagcggtatcagctcactcaaaggcggtaatacggttatccacagaatcaggggataacgcaggaaagaacatgtgagcaaaaggccagcaaaaggccaggaaccgtaaaaaggccgcgttgctggcgtttttccataggctccgcccccctgacgagcatcacaaaaatcgacgctcaagtcagaggtggcgaaacccgacaggactataaagataccaggcgtttccccctggaagctccctcgtgcgctctcctgttccgaccctgccgcttaccggatacctgtccgcctttctcccttcgggaagcgtggcgctttctcatagctcacgctgtaggtatctcagttcggtgtaggtcgttcgctccaagctgggctgtgtgcacgaaccccccgttcagcccgaccgctgcgccttatccggtaactatcgtcttgagtccaacccggtaagacacgacttatcgccactggcagcagccactggtaacaggattagcagagcgaggtatgtaggcggtgctacagagttcttgaagtggtggcctaactacggctacactagaaggacagtatttggtatctgcgctctgctgaagccagttaccttcggaaaaagagttggtagctcttgatccggcaaacaaaccaccgctggtagcggtggtttttttgtttgcaagcagcagattacgcgcagaaaaaaaggatctcaagaagatcctttgatcttttctacggggtctgacgctcagtggaacgaaaactcacgttaagggattttggtcatgcattctaggtgattatttgccgactaccttggtgatctcgcctttcacgtagtggacaaattcttccaactgatctgcgcgcgaggccaagcgatcttcttcttgtccaagataagcctgtctagcttcaagtatgacgggctgatactgggccggcaggcgctccattgcccagtcggcagcgacatccttcggcgcgattttgccggttactgcgctgtaccaaatgcgggacaacgtaagcactacatttcgctcatcaccagcccagtcgggcggcgagttccatagcgttaaggtttcatttagcgcctcaaatagatcctgttcaggaaccggatcaaagagttcctccgccgctggacctaccaaggcaacgctatgttctcttgcttttgtcagcaagatagccagatcaatgtcgatcgtggctggctcgaagatacctgcaagaatgtcattgcgctgccattctccaaattgcagttcgcgcttagctggataacgccacggaatgatgtcgtcgtgcacaacaatggtgacttctacagcgcggagaatctcgctctctccaggggaagccgaagtttccaaaaggtcgttgatcaaagctcgccgcgttgtttcatcaagccttacggtcaccgtaaccagcaaatcaatatcactgtgtggcttcaggccgccatccactgcggagccgtacaaatgtacggccagcaacgtcggttcgagatggcgctcgatgacgccaactacctctgatagttgagtcgatacttcggcgatcaccgcttccctcataatgtttaactttgttttagggcgactgccctgctgcgtaacatcgttgctgctccataacatcaaacatcgacccacggcgtaacgcgcttgctgcttggatgcccgaggcatagactgtaccccaaaaaaacagtcataacaagccatgaaaaccgccactgcgccgttaccaccgctgcgttcggtcaaggttctggaccagttgcgtgagcgcatacgctacttgcattacagcttacgaaccgaacaggcttatgtccactgggttcgtgccttcatccgtttccacggtgtgcgtcacccggcaaccttgggtagcagcgaagtcgaggcatttctgtcctggctggaacagaacttattatttccttcctcttttctacagtatttaaagataccccaagaagctaattataacaagacgaactccaattcactgttccttgcattctaaaaccttaaataccagaaaacagctttttcaaagttgttttcaaagttggcgtataacatagtatcgacggagccgattttgaaaccgcggtgatcacaggcagcaacgctctgtcatcgttacaatcaacatgctaccctccgcgagatcatccgtgtttcaaacccggcagcttagttgccgttcttccgaatagcatcggtaacatgagcaaagtctgccgccttacaacggctctcccgctgacgccgtcccggactgatgggctgcctgtatcgagtggtgattttgtgccgagctgccggtcggggagctgttggctggctggtggcaggatatattgtggtgtaaacataacggatccggtctca

SEQ ID NO: 96 - DNA, 8362 bp, synthetic construct
  source 1..8362: mol_type = other DNA
gtcatgagacgaattctgacaggatatattggcgggtaaacctaagagaaaagagcgtttattagaataatcggatatttaaaagggcgtgaaaaggtttatccgttcgtccatttgtatgtgcatgccaaccacagggttcccctcgggatcaaagtactttgatccaacccctccgctgctatagtgcagtcggcttctgacgttcagtgcagccgtcatctgaaaacgacatgtcgcacaagtcctaagttacgcgacaggctgccgccctgcccttttcctggcgttttcttgtcgcgtgttttagtcgcataaagtagaatacttgcgactagaaccggagacattacgccatgaacaagagcgccgccgctggcctgctgggctatgcccgcgtcagcaccgacgaccaggacttgaccaaccaacgggccgaactgcacgcggccggctgcaccaagctgttttccgagaagatcaccggcaccaggcgcgaccgcccggagctggccaggatgcttgaccacctacgccctggcgacgttgtgacagtgaccaggctagaccgcctggcccgcagcacccgcgacctactggacattgccgagcgcatccaggaggccggcgcgggcctgcgtagcctggcagagccgtgggccgacaccaccacgccggccggccgcatggtgttgaccgtgttcgccggcattgccgagttcgagcgttccctaatcatcgaccgcacccggagcgggcgcgaggccgccaaggcccgaggcgtgaagtttggcccccgccctaccctcaccccggcacagatcgcgcacgcccgcgagctgatcgaccaggaaggccgcaccgtgaaagaggcggctgcactgcttggcgtgcatcgctcgaccctgtaccgcgcacttgagcgcagcgaggaagtgacgcccaccgaggccaggcggcgcggtgccttccgtgaggacgcattgaccgaggccgacgccctggcggccgccgagaatgaacgccaagaggaacaagcatgaaaccgcaccaggacggccaggacgaaccgtttttcattaccgaagagatcgaggcggagatgatcgcggccgggtacgtgttcgagccgcccgcgcacctctcaaccgtgcggctgcatgaaatcctggccggtttgtctgatgccaagctggcggcctggccggccagcttggccgctgaagaaaccgagcgccgccgtctaaaaaggtgatgtgtatttgagtaaaacagcttgcgtcatgcggtcgctgcgtatatgatccgatgagtaaataaacaaatacgcaaggggaacgcatgaaggttatcgctgtacttaaccagaaaggcgggtcaggcaagacgaccatcggaacccatctagcccgcgccctgcaactcgccggggccgatgttctgttagtcgattccgatccccagggcagtgcccgcgattgggcggccgtgcgggaagatcaaccgctaaccgttgtcggcatcgaccgcccgacgattgaccgcgacgtgaaggccatcggccggcgcgacttcgtagtgatcgacggagcgccccaggcggcggacttggctgtgtccgcgatcaaggcagccgacttcgtgctgattccggtgcagccaagcccttacgacatatgggccaccgccgacctggtggagctggttaagcagcgcattgaggtcacggatggaaggctacaagcggcctttgtcgtgtcgcgggcgatcaaaggcacgcgcatcggcggtgaggttgccgaggcgctggccgggtacgagctgcccattcttgagtcccgtatcacgcagcgcgtgagctacccaggcactgccgccgccggcacaaccgttcttgaatcagaacccgagggcgacgctgcccgcgaggtccaggcgctggccgctgaaattaaatcaaaactcatttgagttaatgaggtaaagagaaaatgagcaaaagcacaaacacgctaagtgccggccgtccgagcgcacgcagcagcaaggctgcaacgttggccagcctggcagacacgccagccatgaagcgggtcaactttcagttgccggcggaggatcacaccaagctgaagatgtacgcggtacgccaaggcaagaccattaccgagctgctatctgaatagatcgcgcagctaccagagtaaatgagcaaatgaataaatgagtagatgaattttagcggctaaaggaggcggcatggaaaatcaagaacaaccaggcaccgacgccgtggaatgccccatgtgtggaggaacgggcggttggccaggcgtaagcggctgggttgtctgccggccctgcaatggcactggaacccccaagcccgaggaatcggcgtgacggtcgcaaaccatccggcccggtacaaatcggcgcggcgctgggtgatgacctggtggagaagttgaaggccgcgcaggccgcccagcggcaacgcatcgaggcagaagcacgccccggtgaatcgtggcaagcggccgctgatcgaatccgcaaagaatcccggcaaccgccggcagccggtgcgccgtcgattaggaagccgcccaagggcgacgagcaaccagattttttcgttccgatgctctatgacgtgggcacccgcgatagtcgcagcatcatggacgtggccgttttccgtctgtcgaagcgtgaccgacgagctggcgaggtgatccgctacgagcttccagacgggcacgtagaggtttccgcagggccggccggcatggccagtgtgtgggattacgacctggtactgatggcggtttcccatctaaccgaatccatgaaccgataccgggaagggaagggagacaagcccggccgcgtgttccgtccacacgttgcggacgtactcaagttctgccggcgagccgatggcggaaagcagaaagacgacctggtagaaacctgcattcggttaaacaccacgcacgttgccatgcagcgtacgaagaaggccaagaacggccgcctggtgacggtatccgagggtgaagccttgattagccgctacaagatcgtaaagagcgaaaccgggcggccggagtacatcgagatcgagctagctgattggatgtaccgcgagatcacagaaggcaagaacccggacgtgctgacggttcaccccgattactttttgatcgatcccggcatcggccgttttctctaccgcctggcacgccgcgccgcaggcaaggcagaagccagatggttgttcaagacgatctacgaacgcagtggcagcgccggagagttcaagaagttctgtttcaccgtgcgcaagctgatcgggtcaaatgacctgccggagtacgatttgaaggaggaggcggggcaggctggcccgatcctagtcatgcgctaccgcaacctgatcgagggcgaagcatccgccggttcctaatgtacggagcagatgctagggcaaattgccctagcaggggaaaaaggtcgaaaaggactctttcctgtggatagcacgtacattgggaacccaaagccgtacattgggaaccggaacccgtacattgggaacccaaagccgtacattgggaaccggtcacacatgtaagtgactgatataaaagagaaaaaaggcgatttttccgcctaaaactctttaaaacttattaaaactcttaaaacccgcctggcctgtgcataactgtctggccagcgcacagccgaagagctgcaaaaagcgcctacccttcggtcgctgcgctccctacgccccgccgcttcgcgtcggcctatcgcggccgctggccgctcaaaaatggctggcctacggccaggcaatctaccagggcgcggacaagccgcgccgtcgccactcgaccgccggcgcccacatcaaggcaccctgcctcgcgcgtttcggtgatgacggtgaaaacctctgacacatgcagctcccggtgacggtcacagcttgtctgtaagcggatgccgggagcagacaagcccgtcagggcgcgtcagcgggtgttggcgggtgtcggggcgcagccatgacccagtcacgtagcgatagcggagtgtatactggcttaactatgcggcatcagagcagattgtactgagagtgcaccatatgcggtgtgaaataccgcacagatgcgtaaggagaaaataccgcatcaggcgctcttccgcttcctcgctcactgactcgctgcgctcggtcgttcggctgcggcgagcggtatcagctcactcaaaggcggtaatacggttatccacagaatcaggggataacgcaggaaagaacatgtgagcaaaaggccagcaaaaggccaggaaccgtaaaaaggccgcgttgctggcgtttttccataggctccgcccccctgacgagcatcacaaaaatcgacgctcaagtcagaggtggcgaaacccgacaggactataaagataccaggcgtttccccctggaagctccctcgtgcgctctcctgttccgaccctgccgcttaccggatacctgtccgcctttctcccttcgggaagcgtggcgctttctcatagctcacgctgtaggtatctcagttcggtgtaggtcgttcgctccaagctgggctgtgtgcacgaaccccccgttcagcccgaccgctgcgccttatccggtaactatcgtcttgagtccaacccggtaagacacgacttatcgccactggcagcagccactggtaacaggattagcagagcgaggtatgtaggcggtgctacagagttcttgaagtggtggcctaactacggctacactagaaggacagtatttggtatctgcgctctgctgaagccagttaccttcggaaaaagagttggtagctcttgatccggcaaacaaaccaccgctggtagcggtggtttttttgtttgcaagcagcagattacgcgcagaaaaaaaggatctcaagaagatcctttgatcttttctacggggtctgacgctcagtggaacgaaaactcacgttaagggattttggtcatgcattctaggtgattagaaaaactcatcgagcatcaaatgaaactgcaatttattcatatcaggattatcaataccatatttttgaaaaagccgtttctgtaatgaaggagaaaactcaccgaggcagttccataggatggcaagatcctggtatcggtctgcgattccgactcgtccaacatcaatacaacctattaatttcccctcgtcaaaaataaggttatcaagtgagaaatcaccatgagtgacgactgaatccggtgagaatggcaaaagtttatgcatttctttccagacttgttcaacaggccagccattacgctcgtcatcaaaatcactcgcatcaaccaaaccgttattcattcgtgattgcgcctgagcgagtcgaaatacgcgatcgctgttaaaaggacaattacaaacaggaatcgaatgcaaccggcgcaggaacactgccagcgcatcaacaatattttcacctgaatcaggatattcttctaatacctggaatgctgttttccctgggatcgcagtggtgagtaaccatgcatcatcaggagtacggataaaatgcttgatggtcggaagaggcataaattccgtcagccagtttagtctgaccatctcatctgtaacatcattggcaacgctacctttgccatgtttcagaaacaactctggcgcatcgggcttcccatacaatcggtagattgtcgcacctgattgcccgacattatcgcgagcccatttatacccatataaatcagcatccatgttggaatttaatcgcggccttgagcaagacgtttcccgttgaatatggctcataacagaacttattatttccttcctcttttctacagtatttaaagataccccaagaagctaattataacaagacgaactccaattcactgttccttgcattctaaaaccttaaataccagaaaacagctttttcaaagttgttttcaaagttggcgtataacatagtatcgacggagccgattttgaaaccgcggtgatcacaggcagcaacgctctgtcatcgttacaatcaacatgctaccctccgcgagatcatccgtgtttcaaacccggcagcttagttgccgttcttccgaatagcatcggtaacatgagcaaagtctgccgccttacaacggctctcccgctgacgccgtcccggactgatgggctgcctgtatcgagtggtgattttgtgccgagctgccggtcggggagctgttggctggctggtggcaggatatattgtggtgtaaacataacgaattcgtctcaggagactagagccaagctgatctcctttgccccggagatcaccatggacgactttctctatctctacgatctaggaagaaagttcgacggagaaggtgacgataccatgttcaccaccgataatgagaagattagcctcttcaatttcagaaagaatgctgacccacagatggttagagaggcctacgcggcaggtctgatcaagacgatctacccgagtaataatctccaggagatcaaataccttcccaagaaggttaaagatgcagtcaaaagattcaggactaactgcatcaagaacacagagaaagatatatttctcaagatcagaagtactattccagtatggacgattcaaggcttgcttcataaaccaaggcaagtaatagagattggagtctctaagaaagtagttcctactgaatcaaaggccatggagtcaaaaattcagatcgaggatctaacagaactcgccgtgaagactggcgaacagttcatacagagtcttttacgactcaatgacaagaagaaaatcttcgtcaacatggtggagcacgacactctcgtctactccaagaatatcaaagatacagtctcagaagaccaaagggctattgagacttttcaacaaagggtaatatcgggaaacctcctcggattccattgcccagctatctgtcacttcatcaaaaggacagtagaaaaggaaggtggcacctacaaatgccatcattgcgataaaggaaaggctatcgttcaagatgcctctgccgacagtggtcccaaagatggacccccacccacgaggagcatcgtggaaaaagaagacgttccaaccacgtcttcaaagcaagtggattgatgtgatatctccactgacgtaagggatgacgcacaatcccactatccttcgcaagacccttcctctatataaggaagttcatttcatttggagaggactccggtatttttacaacaataccacaacaaaacaaacaacaaacaacattacaatttactattctagtcgaaatggtgagcaagggcgaggagctgttcaccggggtggtgcccatcctggtcgagctggacggcgacgtaaacggccacaagttcagcgtgtccggcgagggcgagggcgatgccacctacggcaagctgaccctgaagttcatctgcaccaccggcaagctgcccgtgccctggcccaccctcgtgaccaccctgacctacggcgtgcagtgcttcagccgctaccccgaccacatgaagcagcacgacttcttcaagtccgccatgcccgaaggctacgtccaggagcgcaccatcttcttcaaggacgacggcaactacaagacccgcgccgaggtgaagttcgagggcgacaccctggtgaaccgcatcgagctgaagggcatcgacttcaaggaggacggcaacatcctggggcacaagctggagtacaactacaacagccacaacgtctatatcatggccgacaagcagaagaacggcatcaaggtgaacttcaagatccgccacaacatcgaggacggcagcgtgcagctcgccgaccactaccagcagaacacccccatcggcgacggccccgtgctgctgcccgacaaccactacctgagcacccagtccgccctgagcaaagaccccaacgagaagcgcgatcacatggtcctgctggagttcgtgaccgccgccgggatcactctcggcatggacgagctgtacaaggacgagctgtaagcttcggccatgctagagtccgcaaaaatcaccagtctctctctacaaatctatctctctctatttttctccagaataatgtgtgagtagttcccagataagggaattagggttcttatagggtttcgctcatgtgttgagcatataagaaacccttagtatgtatttgtatttgtaaaatacttctatcaataaaatttctaattcctaaaaccaaaatccagtgacctcgct

SEQ ID NO: 97 - DNA, 10139 bp, synthetic construct
  source 1..10139: mol_type = other DNA
ggaggtgccaagcttgcatgcctgcaggtagcagaaggcatgttgttgtgactccgaggggttgcctcaaactctatcttataaccggcgtggaggcatggaggcaggggtattttggtcattttaatagatagtggaaaatgacgtggaatttacttaaagacgaagtctttgcgacaagggggggcccacgccgaatttaatattaccggcgtggcccccccttatcgcgagtgctttagcacgagcggtccagatttaaagtagaaaatttcccgcccactagggttaaaggtgttcacactataaaagcatatacgatgtgatggtatttgatggagcgtatattgtatcaggtatttccgttggatacgaattattcgtacgaccctccctaagattcttgattgtttcgctgtcaggagtctcaatggtaactttactctttatttaaccatacatttttttttatttttttcactttgttcttcatccactattgttctttgttcatcttgaacaaaagctccctccttctttgttcttcatccaccattgttcttcatcaatcatttcgctgtcaggagactagagccaagctgatctcctttgccccggagatcaccatggacgactttctctatctctacgatctaggaagaaagttcgacggagaaggtgacgataccatgttcaccaccgataatgagaagattagcctcttcaatttcagaaagaatgctgacccacagatggttagagaggcctacgcggcaggtctgatcaagacgatctacccgagtaataatctccaggagatcaaataccttcccaagaaggttaaagatgcagtcaaaagattcaggactaactgcatcaagaacacagagaaagatatatttctcaagatcagaagtactattccagtatggacgattcaaggcttgcttcataaaccaaggcaagtaatagagattggagtctctaagaaagtagttcctactgaatcaaaggccatggagtcaaaaattcagatcgaggatctaacagaactcgccgtgaagactggcgaacagttcatacagagtcttttacgactcaatgacaagaagaaaatcttcgtcaacatggtggagcacgacactctcgtctactccaagaatatcaaagatacagtctcagaagaccaaagggctattgagacttttcaacaaagggtaatatcgggaaacctcctcggattccattgcccagctatctgtcacttcatcaaaaggacagtagaaaaggaaggtggcacctacaaatgccatcattgcgataaaggaaaggctatcgttcaagatgcctctgccgacagtggtcccaaagatggacccccacccacgaggagcatcgtggaaaaagaagacgttccaaccacgtcttcaaagcaagtggattgatgtgatatctccactgacgtaagggatgacgcacaatcccactatccttcgcaagacccttcctctatataaggaagttcatttcatttggagaggactccggtatttttacaacaataccacaacaaaacaaacaacaaacaacattacaatttactattctagtcgaaatggtgagcaagggcgaggagctgttcaccggggtggtgcccatcctggtcgagctggacggcgacgtaaacggccacaagttcagcgtgtccggcgagggcgagggcgatgccacctacggcaagctgaccctgaagttcatctgcaccaccggcaagctgcccgtgccctggcccaccctcgtgaccaccctgacctacggcgtgcagtgcttcagccgctaccccgaccacatgaagcagcacgacttcttcaagtccgccatgcccgaaggctacgtccaggagcgcaccatcttcttcaaggacgacggcaactacaagacccgcgccgaggtgaagttcgagggcgacaccctggtgaaccgcatcgagctgaagggcatcgacttcaaggaggacggcaacatcctggggcacaagctggagtacaactacaacagccacaacgtctatatcatggccgacaagcagaagaacggcatcaaggtgaacttcaagatccgccacaacatcgaggacggcagcgtgcagctcgccgaccactaccagcagaacacccccatcggcgacggccccgtgctgctgcccgacaaccactacctgagcacccagtccgccctgagcaaagaccccaacgagaagcgcgatcacatggtcctgctggagttcgtgaccgccgccgggatcactctcggcatggacgagctgtacaaggacgagctgtaagcttcggccatgctagagtccgcaaaaatcaccagtctctctctacaaatctatctctctctatttttctccagaataatgtgtgagtagttcccagataagggaattagggttcttatagggtttcgctcatgtgttgagcatataagaaacccttagtatgtatttgtatttgtaaaatacttctatcaataaaatttctaattcctaaaaccaaaatccagtgacctcgctgtcaggaggagtgtacttcaagtcagtgggaaatcaataaaatgattattttatgaatatatttcattgtgcaagtagatagaaattacatatgttacataacacacgaaataaacaaaaaaagacaatccaaaaacaaacaccccaaaaaaaataatcactttagataaactcgtatgaggagaggcacgttcagtgactcgacgattcccgagcaaaaaaagtctccccgtcacacatgtagtgggtgacgcaattatctttaaagtaatccttctgttgacttgtcattgataacatccagtcttcgtcaggattgcaaagaattatagaagggatcccactcgagcgctgtcaggagggagaggtaagtttcacttcacacattattactgtcttctaatacaaggttttttatcaagctggagaagagcatgatagtgggtagtgccatcttgatgaagctcagaagcaacaccaaggaagaaaataagaaaaggtgtgagtttctcccagagaaactggaataaatcatctctttgagatgagcacttgggataggtaaggaaaacatatttagattggagtctgaagttcttactagcagaaggcatgttgttgtgactccgaggggttgcctcaaactctatcttataaccggcgtggaggcatggaggcaggggtattttggtcattttaatagatagtggaaaatgacgtggaatttacttaaagacgaagtctttgcgacaagggggggcccacgccgaatttaatattaccggcgtggcccccccttatcgcgagtgctttagcacgagcggtccagatttaaagtagaaaatttcccgcccactagggttaaaggtgttcacactataaaagcatatacgatgtgatggtatttgatggagcgtatattgtatcaggtatttccgttggatacgaattattcgtacgaccctccctgcaggtcgactctagaggatccccgggtaccgagctcgaattcgtaatcatggtcatagcgctgtcaggagtctcaatggtaactttactctttatttaaccatacatttttttttatttttttcactttgttcttcatccactattgttctttgttcatcttgaacaaaagctccctccttctttgttcttcatccaccattgttcttcatcaatcatttcgctgtcatgagacgaattctgacaggatatattggcgggtaaacctaagagaaaagagcgtttattagaataatcggatatttaaaagggcgtgaaaaggtttatccgttcgtccatttgtatgtgcatgccaaccacagggttcccctcgggatcaaagtactttgatccaacccctccgctgctatagtgcagtcggcttctgacgttcagtgcagccgtcatctgaaaacgacatgtcgcacaagtcctaagttacgcgacaggctgccgccctgcccttttcctggcgttttcttgtcgcgtgttttagtcgcataaagtagaatacttgcgactagaaccggagacattacgccatgaacaagagcgccgccgctggcctgctgggctatgcccgcgtcagcaccgacgaccaggacttgaccaaccaacgggccgaactgcacgcggccggctgcaccaagctgttttccgagaagatcaccggcaccaggcgcgaccgcccggagctggccaggatgcttgaccacctacgccctggcgacgttgtgacagtgaccaggctagaccgcctggcccgcagcacccgcgacctactggacattgccgagcgcatccaggaggccggcgcgggcctgcgtagcctggcagagccgtgggccgacaccaccacgccggccggccgcatggtgttgaccgtgttcgccggcattgccgagttcgagcgttccctaatcatcgaccgcacccggagcgggcgcgaggccgccaaggcccgaggcgtgaagtttggcccccgccctaccctcaccccggcacagatcgcgcacgcccgcgagctgatcgaccaggaaggccgcaccgtgaaagaggcggctgcactgcttggcgtgcatcgctcgaccctgtaccgcgcacttgagcgcagcgaggaagtgacgcccaccgaggccaggcggcgcggtgccttccgtgaggacgcattgaccgaggccgacgccctggcggccgccgagaatgaacgccaagaggaacaagcatgaaaccgcaccaggacggccaggacgaaccgtttttcattaccgaagagatcgaggcggagatgatcgcggccgggtacgtgttcgagccgcccgcgcacctctcaaccgtgcggctgcatgaaatcctggccggtttgtctgatgccaagctggcggcctggccggccagcttggccgctgaagaaaccgagcgccgccgtctaaaaaggtgatgtgtatttgagtaaaacagcttgcgtcatgcggtcgctgcgtatatgatccgatgagtaaataaacaaatacgcaaggggaacgcatgaaggttatcgctgtacttaaccagaaaggcgggtcaggcaagacgaccatcggaacccatctagcccgcgccctgcaactcgccggggccgatgttctgttagtcgattccgatccccagggcagtgcccgcgattgggcggccgtgcgggaagatcaaccgctaaccgttgtcggcatcgaccgcccgacgattgaccgcgacgtgaaggccatcggccggcgcgacttcgtagtgatcgacggagcgccccaggcggcggacttggctgtgtccgcgatcaaggcagccgacttcgtgctgattccggtgcagccaagcccttacgacatatgggccaccgccgacctggtggagctggttaagcagcgcattgaggtcacggatggaaggctacaagcggcctttgtcgtgtcgcgggcgatcaaaggcacgcgcatcggcggtgaggttgccgaggcgctggccgggtacgagctgcccattcttgagtcccgtatcacgcagcgcgtgagctacccaggcactgccgccgccggcacaaccgttcttgaatcagaacccgagggcgacgctgcccgcgaggtccaggcgctggccgctgaaattaaatcaaaactcatttgagttaatgaggtaaagagaaaatgagcaaaagcacaaacacgctaagtgccggccgtccgagcgcacgcagcagcaaggctgcaacgttggccagcctggcagacacgccagccatgaagcgggtcaactttcagttgccggcggaggatcacaccaagctgaagatgtacgcggtacgccaaggcaagaccattaccgagctgctatctgaatagatcgcgcagctaccagagtaaatgagcaaatgaataaatgagtagatgaattttagcggctaaaggaggcggcatggaaaatcaagaacaaccaggcaccgacgccgtggaatgccccatgtgtggaggaacgggcggttggccaggcgtaagcggctgggttgtctgccggccctgcaatggcactggaacccccaagcccgaggaatcggcgtgacggtcgcaaaccatccggcccggtacaaatcggcgcggcgctgggtgatgacctggtggagaagttgaaggccgcgcaggccgcccagcggcaacgcatcgaggcagaagcacgccccggtgaatcgtggcaagcggccgctgatcgaatccgcaaagaatcccggcaaccgccggcagccggtgcgccgtcgattaggaagccgcccaagggcgacgagcaaccagattttttcgttccgatgctctatgacgtgggcacccgcgatagtcgcagcatcatggacgtggccgttttccgtctgtcgaagcgtgaccgacgagctggcgaggtgatccgctacgagcttccagacgggcacgtagaggtttccgcagggccggccggcatggccagtgtgtgggattacgacctggtactgatggcggtttcccatctaaccgaatccatgaaccgataccgggaagggaagggagacaagcccggccgcgtgttccgtccacacgttgcggacgtactcaagttctgccggcgagccgatggcggaaagcagaaagacgacctggtagaaacctgcattcggttaaacaccacgcacgttgccatgcagcgtacgaagaaggccaagaacggccgcctggtgacggtatccgagggtgaagccttgattagccgctacaagatcgtaaagagcgaaaccgggcggccggagtacatcgagatcgagctagctgattggatgtaccgcgagatcacagaaggcaagaacccggacgtgctgacggttcaccccgattactttttgatcgatcccggcatcggccgttttctctaccgcctggcacgccgcgccgcaggcaaggcagaagccagatggttgttcaagacgatctacgaacgcagtggcagcgccggagagttcaagaagttctgtttcaccgtgcgcaagctgatcgggtcaaatgacctgccggagtacgatttgaaggaggaggcggggcaggctggcccgatcctagtcatgcgctaccgcaacctgatcgagggcgaagcatccgccggttcctaatgtacggagcagatgctagggcaaattgccctagcaggggaaaaaggtcgaaaaggactctttcctgtggatagcacgtacattgggaacccaaagccgtacattgggaaccggaacccgtacattgggaacccaaagccgtacattgggaaccggtcacacatgtaagtgactgatataaaagagaaaaaaggcgatttttccgcctaaaactctttaaaacttattaaaactcttaaaacccgcctggcctgtgcataactgtctggccagcgcacagccgaagagctgcaaaaagcgcctacccttcggtcgctgcgctccctacgccccgccgcttcgcgtcggcctatcgcggccgctggccgctcaaaaatggctggcctacggccaggcaatctaccagggcgcggacaagccgcgccgtcgccactcgaccgccggcgcccacatcaaggcaccctgcctcgcgcgtttcggtgatgacggtgaaaacctctgacacatgcagctcccggtgacggtcacagcttgtctgtaagcggatgccgggagcagacaagcccgtcagggcgcgtcagcgggtgttggcgggtgtcggggcgcagccatgacccagtcacgtagcgatagcggagtgtatactggcttaactatgcggcatcagagcagattgtactgagagtgcaccatatgcggtgtgaaataccgcacagatgcgtaaggagaaaataccgcatcaggcgctcttccgcttcctcgctcactgactcgctgcgctcggtcgttcggctgcggcgagcggtatcagctcactcaaaggcggtaatacggttatccacagaatcaggggataacgcaggaaagaacatgtgagcaaaaggccagcaaaaggccaggaaccgtaaaaaggccgcgttgctggcgtttttccataggctccgcccccctgacgagcatcacaaaaatcgacgctcaagtcagaggtggcgaaacccgacaggactataaagataccaggcgtttccccctggaagctccctcgtgcgctctcctgttccgaccctgccgcttaccggatacctgtccgcctttctcccttcgggaagcgtggcgctttctcatagctcacgctgtaggtatctcagttcggtgtaggtcgttcgctccaagctgggctgtgtgcacgaaccccccgttcagcccgaccgctgcgccttatccggtaactatcgtcttgagtccaacccggtaagacacgacttatcgccactggcagcagccactggtaacaggattagcagagcgaggtatgtaggcggtgctacagagttcttgaagtggtggcctaactacggctacactagaaggacagtatttggtatctgcgctctgctgaagccagttaccttcggaaaaagagttggtagctcttgatccggcaaacaaaccaccgctggtagcggtggtttttttgtttgcaagcagcagattacgcgcagaaaaaaaggatctcaagaagatcctttgatcttttctacggggtctgacgctcagtggaacgaaaactcacgttaagggattttggtcatgcattctaggtgattagaaaaactcatcgagcatcaaatgaaactgcaatttattcatatcaggattatcaataccatatttttgaaaaagccgtttctgtaatgaaggagaaaactcaccgaggcagttccataggatggcaagatcctggtatcggtctgcgattccgactcgtccaacatcaatacaacctattaatttcccctcgtcaaaaataaggttatcaagtgagaaatcaccatgagtgacgactgaatccggtgagaatggcaaaagtttatgcatttctttccagacttgttcaacaggccagccattacgctcgtcatcaaaatcactcgcatcaaccaaaccgttattcattcgtgattgcgcctgagcgagtcgaaatacgcgatcgctgttaaaaggacaattacaaacaggaatcgaatgcaaccggcgcaggaacactgccagcgcatcaacaatattttcacctgaatcaggatattcttctaatacctggaatgctgttttccctgggatcgcagtggtgagtaaccatgcatcatcaggagtacggataaaatgcttgatggtcggaagaggcataaattccgtcagccagtttagtctgaccatctcatctgtaacatcattggcaacgctacctttgccatgtttcagaaacaactctggcgcatcgggcttcccatacaatcggtagattgtcgcacctgattgcccgacattatcgcgagcccatttatacccatataaatcagcatccatgttggaatttaatcgcggccttgagcaagacgtttcccgttgaatatggctcataacagaacttattatttccttcctcttttctacagtatttaaagataccccaagaagctaattataacaagacgaactccaattcactgttccttgcattctaaaaccttaaataccagaaaacagctttttcaaagttgttttcaaagttggcgtataacatagtatcgacggagccgattttgaaaccgcggtgatcacaggcagcaacgctctgtcatcgttacaatcaacatgctaccctccgcgagatcatccgtgtttcaaacccggcagcttagttgccgttcttccgaatagcatcggtaacatgagcaaagtctgccgccttacaacggctctcccgctgacgccgtcccggactgatgggctgcctgtatcgagtggtgattttgtgccgagctgccggtcggggagctgttggctggctggtggcaggatatattgtggtgtaaacataacgaattcgtctca

SEQ ID NO: 98 - DNA, 10264 bp, synthetic construct
  source 1..10264: mol_type = other DNA
ggaggtgccaagcttgcatgcctgcaggtagcagaaggcatgttgttgtgactccgaggggttgcctcaaactctatcttataaccggcgtggaggcatggaggcaggggtattttggtcattttaatagatagtggaaaatgacgtggaatttacttaaagacgaagtctttgcgacaagggggggcccacgccgaatttaatattaccggcgtggcccccccttatcgcgagtgctttagcacgagcggtccagatttaaagtagaaaatttcccgcccactagggttaaaggtgttcacactataaaagcatatacgatgtgatggtatttgatggagcgtatattgtatcaggtatttccgttggatacgaattattcgtacgaccctccctaagattcttgattgtttcgctgtcaggagactagagccaagctgatctcctttgccccggagatcaccatggacgactttctctatctctacgatctaggaagaaagttcgacggagaaggtgacgataccatgttcaccaccgataatgagaagattagcctcttcaatttcagaaagaatgctgacccacagatggttagagaggcctacgcggcaggtctgatcaagacgatctacccgagtaataatctccaggagatcaaataccttcccaagaaggttaaagatgcagtcaaaagattcaggactaactgcatcaagaacacagagaaagatatatttctcaagatcagaagtactattccagtatggacgattcaaggcttgcttcataaaccaaggcaagtaatagagattggagtctctaagaaagtagttcctactgaatcaaaggccatggagtcaaaaattcagatcgaggatctaacagaactcgccgtgaagactggcgaacagttcatacagagtcttttacgactcaatgacaagaagaaaatcttcgtcaacatggtggagcacgacactctcgtctactccaagaatatcaaagatacagtctcagaagaccaaagggctattgagacttttcaacaaagggtaatatcgggaaacctcctcggattccattgcccagctatctgtcacttcatcaaaaggacagtagaaaaggaaggtggcacctacaaatgccatcattgcgataaaggaaaggctatcgttcaagatgcctctgccgacagtggtcccaaagatggacccccacccacgaggagcatcgtggaaaaagaagacgttccaaccacgtcttcaaagcaagtggattgatgtgatatctccactgacgtaagggatgacgcacaatcccactatccttcgcaagacccttcctctatataaggaagttcatttcatttggagaggactccggtatttttacaacaataccacaacaaaacaaacaacaaacaacattacaatttactattctagtcgaaatggctttgtggtacttgttcaataaaaggagtcttggtgcagctgtccttatacttgttgggctgttaatgtgcaatattcaaatgacaggagctcaggtgcagctccaagaaagcggagggggtctggtgcaagctgggggttctttgagattatcctgtgcagctagcggacgtacatttagcgaatatgcaatgggttggttccgtcaggccccaggaaaggagcgagagttcgttgctactattagttggtccggtggctctacatactacaccgactctgtaaaaggacgttttactatttcaagggataatgctaagaacacagtgtatttacaaatgaatagcctcaaaccggacgatacagcagtatactattgcgctgctgctggacttggcactgtagtatccgaatgggattacgactacgactactggggtcaggggactcaggtcacggtgtcctccgcaggggagcccaaatcttgtgacaaaactcacacatgcccaccgtgcccagcacctgaactcctggggggaccgtcagtcttcctcttccccccaaaacccaaggacaccctcatgatctcccggacccctgaggtcacatgcgtggtggtggacgtgagccacgaagaccctgaggtcaagttcaactggtacgtggacggcgtggaggtgcataatgccaagacaaagccgcgggaggagcagtacaacagcacgtaccgtgtggtcagcgtcctcaccgtcctgcaccaggactggctgaatggcaaggagtacaagtgcaaggtgtcaaacaaagccctcccagcccccatcgagaaaaccatctccaaagccaaagggcagccccgagaaccacaggtgtacaccctgcccccatcccgggaggagatgaccaagaaccaggtcagcctgacctgcctggtcaaaggcttctaccccagcgacattgcggtggagtgggagagcaatgggcagccggagaacaactacaagaccacacctcccatgctggactccgacggctccttcttcctctacagcaagctcaccgtggacaagagcaggtggcagcaggggaacgtcttctcatgctccgtgatgcatgaggctctgcacaaccactacacgcagaagagcctctccctgtctccgggtaaatgagcttcggccatgctagagtccgcaaaaatcaccagtctctctctacaaatctatctctctctatttttctccagaataatgtgtgagtagttcccagataagggaattagggttcttatagggtttcgctcatgtgttgagcatataagaaacccttagtatgtatttgtatttgtaaaatacttctatcaataaaatttctaattcctaaaaccaaaatccagtgacctcgctgtcaggaggagtgtacttcaagtcagtgggaaatcaataaaatgattattttatgaatatatttcattgtgcaagtagatagaaattacatatgttacataacacacgaaataaacaaaaaaagacaatccaaaaacaaacaccccaaaaaaaataatcactttagataaactcgtatgaggagaggcacgttcagtgactcgacgattcccgagcaaaaaaagtctccccgtcacacatgtagtgggtgacgcaattatctttaaagtaatccttctgttgacttgtcattgataacatccagtcttcgtcaggattgcaaagaattatagaagggatcccactcgagcgctgtcaggagggagaggtaagtttcacttcacacattattactgtcttctaatacaaggttttttatcaagctggagaagagcatgatagtgggtagtgccatcttgatgaagctcagaagcaacaccaaggaagaaaataagaaaaggtgtgagtttctcccagagaaactggaataaatcatctctttgagatgagcacttgggataggtaaggaaaacatatttagattggagtctgaagttcttactagcagaaggcatgttgttgtgactccgaggggttgcctcaaactctatcttataaccggcgtggaggcatggaggcaggggtattttggtcattttaatagatagtggaaaatgacgtggaatttacttaaagacgaagtctttgcgacaagggggggcccacgccgaatttaatattaccggcgtggcccccccttatcgcgagtgctttagcacgagcggtccagatttaaagtagaaaatttcccgcccactagggttaaaggtgttcacactataaaagcatatacgatgtgatggtatttgatggagcgtatattgtatcaggtatttccgttggatacgaattattcgtacgaccctccctgcaggtcgactctagaggatccccgggtaccgagctcgaattcgtaatcatggtcatagcgcttgagacgaagctttgacaggatatattggcgggtaaacctaagagaaaagagcgtttattagaataatcggatatttaaaagggcgtgaaaaggtttatccgttcgtccatttgtatgtgcatgccaaccacagggttcccctcgggatcaaagtactttgatccaacccctccgctgctatagtgcagtcggcttctgacgttcagtgcagccgtcatctgaaaacgacatgtcgcacaagtcctaagttacgcgacaggctgccgccctgcccttttcctggcgttttcttgtcgcgtgttttagtcgcataaagtagaatacttgcgactagaaccggagacattacgccatgaacaagagcgccgccgctggcctgctgggctatgcccgcgtcagcaccgacgaccaggacttgaccaaccaacgggccgaactgcacgcggccggctgcaccaagctgttttccgagaagatcaccggcaccaggcgcgaccgcccggagctggccaggatgcttgaccacctacgccctggcgacgttgtgacagtgaccaggctagaccgcctggcccgcagcacccgcgacctactggacattgccgagcgcatccaggaggccggcgcgggcctgcgtagcctggcagagccgtgggccgacaccaccacgccggccggccgcatggtgttgaccgtgttcgccggcattgccgagttcgagcgttccctaatcatcgaccgcacccggagcgggcgcgaggccgccaaggcccgaggcgtgaagtttggcccccgccctaccctcaccccggcacagatcgcgcacgcccgcgagctgatcgaccaggaaggccgcaccgtgaaagaggcggctgcactgcttggcgtgcatcgctcgaccctgtaccgcgcacttgagcgcagcgaggaagtgacgcccaccgaggccaggcggcgcggtgccttccgtgaggacgcattgaccgaggccgacgccctggcggccgccgagaatgaacgccaagaggaacaagcatgaaaccgcaccaggacggccaggacgaaccgtttttcattaccgaagagatcgaggcggagatgatcgcggccgggtacgtgttcgagccgcccgcgcacctctcaaccgtgcggctgcatgaaatcctggccggtttgtctgatgccaagctggcggcctggccggccagcttggccgctgaagaaaccgagcgccgccgtctaaaaaggtgatgtgtatttgagtaaaacagcttgcgtcatgcggtcgctgcgtatatgatccgatgagtaaataaacaaatacgcaaggggaacgcatgaaggttatcgctgtacttaaccagaaaggcgggtcaggcaagacgaccatcggaacccatctagcccgcgccctgcaactcgccggggccgatgttctgttagtcgattccgatccccagggcagtgcccgcgattgggcggccgtgcgggaagatcaaccgctaaccgttgtcggcatcgaccgcccgacgattgaccgcgacgtgaaggccatcggccggcgcgacttcgtagtgatcgacggagcgccccaggcggcggacttggctgtgtccgcgatcaaggcagccgacttcgtgctgattccggtgcagccaagcccttacgacatatgggccaccgccgacctggtggagctggttaagcagcgcattgaggtcacggatggaaggctacaagcggcctttgtcgtgtcgcgggcgatcaaaggcacgcgcatcggcggtgaggttgccgaggcgctggccgggtacgagctgcccattcttgagtcccgtatcacgcagcgcgtgagctacccaggcactgccgccgccggcacaaccgttcttgaatcagaacccgagggcgacgctgcccgcgaggtccaggcgctggccgctgaaattaaatcaaaactcatttgagttaatgaggtaaagagaaaatgagcaaaagcacaaacacgctaagtgccggccgtccgagcgcacgcagcagcaaggctgcaacgttggccagcctggcagacacgccagccatgaagcgggtcaactttcagttgccggcggaggatcacaccaagctgaagatgtacgcggtacgccaaggcaagaccattaccgagctgctatctgaatagatcgcgcagctaccagagtaaatgagcaaatgaataaatgagtagatgaattttagcggctaaaggaggcggcatggaaaatcaagaacaaccaggcaccgacgccgtggaatgccccatgtgtggaggaacgggcggttggccaggcgtaagcggctgggttgtctgccggccctgcaatggcactggaacccccaagcccgaggaatcggcgtgacggtcgcaaaccatccggcccggtacaaatcggcgcggcgctgggtgatgacctggtggagaagttgaaggccgcgcaggccgcccagcggcaacgcatcgaggcagaagcacgccccggtgaatcgtggcaagcggccgctgatcgaatccgcaaagaatcccggcaaccgccggcagccggtgcgccgtcgattaggaagccgcccaagggcgacgagcaaccagattttttcgttccgatgctctatgacgtgggcacccgcgatagtcgcagcatcatggacgtggccgttttccgtctgtcgaagcgtgaccgacgagctggcgaggtgatccgctacgagcttccagacgggcacgtagaggtttccgcagggccggccggcatggccagtgtgtgggattacgacctggtactgatggcggtttcccatctaaccgaatccatgaaccgataccgggaagggaagggagacaagcccggccgcgtgttccgtccacacgttgcggacgtactcaagttctgccggcgagccgatggcggaaagcagaaagacgacctggtagaaacctgcattcggttaaacaccacgcacgttgccatgcagcgtacgaagaaggccaagaacggccgcctggtgacggtatccgagggtgaagccttgattagccgctacaagatcgtaaagagcgaaaccgggcggccggagtacatcgagatcgagctagctgattggatgtaccgcgagatcacagaaggcaagaacccggacgtgctgacggttcaccccgattactttttgatcgatcccggcatcggccgttttctctaccgcctggcacgccgcgccgcaggcaaggcagaagccagatggttgttcaagacgatctacgaacgcagtggcagcgccggagagttcaagaagttctgtttcaccgtgcgcaagctgatcgggtcaaatgacctgccggagtacgatttgaaggaggaggcggggcaggctggcccgatcctagtcatgcgctaccgcaacctgatcgagggcgaagcatccgccggttcctaatgtacggagcagatgctagggcaaattgccctagcaggggaaaaaggtcgaaaaggactctttcctgtggatagcacgtacattgggaacccaaagccgtacattgggaaccggaacccgtacattgggaacccaaagccgtacattgggaaccggtcacacatgtaagtgactgatataaaagagaaaaaaggcgatttttccgcctaaaactctttaaaacttattaaaactcttaaaacccgcctggcctgtgcataactgtctggccagcgcacagccgaagagctgcaaaaagcgcctacccttcggtcgctgcgctccctacgccccgccgcttcgcgtcggcctatcgcggccgctggccgctcaaaaatggctggcctacggccaggcaatctaccagggcgcggacaagccgcgccgtcgccactcgaccgccggcgcccacatcaaggcaccctgcctcgcgcgtttcggtgatgacggtgaaaacctctgacacatgcagctcccggtgacggtcacagcttgtctgtaagcggatgccgggagcagacaagcccgtcagggcgcgtcagcgggtgttggcgggtgtcggggcgcagccatgacccagtcacgtagcgatagcggagtgtatactggcttaactatgcggcatcagagcagattgtactgagagtgcaccatatgcggtgtgaaataccgcacagatgcgtaaggagaaaataccgcatcaggcgctcttccgcttcctcgctcactgactcgctgcgctcggtcgttcggctgcggcgagcggtatcagctcactcaaaggcggtaatacggttatccacagaatcaggggataacgcaggaaagaacatgtgagcaaaaggccagcaaaaggccaggaaccgtaaaaaggccgcgttgctggcgtttttccataggctccgcccccctgacgagcatcacaaaaatcgacgctcaagtcagaggtggcgaaacccgacaggactataaagataccaggcgtttccccctggaagctccctcgtgcgctctcctgttccgaccctgccgcttaccggatacctgtccgcctttctcccttcgggaagcgtggcgctttctcatagctcacgctgtaggtatctcagttcggtgtaggtcgttcgctccaagctgggctgtgtgcacgaaccccccgttcagcccgaccgctgcgccttatccggtaactatcgtcttgagtccaacccggtaagacacgacttatcgccactggcagcagccactggtaacaggattagcagagcgaggtatgtaggcggtgctacagagttcttgaagtggtggcctaactacggctacactagaaggacagtatttggtatctgcgctctgctgaagccagttaccttcggaaaaagagttggtagctcttgatccggcaaacaaaccaccgctggtagcggtggtttttttgtttgcaagcagcagattacgcgcagaaaaaaaggatctcaagaagatcctttgatcttttctacggggtctgacgctcagtggaacgaaaactcacgttaagggattttggtcatgcattctaggtgattagaaaaactcatcgagcatcaaatgaaactgcaatttattcatatcaggattatcaataccatatttttgaaaaagccgtttctgtaatgaaggagaaaactcaccgaggcagttccataggatggcaagatcctggtatcggtctgcgattccgactcgtccaacatcaatacaacctattaatttcccctcgtcaaaaataaggttatcaagtgagaaatcaccatgagtgacgactgaatccggtgagaatggcaaaagtttatgcatttctttccagacttgttcaacaggccagccattacgctcgtcatcaaaatcactcgcatcaaccaaaccgttattcattcgtgattgcgcctgagcgagtcgaaatacgcgatcgctgttaaaaggacaattacaaacaggaatcgaatgcaaccggcgcaggaacactgccagcgcatcaacaatattttcacctgaatcaggatattcttctaatacctggaatgctgttttccctgggatcgcagtggtgagtaaccatgcatcatcaggagtacggataaaatgcttgatggtcggaagaggcataaattccgtcagccagtttagtctgaccatctcatctgtaacatcattggcaacgctacctttgccatgtttcagaaacaactctggcgcatcgggcttcccatacaatcggtagattgtcgcacctgattgcccgacattatcgcgagcccatttatacccatataaatcagcatccatgttggaatttaatcgcggccttgagcaagacgtttcccgttgaatatggctcataacagaacttattatttccttcctcttttctacagtatttaaagataccccaagaagctaattataacaagacgaactccaattcactgttccttgcattctaaaaccttaaataccagaaaacagctttttcaaagttgttttcaaagttggcgtataacatagtatcgacggagccgattttgaaaccgcggtgatcacaggcagcaacgctctgtcatcgttacaatcaacatgctaccctccgcgagatcatccgtgtttcaaacccggcagcttagttgccgttcttccgaatagcatcggtaacatgagcaaagtctgccgccttacaacggctctcccgctgacgccgtcccggactgatgggctgcctgtatcgagtggtgattttgtgccgagctgccggtcggggagctgttggctggctggtggcaggatatattgtggtgtaaacataacaagcttcgtctcagtca

SEQ ID NO: 99 - DNA, 20 bp, synthetic construct
  source 1..20: mol_type = other DNA
agggaagtcaacaatgcatg

SEQ ID NO: 100 - DNA, 20 bp, synthetic construct
  source 1..20: mol_type = other DNA
atcaggatccaccataacct

SEQ ID NO: 101 - DNA, 20 bp, synthetic construct
  source 1..20: mol_type = other DNA
agtttgtatctgtagttgct

SEQ ID NO: 102 - DNA, 20 bp, synthetic construct
  source 1..20: mol_type = other DNA
aaggaagtcaacaatgcatg

SEQ ID NO: 103 - DNA, 20 bp, synthetic construct
  source 1..20: mol_type = other DNA
ccagagtgtaaaaggtacga

SEQ ID NO: 104 - DNA, 20 bp, synthetic construct
  source 1..20: mol_type = other DNA
aggacgatactaaccaatgg

SEQ ID NO: 105 - DNA, 20 bp, synthetic construct
  source 1..20: mol_type = other DNA
cttctgttcagaatgtgcac

SEQ ID NO: 106 - DNA, 20 bp, synthetic construct
  source 1..20: mol_type = other DNA
aaggaaaaagaagttgccgc

SEQ ID NO: 107 - DNA, 20 bp, synthetic construct
  source 1..20: mol_type = other DNA
cgattagacaaaagagatcc

SEQ ID NO: 108 - DNA, 20 bp, synthetic construct
  source 1..20: mol_type = other DNA
catgtgattctcctggagaa

SEQ ID NO: 109 - DNA, 20 bp, synthetic construct
  source 1..20: mol_type = other DNA
gaaattcacagaccttgtgg

SEQ ID NO: 110 - DNA, 20 bp, synthetic construct
  source 1..20: mol_type = other DNA
gaaactcgcacaccttgtgg

SEQ ID NO: 111 - DNA, 20 bp, synthetic construct
  source 1..20: mol_type = other DNA
aatcatatgaagttttacgg

SEQ ID NO: 112 - DNA, 20 bp, synthetic construct
  source 1..20: mol_type = other DNA
gagggtcaagtactactcaa

SEQ ID NO: 113 - DNA, 20 bp, synthetic construct
  source 1..20: mol_type = other DNA
gtttggctggacacaacgaa

SEQ ID NO: 114 - DNA, 20 bp, synthetic construct
  source 1..20: mol_type = other DNA
cgacggcttgagactttgca

SEQ ID NO: 115 - DNA, 20 bp, synthetic construct
  source 1..20: mol_type = other DNA
aatcgaaaaggagttgcagg

SEQ ID NO: 116 - DNA, 20 bp, synthetic construct
  source 1..20: mol_type = other DNA
aagggtcaagtacttcaatg

SEQ ID NO: 117 - DNA, 20 bp, synthetic construct
  source 1..20: mol_type = other DNA
cgacggcttgagcctttgca

SEQ ID NO: 118 - DNA, 20 bp, synthetic construct
  source 1..20: mol_type = other DNA
ggacctcacaaactttatgg

SEQ ID NO: 119 - DNA, 20 bp, synthetic construct
  source 1..20: mol_type = other DNA
atggacataacaggcgtcga

SEQ ID NO: 120 - DNA, 20 bp, synthetic construct
  source 1..20: mol_type = other DNA
cgaacagttgaaagcaacag

SEQ ID NO: 121 - DNA, 20 bp, synthetic construct
  source 1..20: mol_type = other DNA
tcatcataggaggtgccgag

SEQ ID NO: 122 - DNA, 20 bp, synthetic construct
  source 1..20: mol_type = other DNA
tagaaattcaccccccatgg

SEQ ID NO: 123 - DNA, 20 bp, synthetic construct
  source 1..20: mol_type = other DNA
tgtgatcagagagcctcctg

SEQ ID NO: 124 - DNA, 20 bp, synthetic construct
  source 1..20: mol_type = other DNA
ggaaaccatccagttcaact

SEQ ID NO: 125 - DNA, 20 bp, synthetic construct
  source 1..20: mol_type = other DNA
ttaaaggggcatcagtccaa

SEQ ID NO: 126 - DNA, 20 bp, synthetic construct
  source 1..20: mol_type = other DNA
atctactttgaaaatgtggg

SEQ ID NO: 127 - DNA, 20 bp, synthetic construct
  source 1..20: mol_type = other DNA
gaaattcacagaccttgtgg

SEQ ID NO: 128 - DNA, 20 bp, synthetic construct
  source 1..20: mol_type = other DNA
cagtcattccaaatgcccaa

SEQ ID NO: 129 - DNA, 20 bp, synthetic construct
  source 1..20: mol_type = other DNA
agatggagtggaatgcaaag

SEQ ID NO: 130 - DNA, 20 bp, synthetic construct
  source 1..20: mol_type = other DNA
ccttcaacttgacacctagg

SEQ ID NO: 131 - DNA, 16 bp, synthetic construct
  source 1..16: mol_type = other DNA
ccatgcaaaggctcaa

SEQ ID NO: 132 - DNA, 25 bp, synthetic construct
  source 1..25: mol_type = other DNA
ccacagcaggaaaccatccagttca

SEQ ID NO: 133 - DNA, 20 bp, synthetic construct
  source 1..20: mol_type = other DNA
gcaggaaaccatccagttca

SEQ ID NO: 134 - DNA, 80 bp, synthetic construct
  source 1..80: mol_type = other DNA
atttagttgcaatttttgtcaaggatatctacctgctaatagcttgccttttagcaattttcgcaggaggctctctgatc

SEQ ID NO: 135 - DNA, 59 bp, synthetic construct
  source 1..59: mol_type = other DNA
gaggctctctgatcacaatgcacgacgccgcaaaccacagcaggaaaccatccagttca

SEQ ID NO: 136 - DNA, 14 bp, synthetic construct
  source 1..14: mol_type = other DNA
agttcaactcggca

SEQ ID NO: 137 - DNA, 10321 bp, synthetic construct
  source 1..10321: mol_type = other DNA
ggagagcgatcagcttgcatgccggtcgatctagtaacatagatgacaccgcgcgcgataatttatcctagtttgcgcgctatattttgttttctatcgcgtattaaatgtataattgcgggactctaatcataaaaacccatctcataaataacgtcatgcattacatgttaattattacatgcttaacgtaattcaacagaaattatatgataatcatggcaagaccggcaacaggattcaatcttaagaaactttattgccaaatgtttgaacgatctgcttgactctagctagagtccgaaccccagagtcccgctcagaagaactcgtcaagaaggcgatagaaggctatgcgctgcgaatcgggagcggcgataccgtaaagcacgaggaagcggtcagcccattcgccgccaagctcttcagcaatatcacgggtagccaacgctatgtcctgatagcggtccgccacacccagccggccacagtcgatgaatccagaaaagcggccattttccaccatgatattcggcaagcaggcgtcgccgtgggtcacgacgagatcctcgccgtcgggcatccgcgccttgagcctggcgaacagttcggctggcgcgagcccctgatgctcttcgtccagatcatcctgatcgacaagaccggcttccatccgagtacgtgctcgctcgatgcggtgtttcgcttggtggtcgaatgggcaggtagccggatcaagcgtatgcagccgccgcattgcatcagccatgatggatactttctcggcaggagcaaggtgagatgacaggagatcctgccccggcacttcgcccaatagcagccagtcccttcccgcttcagtgacaacgtcgagcacagctgcgcaaggaacgcccgtcgtggccagccacgatagccgcgctgcctcgtcttggagttcattcagggcaccggacaggtcggtcttgacaaaaagaaccgggcgcccctgcgctgacagccggaacacggcggcatcagagcagccgattgtctgttgtgcccagtcatagccgaatagcctctccacccaagcggccggagaacctgcgtgcaatccatcttgttcaatcatgcctcgatcgagttgagagtgaatatgagactctaattggataccgaggggaatttatggaacgtcagtggagcatttttgacaagaaatatttgctagctgatagtgaccttaggcgacttttgaacgcgcaataatggtttctgacgtatgtgcttagctcattaaactccagaaacccgcggctgagtggctccttcaacgttgcggttctgtcagttccaaacgtaaaacggcttgtcccgcgtcatcggcgggggtcataacgtgactcccttaattctcatgtatctccgtcaggagactagagccaagctgatctcctttgccccggagatcaccatggacgactttctctatctctacgatctaggaagaaagttcgacggagaaggtgacgataccatgttcaccaccgataatgagaagattagcctcttcaatttcagaaagaatgctgacccacagatggttagagaggcctacgcggcaggtctgatcaagacgatctacccgagtaataatctccaggagatcaaataccttcccaagaaggttaaagatgcagtcaaaagattcaggactaactgcatcaagaacacagagaaagatatatttctcaagatcagaagtactattccagtatggacgattcaaggcttgcttcataaaccaaggcaagtaatagagattggagtctctaagaaagtagttcctactgaatcaaaggccatggagtcaaaaattcagatcgaggatctaacagaactcgccgtgaagactggcgaacagttcatacagagtcttttacgactcaatgacaagaagaaaatcttcgtcaacatggtggagcacgacactctcgtctactccaagaatatcaaagatacagtctcagaagaccaaagggctattgagacttttcaacaaagggtaatatcgggaaacctcctcggattccattgcccagctatctgtcacttcatcaaaaggacagtagaaaaggaaggtggcacctacaaatgccatcattgcgataaaggaaaggctatcgttcaagatgcctctgccgacagtggtcccaaagatggacccccacccacgaggagcatcgtggaaaaagaagacgttccaaccacgtcttcaaagcaagtggattgatgtgatatctccactgacgtaagggatgacgcacaatcccactatccttcgcaagacccttcctctatataaggaagttcatttcatttggagaggactccggtatttttacaacaataccacaacaaaacaaacaacaaacaacattacaatttactattctagtcgaaatggcctcctccgagaacgtcatcaccgagttcatgcgcttcaaggtgcgcatggagggcaccgtgaacggccacgagttcgagatcgagggcgagggcgagggccgcccctacgagggccacaacaccgtgaagctgaaggtgaccaagggcggccccctgcccttcgcctgggacatcctgtccccccagttccagtacggctccaaggtgtacgtgaagcaccccgccgacatccccgactacaagaagctgtccttccccgagggcttcaagtgggagcgcgtgatgaacttcgaggacggcggcgtggcgaccgtgacccaggactcctccctgcaggacggctgcttcatctacaaggtgaagttcatcggcgtgaacttcccctccgacggccccgtgatgcagaagaagacgatgggctgggaggcctccaccgagcgcctgtacccccgcgacggcgtgctgaagggcgagacacacaaggccctgaagctgaaggacggcggccactacctggtggagttcaagtccatctacatggccaagaagcccgtgcagctgcccggctactactacgtggacgccaagctggacatcacctcccacaacgaggactacaccatcgtggagcagtacgagcgcaccgagggccgccaccacctgttcctgtaggcttggaatggatcttcgatcccgatcgttcaaacatttggcaataaagtttcttaagattgaatcctgttgccggtcttgcgacgattatcatataatttctgttgaattacgttaagcatgtaataattaacatgtaatgcatgacgttatttatgagatgggtttttatgattagagtcccgcaattatacatttaatacgcgatagaaaacaaaatatagcgcgcaaactaggataaattatcgcgcdcggtgtcatctatgttactagatcgggaattgccaagctaattcttgaagacgaaagggcctcgtgatacgcctatttttataggttaatgtcatgataataatggtttcttagacgtcaggtggcacttttcggggaaatgtgcgcggaacccctatttgtttatttttctaaatacattcaaatatgtatccgctcatgagacaataaccctgataaatgcttcaataatgggaccgactcgcgctgtcatgagaccggatcctgacaggatatattggcgggtaaacctaagagaaaagagcgtttattagaataatcggatatttaaaagggcgtgaaaaggtttatccgttcgtccatttgtatgtgcatgccaaccacagggttcccctcgggatcaaagtactttgatccaacccctccgctgctatagtgcagtcggcttctgacgttcagtgcagccgtcatctgaaaacgacatgtcgcacaagtcctaagttacgcgacaggctgccgccctgcccttttcctggcgttttcttgtcgcgtgttttagtcgcataaagtagaatacttgcgactagaaccggagacattacgccatgaacaagagcgccgccgctggcctgctgggctatgcccgcgtcagcaccgacgaccaggacttgaccaaccaacgggccgaactgcacgcggccggctgcaccaagctgttttccgagaagatcaccggcaccaggcgcgaccgcccggagctggccaggatgcttgaccacctacgccctggcgacgttgtgacagtgaccaggctagaccgcctggcccgcagcacccgcgacctactggacattgccgagcgcatccaggaggccggcgcgggcctgcgtagcctggcagagccgtgggccgacaccaccacgccggccggccgcatggtgttgaccgtgttcgccggcattgccgagttcgagcgttccctaatcatcgaccgcacccggagcgggcgcgaggccgccaaggcccgaggcgtgaagtttggcccccgccctaccctcaccccggcacagatcgcgcacgcccgcgagctgatcgaccaggaaggccgcaccgtgaaagaggcggctgcactgcttggcgtgcatcgctcgaccctgtaccgcgcacttgagcgcagcgaggaagtgacgcccaccgaggccaggcggcgcggtgccttccgtgaggacgcattgaccgaggccgacgccctggcggccgccgagaatgaacgccaagaggaacaagcatgaaaccgcaccaggacggccaggacgaaccgtttttcattaccgaagagatcgaggcggagatgatcgcggccgggtacgtgttcgagccgcccgcgcacctctcaaccgtgcggctgcatgaaatcctggccggtttgtctgatgccaagctggcggcctggccggccagcttggccgctgaagaaaccgagcgccgccgtctaaaaaggtgatgtgtatttgagtaaaacagcttgcgtcatgcggtcgctgcgtatatgatccgatgagtaaataaacaaatacgcaaggggaacgcatgaaggttatcgctgtacttaaccagaaaggcgggtcaggcaagacgaccatcggaacccatctagcccgcgccctgcaactcgccggggccgatgttctgttagtcgattccgatccccagggcagtgcccgcgattgggcggccgtgcgggaagatcaaccgctaaccgttgtcggcatcgaccgcccgacgattgaccgcgacgtgaaggccatcggccggcgcgacttcgtagtgatcgacggagcgccccaggcggcggacttggctgtgtccgcgatcaaggcagccgacttcgtgctgattccggtgcagccaagcccttacgacatatgggccaccgccgacctggtggagctggttaagcagcgcattgaggtcacggatggaaggctacaagcggcctttgtcgtgtcgcgggcgatcaaaggcacgcgcatcggcggtgaggttgccgaggcgctggccgggtacgagctgcccattcttgagtcccgtatcacgcagcgcgtgagctacccaggcactgccgccgccggcacaaccgttcttgaatcagaacccgagggcgacgctgcccgcgaggtccaggcgctggccgctgaaattaaatcaaaactcatttgagttaatgaggtaaagagaaaatgagcaaaagcacaaacacgctaagtgccggccgtccgagcgcacgcagcagcaaggctgcaacgttggccagcctggcagacacgccagccatgaagcgggtcaactttcagttgccggcggaggatcacaccaagctgaagatgtacgcggtacgccaaggcaagaccattaccgagctgctatctgaatagatcgcgcagctaccagagtaaatgagcaaatgaataaatgagtagatgaattttagcggctaaaggaggcggcatggaaaatcaagaacaaccaggcaccgacgccgtggaatgccccatgtgtggaggaacgggcggttggccaggcgtaagcggctgggttgtctgccggccctgcaatggcactggaacccccaagcccgaggaatcggcgtgacggtcgcaaaccatccggcccggtacaaatcggcgcggcgctgggtgatgacctggtggagaagttgaaggccgcgcaggccgcccagcggcaacgcatcgaggcagaagcacgccccggtgaatcgtggcaagcggccgctgatcgaatccgcaaagaatcccggcaaccgccggcagccggtgcgccgtcgattaggaagccgcccaagggcgacgagcaaccagattttttcgttccgatgctctatgacgtgggcacccgcgatagtcgcagcatcatggacgtggccgttttccgtctgtcgaagcgtgaccgacgagctggcgaggtgatccgctacgagcttccagacgggcacgtagaggtttccgcagggccggccggcatggccagtgtgtgggattacgacctggtactgatggcggtttcccatctaaccgaatccatgaaccgataccgggaagggaagggagacaagcccggccgcgtgttccgtccacacgttgcggacgtactcaagttctgccggcgagccgatggcggaaagcagaaagacgacctggtagaaacctgcattcggttaaacaccacgcacgttgccatgcagcgtacgaagaaggccaagaacggccgcctggtgacggtatccgagggtgaagccttgattagccgctacaagatcgtaaagagcgaaaccgggcggccggagtacatcgagatcgagctagctgattggatgtaccgcgagatcacagaaggcaagaacccggacgtgctgacggttcaccccgattactttttgatcgatcccggcatcggccgttttctctaccgcctggcacgccgcgccgcaggcaaggcagaagccagatggttgttcaagacgatctacgaacgcagtggcagcgccggagagttcaagaagttctgtttcaccgtgcgcaagctgatcgggtcaaatgacctgccggagtacgatttgaaggaggaggcggggcaggctggcccgatcctagtcatgcgctaccgcaacctgatcgagggcgaagcatccgccggttcctaatgtacggagcagatgctagggcaaattgccctagcaggggaaaaaggtcgaaaaggactctttcctgtggatagcacgtacattgggaacccaaagccgtacattgggaaccggaacccgtacattgggaacccaaagccgtacattgggaaccggtcacacatgtaagtgactgatataaaagagaaaaaaggcgatttttccgcctaaaactctttaaaacttattaaaactcttaaaacccgcctggcctgtgcataactgtctggccagcgcacagccgaagagctgcaaaaagcgcctacccttcggtcgctgcgctccctacgccccgccgcttcgcgtcggcctatcgcggccgctggccgctcaaaaatggctggcctacggccaggcaatctaccagggcgcggacaagccgcgccgtcgccactcgaccgccggcgcccacatcaaggcaccctgcctcgcgcgtttcggtgatgacggtgaaaacctctgacacatgcagctcccggtgacggtcacagcttgtctgtaagcggatgccgggagcagacaagcccgtcagggcgcgtcagcgggtgttggcgggtgtcggggcgcagccatgacccagtcacgtagcgatagcggagtgtatactggcttaactatgcggcatcagagcagattgtactgagagtgcaccatatgcggtgtgaaataccgcacagatgcgtaaggagaaaataccgcatcaggcgctcttccgcttcctcgctcactgactcgctgcgctcggtcgttcggctgcggcgagcggtatcagctcactcaaaggcggtaatacggttatccacagaatcaggggataacgcaggaaagaacatgtgagcaaaaggccagcaaaaggccaggaaccgtaaaaaggccgcgttgctggcgtttttccataggctccgcccccctgacgagcatcacaaaaatcgacgctcaagtcagaggtggcgaaacccgacaggactataaagataccaggcgtttccccctggaagctccctcgtgcgctctcctgttccgaccctgccgcttaccggatacctgtccgcctttctcccttcgggaagcgtggcgctttctcatagctcacgctgtaggtatctcagttcggtgtaggtcgttcgctccaagctgggctgtgtgcacgaaccccccgttcagcccgaccgctgcgccttatccggtaactatcgtcttgagtccaacccggtaagacacgacttatcgccactggcagcagccactggtaacaggattagcagagcgaggtatgtaggcggtgctacagagttcttgaagtggtggcctaactacggctacactagaaggacagtatttggtatctgcgctctgctgaagccagttaccttcggaaaaagagttggtagctcttgatccggcaaacaaaccaccgctggtagcggtggtttttttgtttgcaagcagcagattacgcgcagaaaaaaaggatctcaagaagatcctttgatcttttctacggggtctgacgctcagtggaacgaaaactcacgttaagggattttggtcatgcattctaggtgattatttgccgactaccttggtgatctcgcctttcacgtagtggacaaattcttccaactgatctgcgcgcgaggccaagcgatcttcttcttgtccaagataagcctgtctagcttcaagtatgacgggctgatactgggccggcaggcgctccattgcccagtcggcagcgacatccttcggcgcgattttgccggttactgcgctgtaccaaatgcgggacaacgtaagcactacatttcgctcatcaccagcccagtcgggcggcgagttccatagcgttaaggtttcatttagcgcctcaaatagatcctgttcaggaaccggatcaaagagttcctccgccgctggacctaccaaggcaacgctatgttctcttgcttttgtcagcaagatagccagatcaatgtcgatcgtggctggctcgaagatacctgcaagaatgtcattgcgctgccattctccaaattgcagttcgcgcttagctggataacgccacggaatgatgtcgtcgtgcacaacaatggtgacttctacagcgcggagaatctcgctctctccaggggaagccgaagtttccaaaaggtcgttgatcaaagctcgccgcgttgtttcatcaagccttacggtcaccgtaaccagcaaatcaatatcactgtgtggcttcaggccgccatccactgcggagccgtacaaatgtacggccagcaacgtcggttcgagatggcgctcgatgacgccaactacctctgatagttgagtcgatacttcggcgatcaccgcttccctcataatgtttaactttgttttagggcgactgccctgctgcgtaacatcgttgctgctccataacatcaaacatcgacccacggcgtaacgcgcttgctgcttggatgcccgaggcatagactgtaccccaaaaaaacagtcataacaagccatgaaaaccgccactgcgccgttaccaccgctgcgttcggtcaaggttctggaccagttgcgtgagcgcatacgctacttgcattacagcttacgaaccgaacaggcttatgtccactgggttcgtgccttcatccgtttccacggtgtgcgtcacccggcaaccttgggtagcagcgaagtcgaggcatttctgtcctggctggaacagaacttattatttccttcctcttttctacagtatttaaagataccccaagaagctaattataacaagacgaactccaattcactgttccttgcattctaaaaccttaaataccagaaaacagctttttcaaagttgttttcaaagttggcgtataacatagtatcgacggagccgattttgaaaccgcggtgatcacaggcagcaacgctctgtcatcgttacaatcaacatgctaccctccgcgagatcatccgtgtttcaaacccggcagcttagttgccgttcttccgaatagcatcggtaacatgagcaaagtctgccgccttacaacggctctcccgctgacgccgtcccggactgatgggctgcctgtatcgagtggtgattttgtgccgagctgccggtcggggagctgttggctggctggtggcaggatatattgtggtgtaaacataacggatccggtctca

SEQ ID NO: 138 - DNA, 8254 bp, synthetic construct
  source 1..8254: mol_type = other DNA
ggagatacatgagaattaagggagtcacggtatgacccccgccgatgacgcgggacaagccgttttacgtttggaactgacagaaccgcaacgttgaaggagccactgagccgcgggtttctggagtttaatgagctaagcacatacgtcagaaaccattattgcgcgttcaaaagtcgcctaaggtcactatcagctagcaaatatttcttgtcaaaaatgctccactgacgttccataaattcccctcggtatccaattagagtctcatattcactctcaactcgatcgaggcaatgccttctgctagtaagaacttcagactccaatctaaatatgttttccttacctatcccaagtgctcatctcaaagagatgatttattccagtttctctgggagaaactcacaccttttcttattttcttccttggtgttgcttctgagcttcatcaagatggcactacccactatcatgctcttctccagcttgataaaaaaccttgtattagggatccttcttttttcgattttgaaggaaatcaccctaatatccagccagctagaaactctaaacaagtccttgattacatatcaaaggacggagatattaaaaccagaggagatttccgagatcataaggtttctcctcgcaaatctgacgcacgatggagaactattatccagactgcaacgtctaaggaggaatatcttgacatgatcaaggaagaattccctcatgaatgggcaacaaagcttcaatggctggaatattcagccaacaaattattccctccacaacctgaaccgtatgtgtcgcccttcacagaatcagatcttcgctgccacgaagatctacactcctggagggaaacccatctataccatgtaagcatagacgcttatacttacatacatcctgtctcataccaacaagctcaatctgaccttgaatggatggccgatttaaccaggacaatggaaggaatggaatccgacaccccagcctctacatctgcggaccaactcgtaccggaaagaccacctgggctagaagtctcggacgacacaactattggaacggtaccatcgatttcaccaactacgatgaacacgccacctataatatcatcgacgacatccccttcaagttcgtcccattgtggaagcaattaataggttgccagtctgatttcactgtcaaccctaaatatggaaaaaagaagaaaataaaaggtgggatcccttctataattctttgcaatcctgacgaagactggatgttatcaatgacaagtcaacagaaggattactttaaagataattgcgtcacccactacatgtgtgacggggagactttttttgctcgggaatcgtcgagtcactgagcttggaatggatcttcgatcccgatcgttcaaacatttggcaataaagtttcttaagattgaatcctgttgccggtcttgcgacgattatcatataatttctgttgaattacgttaagcatgtaataattaacatgtaatgcatgacgttatttatgagatgggtttttatgattagagtcccgcaattatacatttaatacgcgatagaaaacaaaatatagcgcgcaaactaggataaattatcgcgcdcggtgtcatctatgttactagatcgggaattgccaagctaattcttgaagacgaaagggcctcgtgatacgcctatttttataggttaatgtcatgataataatggtttcttagacgtcaggtggcacttttcggggaaatgtgcgcggaacccctatttgtttatttttctaaatacattcaaatatgtatccgctcatgagacaataaccctgataaatgcttcaataatgggaccgactcgcgctgtcatgagacgaattctgacaggatatattggcgggtaaacctaagagaaaagagcgtttattagaataatcggatatttaaaagggcgtgaaaaggtttatccgttcgtccatttgtatgtgcatgccaaccacagggttcccctcgggatcaaagtactttgatccaacccctccgctgctatagtgcagtcggcttctgacgttcagtgcagccgtcatctgaaaacgacatgtcgcacaagtcctaagttacgcgacaggctgccgccctgcccttttcctggcgttttcttgtcgcgtgttttagtcgcataaagtagaatacttgcgactagaaccggagacattacgccatgaacaagagcgccgccgctggcctgctgggctatgcccgcgtcagcaccgacgaccaggacttgaccaaccaacgggccgaactgcacgcggccggctgcaccaagctgttttccgagaagatcaccggcaccaggcgcgaccgcccggagctggccaggatgcttgaccacctacgccctggcgacgttgtgacagtgaccaggctagaccgcctggcccgcagcacccgcgacctactggacattgccgagcgcatccaggaggccggcgcgggcctgcgtagcctggcagagccgtgggccgacaccaccacgccggccggccgcatggtgttgaccgtgttcgccggcattgccgagttcgagcgttccctaatcatcgaccgcacccggagcgggcgcgaggccgccaaggcccgaggcgtgaagtttggcccccgccctaccctcaccccggcacagatcgcgcacgcccgcgagctgatcgaccaggaaggccgcaccgtgaaagaggcggctgcactgcttggcgtgcatcgctcgaccctgtaccgcgcacttgagcgcagcgaggaagtgacgcccaccgaggccaggcggcgcggtgccttccgtgaggacgcattgaccgaggccgacgccctggcggccgccgagaatgaacgccaagaggaacaagcatgaaaccgcaccaggacggccaggacgaaccgtttttcattaccgaagagatcgaggcggagatgatcgcggccgggtacgtgttcgagccgcccgcgcacctctcaaccgtgcggctgcatgaaatcctggccggtttgtctgatgccaagctggcggcctggccggccagcttggccgctgaagaaaccgagcgccgccgtctaaaaaggtgatgtgtatttgagtaaaacagcttgcgtcatgcggtcgctgcgtatatgatccgatgagtaaataaacaaatacgcaaggggaacgcatgaaggttatcgctgtacttaaccagaaaggcgggtcaggcaagacgaccatcggaacccatctagcccgcgccctgcaactcgccggggccgatgttctgttagtcgattccgatccccagggcagtgcccgcgattgggcggccgtgcgggaagatcaaccgctaaccgttgtcggcatcgaccgcccgacgattgaccgcgacgtgaaggccatcggccggcgcgacttcgtagtgatcgacggagcgccccaggcggcggacttggctgtgtccgcgatcaaggcagccgacttcgtgctgattccggtgcagccaagcccttacgacatatgggccaccgccgacctggtggagctggttaagcagcgcattgaggtcacggatggaaggctacaagcggcctttgtcgtgtcgcgggcgatcaaaggcacgcgcatcggcggtgaggttgccgaggcgctggccgggtacgagctgcccattcttgagtcccgtatcacgcagcgcgtgagctacccaggcactgccgccgccggcacaaccgttcttgaatcagaacccgagggcgacgctgcccgcgaggtccaggcgctggccgctgaaattaaatcaaaactcatttgagttaatgaggtaaagagaaaatgagcaaaagcacaaacacgctaagtgccggccgtccgagcgcacgcagcagcaaggctgcaacgttggccagcctggcagacacgccagccatgaagcgggtcaactttcagttgccggcggaggatcacaccaagctgaagatgtacgcggtacgccaaggcaagaccattaccgagctgctatctgaatagatcgcgcagctaccagagtaaatgagcaaatgaataaatgagtagatgaattttagcggctaaaggaggcggcatggaaaatcaagaacaaccaggcaccgacgccgtggaatgccccatgtgtggaggaacgggcggttggccaggcgtaagcggctgggttgtctgccggccctgcaatggcactggaacccccaagcccgaggaatcggcgtgacggtcgcaaaccatccggcccggtacaaatcggcgcggcgctgggtgatgacctggtggagaagttgaaggccgcgcaggccgcccagcggcaacgcatcgaggcagaagcacgccccggtgaatcgtggcaagcggccgctgatcgaatccgcaaagaatcccggcaaccgccggcagccggtgcgccgtcgattaggaagccgcccaagggcgacgagcaaccagattttttcgttccgatgctctatgacgtgggcacccgcgatagtcgcagcatcatggacgtggccgttttccgtctgtcgaagcgtgaccgacgagctggcgaggtgatccgctacgagcttccagacgggcacgtagaggtttccgcagggccggccggcatggccagtgtgtgggattacgacctggtactgatggcggtttcccatctaaccgaatccatgaaccgataccgggaagggaagggagacaagcccggccgcgtgttccgtccacacgttgcggacgtactcaagttctgccggcgagccgatggcggaaagcagaaagacgacctggtagaaacctgcattcggttaaacaccacgcacgttgccatgcagcgtacgaagaaggccaagaacggccgcctggtgacggtatccgagggtgaagccttgattagccgctacaagatcgtaaagagcgaaaccgggcggccggagtacatcgagatcgagctagctgattggatgtaccgcgagatcacagaaggcaagaacccggacgtgctgacggttcaccccgattactttttgatcgatcccggcatcggccgttttctctaccgcctggcacgccgcgccgcaggcaaggcagaagccagatggttgttcaagacgatctacgaacgcagtggcagcgccggagagttcaagaagttctgtttcaccgtgcgcaagctgatcgggtcaaatgacctgccggagtacgatttgaaggaggaggcggggcaggctggcccgatcctagtcatgcgctaccgcaacctgatcgagggcgaagcatccgccggttcctaatgtacggagcagatgctagggcaaattgccctagcaggggaaaaaggtcgaaaaggactctttcctgtggatagcacgtacattgggaacccaaagccgtacattgggaaccggaacccgtacattgggaacccaaagccgtacattgggaaccggtcacacatgtaagtgactgatataaaagagaaaaaaggcgatttttccgcctaaaactctttaaaacttattaaaactcttaaaacccgcctggcctgtgcataactgtctggccagcgcacagccgaagagctgcaaaaagcgcctacccttcggtcgctgcgctccctacgccccgccgcttcgcgtcggcctatcgcggccgctggccgctcaaaaatggctggcctacggccaggcaatctaccagggcgcggacaagccgcgccgtcgccactcgaccgccggcgcccacatcaaggcaccctgcctcgcgcgtttcggtgatgacggtgaaaacctctgacacatgcagctcccggtgacggtcacagcttgtctgtaagcggatgccgggagcagacaagcccgtcagggcgcgtcagcgggtgttggcgggtgtcggggcgcagccatgacccagtcacgtagcgatagcggagtgtatactggcttaactatgcggcatcagagcagattgtactgagagtgcaccatatgcggtgtgaaataccgcacagatgcgtaaggagaaaataccgcatcaggcgctcttccgcttcctcgctcactgactcgctgcgctcggtcgttcggctgcggcgagcggtatcagctcactcaaaggcggtaatacggttatccacagaatcaggggataacgcaggaaagaacatgtgagcaaaaggccagcaaaaggccaggaaccgtaaaaaggccgcgttgctggcgtttttccataggctccgcccccctgacgagcatcacaaaaatcgacgctcaagtcagaggtggcgaaacccgacaggactataaagataccaggcgtttccccctggaagctccctcgtgcgctctcctgttccgaccctgccgcttaccggatacctgtccgcctttctcccttcgggaagcgtggcgctttctcatagctcacgctgtaggtatctcagttcggtgtaggtcgttcgctccaagctgggctgtgtgcacgaaccccccgttcagcccgaccgctgcgccttatccggtaactatcgtcttgagtccaacccggtaagacacgacttatcgccactggcagcagccactggtaacaggattagcagagcgaggtatgtaggcggtgctacagagttcttgaagtggtggcctaactacggctacactagaaggacagtatttggtatctgcgctctgctgaagccagttaccttcggaaaaagagttggtagctcttgatccggcaaacaaaccaccgctggtagcggtggtttttttgtttgcaagcagcagattacgcgcagaaaaaaaggatctcaagaagatcctttgatcttttctacggggtctgacgctcagtggaacgaaaactcacgttaagggattttggtcatgcattctaggtgattagaaaaactcatcgagcatcaaatgaaactgcaatttattcatatcaggattatcaataccatatttttgaaaaagccgtttctgtaatgaaggagaaaactcaccgaggcagttccataggatggcaagatcctggtatcggtctgcgattccgactcgtccaacatcaatacaacctattaatttcccctcgtcaaaaataaggttatcaagtgagaaatcaccatgagtgacgactgaatccggtgagaatggcaaaagtttatgcatttctttccagacttgttcaacaggccagccattacgctcgtcatcaaaatcactcgcatcaaccaaaccgttattcattcgtgattgcgcctgagcgagtcgaaatacgcgatcgctgttaaaaggacaattacaaacaggaatcgaatgcaaccggcgcaggaacactgccagcgcatcaacaatattttcacctgaatcaggatattcttctaatacctggaatgctgttttccctgggatcgcagtggtgagtaaccatgcatcatcaggagtacggataaaatgcttgatggtcggaagaggcataaattccgtcagccagtttagtctgaccatctcatctgtaacatcattggcaacgctacctttgccatgtttcagaaacaactctggcgcatcgggcttcccatacaatcggtagattgtcgcacctgattgcccgacattatcgcgagcccatttatacccatataaatcagcatccatgttggaatttaatcgcggccttgagcaagacgtttcccgttgaatatggctcataacagaacttattatttccttcctcttttctacagtatttaaagataccccaagaagctaattataacaagacgaactccaattcactgttccttgcattctaaaaccttaaataccagaaaacagctttttcaaagttgttttcaaagttggcgtataacatagtatcgacggagccgattttgaaaccgcggtgatcacaggcagcaacgctctgtcatcgttacaatcaacatgctaccctccgcgagatcatccgtgtttcaaacccggcagcttagttgccgttcttccgaatagcatcggtaacatgagcaaagtctgccgccttacaacggctctcccgctgacgccgtcccggactgatgggctgcctgtatcgagtggtgattttgtgccgagctgccggtcggggagctgttggctggctggtggcaggatatattgtggtgtaaacataacgaattcgtctca

SEQ ID NO: 139 - DNA, 13311 bp, synthetic construct
  source 1..13311: mol_type = other DNA
gcggccgcgattccattgcccagctatctgtcactttattgtgaagatagtggaaaaggaaggtggctcctacaaatgccatcattgcgataaaggaaaggccatcgttgaagatgcctctgccgacagtggtcccaaagatggacccccacccacgaggagcatcgtggaaaaagaagacgttccaaccacgtcttcaaagcaagtggattgatgtgatatctccactgacgtaagggatgacgcacaatcccactatccttcgcaagacccttcctctatataaggaagttcatttcatttggagaggaaaataacaaatctcaacacaacatatacaaaacaaacgaatctcaagcaatcaagcattctacttctattgcagcaatttaaatcatttcttttaaagcaaaagcaattttctgaaaattttcaccatttacgaacgatagccatggcactcatctttggcacagtcaacgctaacatcctgaaggaagtgttcggtggagctcgtatggcttgcgttaccagcgcacatatggctggagcgaatggaagcattttgaagaaggcagaagaaacctctcgtgcaatcatgcacaaaccagtgatcttcggagaagactacattaccgaggcagacttgccttacacaccactccatttagaggtcgatgctgaaatggagcggatgtattatcttggtcgtcgcgcgctcacccatggcaagagacgcaaagtttctgtgaataacaagaggaacaggagaaggaaagtggccaaaacgtacgtggggcgtgattccattgttgagaagattgtagtgccccacaccgagagaaaggttgataccacagcagcagtggaagacatttgcaatgaagctaccactcaacttgtgcataatagtatgccaaagcgtaagaagcagaaaaacttcttgcccgccacttcactaagtaacgtgtatgcccaaacttggagcatagtgcgcaaacgccatatgcaggtggagatcattagcaagaagagcgtccgagcgagggtcaagagatttgagggctcggtgcaattgttcgcaagtgtgcgtcacatgtatggcgagaggaaaagggtggacttacgtattgacaactggcagcaagagacacttctagaccttgctaaaagatttaagaatgagagagtggatcaatcgaagctcacttttggttcaagtggcctagttttgaggcaaggctcgtacggacctgcgcattggtatcgacatggtatgttcattgtacgcggtcggtcggatgggatgttggtggatgctcgtgcgaaggtaacgttcgctgtttgtcactcaatgacacattatagcgacaaatcaatctctgaggcattcttcataccatactctaagaaattcttggagttgaggccagatggaatctcccatgagtgtacaagaggagtatcagttgagcggtgcggtgaggtggctgcaatcctgacacaagcactttcaccgtgtggtaagatcacatgcaaacgttgcatggttgaaacacctgacattgttgagggtgagtcgggagacagtgtcaccaaccaaggtaagctcctagcaatgctgaaagaacagtatccagatttcccaatggccgagaaactactcacaaggtttttgcaacagaaatcactagtaaatacaaatttgacagcctgcgtgagcgtcaaacaactcattggtgaccgcaaacaagctccattcacacacgtactggctgtcagcgaaattctgtttaaaggcaataaactaacaggggccgatctcgaagaggcaagcacacatatgcttgaaatagcaaggttcttgaacaatcgcactgaaaatatgcgcattggccaccttggttctttcagaaataaaatctcatcgaaggcccatgtgaataacgcactcatgtgtgataatcaacttgatcagaatgggaattttatttggggactaaggggtgcacacgcaaagaggtttcttaaaggatttttcactgagattgacccaaatgaaggatacgataagtatgttatcaggaaacatatcaggggtagcagaaagctagcaattggcaatttgataatgtcaactgacttccagacgctcaggcaacaaattcaaggcgaaactattgagcgtaaagaaattgggaatcactgcatttcaatgcggaatggtaattacgtgtacccatgttgttgtgttactcttgaagatggtaaggctcaatattcggatctaaagcatccaacgaagagacatctggtcattggcaactctggcgattcaaagtacctagaccttccagttctcaatgaagagaaaatgtatatagctaatgaaggttattgctacatgaacattttctttgctctactagtgaatgtcaaggaagaggatgcaaaggacttcaccaagtttataagggacacaattgttccaaagcttggagcgtggccaacaatgcaagatgttgcaactgcatgctacttactttccattctttacccagatgtcctgagtgctgaattacccagaattttggttgatcatgacaacaaaacaatgcatgttttggattcgtatgggtctagaacgacaggataccacatgttgaaaatgaacacaacatcccagctaattgaattcgttcattcaggtttggaatccgaaatgaaaacttacaatgttggagggatgaaccgagatatggtcacacaaggtgcaattgagatgttgatcaagtccatatacaaaccacatctcatgaagcagttacttgaggaggagccatacataattgtcctggcaatagtctccccttcaattttaattgccatgtacaactctggaacttttgagcaggcgttacaaatgtggttgccaaatacaatgaggttagctaacctcgctgccatcttgtcagccttggcgcaaaagttaactttggcagacttgttcgtccagcagcgtaatttgattaatgagtatgcgcaggtaattttggacaatctgattgacggtgtcagggttaaccattcgctatccctagcaatggaaattgttactattaagctggccacccaagagatggacatggcgttgagggaaggtggctatgctgtgacctctgaaaaggtgcatgaaatgttggaaaaaaactatgtaaaggctttgaaggatgcatgggacgaattaacttggttggaaaaattctccgcaatcaggcattcaagaaagctcttgaaatttgggcgaaagcctttaatcatgaaaaacaccgtagattgcggcggacatatagacttgtctgtgaaatcgcttttcaagttccacttggaactcctgaagggaaccatctcaagagccgtaaatggtggtgcaagaaaggtaagagtagcgaagaatgccatgacaaaaggggtttttctcaaaatctacagcatgcttcctgacgtctacaagtttatcacagtctcgagtgtcctttccttgttgttgacattcttatttcaaattgactgcatgataagggcacaccgagaggcgaaggttgctgcacagttgcagaaagagagcgagtgggacaatatcatcaatagaactttccagtattctaagcttgaaaatcctattggctatcgctctacagcggaggaaagactccaatcagaacaccccgaggctttcgagtactacaagttttgcattggaaaggaagacctcgttgaacaggcaaaacaaccggagatagcatactttgaaaagattatagctttcatcacacttgtattaatggcttttgacgctgagcggagtgatggagtgttcaagatactcaataagttcaaaggaatactgagctcaacggagagggagatcatctacacgcagagtttggatgattacgttacaacctttgatgacaatatgacaatcaacctcgagttgaatatggatgaactccacaagacgagccttcctggagtcacttttaagcaatggtggaacaaccaaatcagccgaggcaacgtgaagccacattatagaactgaggggcacttcatggagtttaccagagatactgcggcatcggttgccagcgagatatcacactcacccgcaagagattttcttgtgagaggtgctgttggatctggaaaatccacaggacttccataccatttatcaaagagagggagagtgttaatgcttgagcctaccagaccactcacagataacgtgcacaagcaactgagaagtgaaccatttaactgcttcccaactttgaggatgagagggaagtcaacttttgggtcatcaccgattacagtcatgactagtggattcgctttacaccattttgcacgaaacatagctgaggtaaaaacatacgattttgtcataattgatgaatgtcatgtgaatgatgcttctgctatagcgtttaggaatctactgtttgaacatgaatttgaaggaaaagtcctcaaagtgtcagccacaccaccaggtagagaagttgaattcacaactcagtttcccgtgaaactcaagatagaagaggctcttagctttcaggaatttgtaagtttacaagggacaggtgccaacgccgatgtgattagttgtggcgacaacatactagtatatgttgctagctacaatgatgttgatagtcttggcaagctccttgtgcaaaagggatacaaagtgtcgaagattgatggaagaacaatgaagagtggaggaactgaaataatcactgaaggtacttcagtgaaaaagcatttcatagtcgcaactaatattattgagaatggtgtaaccattgacattgatgtagttgtggattttgggactaaggttgtaccagttttggatgtggacaatagagcggtgcagtacaacaaaactgtggtgagttatggggagcgcatccaaagactcggtagagttgggcgacacaaggaaggagtagcacttcgaattggccaaacaaataaaacactggttgaaattccagaaatggttgccactgaagctgcctttctatgcttcatgtacaatttgccagtgacaacacagagtgtttcaaccacactgctggaaaatgccacattattacaagctagaactatggcacagtttgagctatcatatttttacacaattaattttgtgcgatttgatggtagtatgcatccagtcatacatgacaagctgaagcgctttaagctacacacttgtgagacattcctcaataagttggcgatcccaaataaaggcttatcctcttggcttacgagtggagagtataagcgacttggttacatagcagaggatgctggcataagaatcccattcgtgtgcaaagaaattccagactccttgcatgaggaaatttggcacattgtagtcgcccataaaggtgactcgggtattgggaggctcactagcgtacaggcagcaaaggttgtttatactctgcaaacggatgtgcactcaattgcgaggactctagcatgcatcaatagactcatagcacatgaacaaatgaagcagagtcattttgaagccgcaactgggagagcattttccttcacaaattactcaatacaaagcatatttgacacgctgaaagcaaattatgctacaaagcatacgaaagaaaatattgcagtgcttcagcaggcaaaagatcaattgctagagttttcgaacctagcaaaggatcaagatgtcacgggtatcatccaagacttcaatcacctggaaactatctatctccaatcagatagcgaagtggctaagcatctgaagcttaaaagtcactggaataaaagccaaatcactagggacatcataatagctttgtctgtgttaattggtggtggatggatgcttgcaacgtacttcaaggacaagttcaatgaaccagtctatttccaagggaagaagaatcagaagcacaagcttaagatgagagaggcgcgtggggctagagggcaatatgaggttgcagcggagccagaggcgctagaacattactttggaagcgcatataataacaaaggaaagcgcaagggcaccacgagaggaatgggtgcaaagtctcggaaattcataaacatgtatgggtttgatccaactgatttttcatacattaggtttgtggatccattgacaggtcacactattgatgagtccacaaacgcacctattgatttagtgcagcatgagtttggaaaggttagaacacgcatgttaattgacgatgagatagagcctcaaagtcttagcacccacaccacaatccatgcttatttggtgaatagtggcacgaagaaagttcttaaggttgatttaacaccacactcgtcgctacgtgcgagtgagaaatcaacagcaataatgggatttcctgaaagggagaatgaattgcgtcaaaccggcatggcagtgccagtggcttatgatcaattgccaccaaagagtgaggacttgacgtttgaaggagaaagcttgtttaagggaccacgtgattacaacccgatatcgagcaccatttgtcacttgacgaatgaatctgatgggcacacaacatcgttgtatggtattggatttggtcccttcatcattacaaacaagcacttgtttagaagaaataatggaacactgttggtccaatcactacatggtgtattcaaggtcaagaacaccacgactttgcaacaacacctcattgatgggagggacatgataattattcgcatgcctaaggatttcccaccatttcctcaaaagctgaaatttagagagccacaaagggaagagcgcatatgtcttgtgacaaccaacttccaaactaagagcatgtctagcatggtgtcagacactagttgcacattcccttcatctgatggcatattctggaagcattggattcaaaccaaggatgggcagtgtggcagtccattagtatcaactagagatgggttcattgttggtatacactcagcatcgaatttcaccaacacaaacaattatttcacaagcgtgccgaaaaacttcatggaattgttgacaaatcaggaggcgcagcagtgggttagtggttggcgattaaatgctgactcagtattgtgggggggccataaagttttcatgagcaaacctgaagagccttttcagccagttaaggaagcgactcaactcatgagtgaattggtgtactcgcaaggggagaagaggaaatgggtcgtggaagcactgtcagggaacttgaggccagtggctgagtgtcccagtcagttagtcacaaagcatgtggttaaaggaaagtgtcccctctttgagctctacttgcagttgaatccagaaaaggaagcatattttaaaccgatgatgggagcatataagccaagtcgacttaatagagaggcgttcctcaaggacattctaaaatatgctagtgaaattgagattgggaatgtggattgtgacttgctggagcttgcaataagcatgctcatcacaaagctcaaggcgttaggattcccaactgtgaactacatcactgacccagaggaaatttttagtgcattgaatatgaaagcagctatgggagcactatacaaaggcaagaagaaagaagctctcagcgagctcacactagatgagcaggaggcaatgctcaaagcaagttgcctgcgactgtatacgggaaagctgggaatttggaatggctcattgaaagcagagttgcgtccaattgagaaggttgaaaacaacaaaacgcgaactttcacagcagcaccaatagacactcttcttgctggtaaagtttgcgtggatgatttcaacaatcaattttatgatctcaacataaaggcaccatggacagttggtatgactaagttttatcaggggtggaatgaattgatggaggctttaccaagtgggtgggtgtattgtgacgctgatggttcgcaattcgacagttccttgactccattcctcattaatgctgtattgaaagtgcgacttgccttcatggaggaatgggatattggtgagcaaatgctgcgaaatttgtacactgagatagtgtatacaccaatcctcacaccggatggtactatcattaagaagcataaaggcaacaatagcgggcaaccttcaacagtggtggacaacacactcatggtcattattgcaatgttatacacatgtgagaagtgtggaatcaacaaggaagagattgtgtattacgtcaatggcgatgacctattgattgccattcacccagataaagctgagaggttgagtggattcaaagaatctttcggagagttgggcctgaaatatgaatttgactgcaccaccagggacaagacacagttgtggttcatgtcacacagggctttggagagggatggcatgtatataccaaagctagaagaagaaaggattgtttctattttggaatgggacagatccaaagagccgtcacataggcttgaagccatctgtgcatcaatgatcgaagcatggggttatgacaagctggttgaagaaatccgcaatttctatgcatgggttttggaacaagcgccgtattcacagcttgcagaagaaggaaaggcgccatatctggctgagactgcgcttaagtttttgtacacatctcagcacggaacaaactctgagatagaagagtatttaaaagtgttgtatgattacgatattccaacgactgagaatctttattttcagtcaggtacaatgtctataaatataagggaccctcttatagtaagcagagttgttggcgacgttcttgatccgtttaatagatcaatcactctaaaggttacttatggccaaagagaggtgactaatggcttggatctaaggccttctcaggttcaaaacaagccaagagttgagattggtggagaagacctcaggaacttctatactttggttatggtggatccagatgttccaagtcctagcaaccctcacctccgagaatatctccattggttggtgactgatatccctgctacaactggaacaacctttggcaatgagattgtgtgttacgaaaatccaagtcccactgcaggaattcatcgtgtcgtgtttatattgtttcgacagcttggcaggcaaacagtgtatgcaccagggtggcgccagaacttcaacactcgcgagtttgctgagatctacaatctcggccttcccgtggccgcagttttctacaattgtcagagggagagtggctgcggaggaagaagacttactacagagaacctctactttcaaagtggcactgtgggtgctggtgttgacgctggtaagaagaaagatcaaaaggatgataaagtcgctgagcaggcttcaaaggatagggatgttaatgctggaacttcaggaacattctcagttccacgaataaatgctatggccacaaaacttcaatatccaaggatgaggggagaggtggttgtaaacttgaatcaccttttaggatacaagccacagcaaattgatttgtcaaatgctcgagccacacatgagcagtttgccgcgtggcatcaggcagtgatgacagcctatggagtgaatgaagagcaaatgaaaatattgctaaatggatttatggtgtggtgcatagaaaatgggacttccccaaatttgaacggaacttgggttatgatggatggtgaggagcaagtttcatacccgctgaaaccaatggttgaaaacgcgcagccaacactgaggcaaattatgacacacttcagtgacctggctgaagcgtatattgagatgaggaatagggagcgaccatacatgcctaggtatggtctacagagaaacattacagacatgagtttgtcacgctatgcgttcgacttctatgagctaacttcaaaaacacctgttagagcgagggaggcgcatatgcaaatgaaagctgctgcagtacgaaacagtggaactaggttatttggtcttgatggcaacgtgggtactgcagaggaagacactgaacggcacacagcgcacgatgtgaaccgtaacatgcacacactattaggggtccgccagtgatagtttctgcgtgtctttgctttccgcttttaagcttattgtaatatatatgaatagctattcacagtgggacttggtcttgtgttgaatggtatcttatatgttttaatatgtcttattagtctcattacttaggcgaacgacaaagtgaggtcacctcggtctaattctcctatgtagtgcgagaaaaaaaaaaaaaaaaaaaaaaaaaaaaaaaaaaaaaaaaaaaaagatctcgctgaaatcaccagtctctctctacaaatctatctctctctattttctccataaataatgtgtgagtagtttcccgataagggaaattagggttcttatagggtttcgctcatgtgttgagcatataagaaacccttagtatgtatttgtatttgtaaaatacttctatcaataaaatttctaattcctaaaaccaaaatccaggggccctcgacgttccttgacaggatatattggcgggtaaactaagtcgctgtatgtgtttgtttgagatcctctagggcatgcaagctgatctggatctcatgtgagcaaaaggccagcaaaaggccaggaaccgtaaaaaggccgcgttgctggcgtttttccataggctccgcccccctgacgagcatcacaaaaatcgacgctcaagtcagaggtggcgaaacccgacaggactataaagataccaggcgtttccccctggaagctccctcgtgcgctctcctgttccgaccctgccgcttaccggatacctgtccgcctttctcccttcgggaagcgtggcgctttctcatagctcacgctgtaggtatctcagttcggtgtaggtcgttcgctccaagctgggctgtgtgcacgaaccccccgttcagcccgaccgctgcgccttatccggtaactatcgtcttgagtccaacccggtaagacacgacttatcgccactggcagcagccactggtaacaggattagcagagcgaggtatgtaggcggtgctacagagttcttgaagtggtggcctaactacggctacactagaagaacagtatttggtatctgcgctctgctgaagccagttaccttcggaagaagagttggtagctcttgatccggcaaacaaaccaccgctggtagcggtggtttttttgtttgcaagcagcagattacgcgcagaaaaaaaggatctcaagaagatcctttgatcttttctacggggtctgacgctcagtggaacgaaaactcacgttaagggattttggtcatgagattatcaaaaaggatcttcacctagatccttttaaattaaaaatgaagttttaaatcaatctaaagtatatatgtgtaacattggtctagtgattagaaaaactcatcgagcatcaaatgaaactgcaatttattcatatcaggattatcaataccatatttttgaaaaagccgtttctgtaatgaaggagaaaactcaccgaggcagttccataggatggcaagatcctggtatcggtctgcgattccgactcgtccaacatcaatacaacctattaatttcccctcgtcaaaaataaggttatcaagtgagaaatcaccatgagtgacgactgaatccggtgagaatggcaaaagtttatgcatttctttccagacttgttcaacaggccagccattacgctcgtcatcaaaatcactcgcatcaaccaaaccgttattcattcgtgattgcgcctgagcgagacgaaatacgcgatcgctgttaaaaggacaattacaaacaggaatcgaatgcaaccggcgcaggaacactgccagcgcatcaacaatattttcacctgaatcaggatattcttctaatacctggaatgctgttttccctgggatcgcagtggtgagtaaccatgcatcatcaggagtacggataaaatgcttgatggtcggaagaggcataaattccgtcagccagtttagtctgaccatctcatctgtaacaacattggcaacgctacctttgccatgtttcagaaacaactctggcgcatcgggcttcccatacaatcggtagattgtcgcacctgattgcccgacattatcgcgagcccatttatacccatataaatcagcatccatgttggaatttaatcgcggccttgagcaagacgtttcccgttgaatatggctcataacaccccttgtattactgtttatgtaagcagacagttttattgttcatgatgatatatttttatcttgtgcaatgtaacatcagagattttgagacacaacgtggctttgttgaataaatcgaacttttgctgagttgaaggatcagatcacgcatcttcccgacaacgcagaccgttccgtggcaaagcaaaagttcaaaatcaccaactggtccacctacaacaaagctctcatcaaccgtggctccctcactttctggctggatgatggggcgattcaggcgatccccatccaacagcccgccgtcgagcgggcttttttatccccggaagcctgtggatagagggtagttatccacgtgaaaccgctaatgccccgcaaagccttgattcacggggctttccggcccgctccaaaaactatccacgtgaaatcgctaatcagggtacgtgaaatcgctaatcggagtacgtgaaatcgctaataaggtcacgtgaaatcgctaatcaaaaaggcacgtgagaacgctaatagccctttcagatcaacagcttgcaaacacccctcgctccggcaagtagttacagcaagtagtatgttcaattagcttttcaattatgaatatatatatcaattattggtcgcccttggcttgtggacaatgcgctacgcgcaccggctccgcccgtggacaaccgcaagcggttgcccaccgtcgagcgcctttgcccacaacccggcggccggccgcaacagatcgttttataaatttttttttttgaaaaagaaaaagcccgaaaggcggcaacctctcgggcttctggatttccgatccccggaattagatccgtttaaactacgtaagatcgatcttggcaggatatattgtggtgtaaacgttcctgcggcggtcgagatggatcttggcaggatatattgtggtgtaaacgttcct